European Patent Application EP 4 382 601 A1, published June 12, 2024. Title: 用于治疗由于ND4突变造成的莱伯氏遗传性视神经病变的组合物和方法. Applicant: 武汉纽福斯生物科技有限公司. The sequence listing filed with the application follows.

SEQUENCE LISTING (185 sequences)

SEQ ID NO: 1 - DNA, 84 bp, synthetic construct
  source 1..84: mol_type = other DNA
atggccgcatctccgcacactctctcctcacgcctcctgacaggttgcgtaggaggctctgtctggtatcttgaaagaagaact

SEQ ID NO: 2 - DNA, 84 bp, synthetic construct
  source 1..84: mol_type = other DNA
atggccgcctctccacacacactgagtagcagactgctgaccggctgtgttggcggctctgtgtggtatctggaacggcggaca

SEQ ID NO: 3 - DNA, 84 bp, synthetic construct
  source 1..84: mol_type = other DNA
atggccgccagcccccacaccctgagcagccgcctgctgaccggctgcgtgggcggcagcgtgtggtacctggagcgccgcacc

SEQ ID NO: 4 - DNA, 87 bp, synthetic construct
  source 1..87: mol_type = other DNA
atgtccgtcctgacgcgcctgctgctgcggggcttgacacggctcggctcggcggctccagtgcggcgcgccagaatccattcgttg

SEQ ID NO: 5 - DNA, 266 bp, synthetic construct
  source 1..266: mol_type = other DNA
gtgctgcccgcctagaaagggtgaagtggttgtttccgtgacggactgagtacgggtgcctgtcaggctcttgcggaagtccatgcgccattgggagggcctcggccgcggctctgtgcccttgctgctgagggccacttcctgggtcattcctggaccgggagccgggctggggctcacacgggggctcccgcgtggccgtctcggcgcctgcgtgacctccccgccggcgggatgtggcgactacgtcgggccgctgtggcctg

SEQ ID NO: 6 - DNA, 1380 bp, synthetic construct
  source 1..1380: mol_type = other DNA
atgctaaaactaatcgtcccaacaattatgttactaccactgacatggctttccaaaaaacacatgatttggatcaacacaaccacccacagcctaattattagcatcatccctctactattttttaaccaaatcaacaacaacctatttagctgttccccaaccttttcctccgaccccctaacaacccccctcctaatgctaactacctggctcctacccctcacaatcatggcaagccaacgccacttatccagtgaaccactatcacgaaaaaaactctacctctctatgctaatctccctacaaatctccttaattatgacattcacagccacagaactaatcatgttttatatcttcttcgaaaccacacttatccccaccttggctatcatcacccgatggggcaaccagccagaacgcctgaacgcaggcacatacttcctattctacaccctagtaggctcccttcccctactcatcgcactaatttacactcacaacaccctaggctcactaaacattctactactcactctcactgcccaagaactatcaaactcctgggccaacaacttaatgtggctagcttacacaatggcttttatggtaaagatgcctctttacggactccacttatggctccctaaagcccatgtcgaagcccccatcgctgggtcaatggtacttgccgcagtactcttaaaactaggcggctatggtatgatgcgcctcacactcattctcaaccccctgacaaaacacatggcctaccccttccttgtactatccctatggggcatgattatgacaagctccatctgcctacgacaaacagacctaaaatcgctcattgcatactcttcaatcagccacatggccctcgtagtaacagccattctcatccaaaccccctggagcttcaccggcgcagtcattctcatgatcgcccacgggcttacatcctcattactattctgcctagcaaactcaaactacgaacgcactcacagtcgcatcatgatcctctctcaaggacttcaaactctactcccactaatggctttttggtggcttctagcaagcctcgctaacctcgccttaccccccactattaacctactgggagaactctctgtgctagtaaccacgttctcctggtcaaatatcactctcctacttacaggactcaacatgctagtcacagccctatactccctctacatgtttaccacaacacaatggggctcactcacccaccacattaacaacatgaaaccctcattcacacgagaaaacaccctcatgttcatgcacctatcccccattctcctcctatccctcaaccccgacatcattaccgggttttcctcttaa

SEQ ID NO: 7 - DNA, 1380 bp, synthetic construct
  source 1..1380: mol_type = other DNA
atgctgaagctgatcgtgcccaccatcatgctgctgcctctgacctggctgagcaagaaacacatgatctggatcaacaccaccacgcacagcctgatcatcagcatcatccctctgctgttcttcaaccagatcaacaacaacctgttcagctgcagccccaccttcagcagcgaccctctgacaacacctctgctgatgctgaccacctggctgctgcccctcacaatcatggcctctcagagacacctgagcagcgagcccctgagccggaagaaactgtacctgagcatgctgatctccctgcagatctctctgatcatgaccttcaccgccaccgagctgatcatgttctacatctttttcgagacaacgctgatccccacactggccatcatcaccagatggggcaaccagcctgagagactgaacgccggcacctactttctgttctacaccctcgtgggcagcctgccactgctgattgccctgatctacacccacaacaccctgggctccctgaacatcctgctgctgacactgacagcccaagagctgagcaacagctgggccaacaatctgatgtggctggcctacacaatggccttcatggtcaagatgcccctgtacggcctgcacctgtggctgcctaaagctcatgtggaagcccctatcgccggctctatggtgctggctgcagtgctgctgaaactcggcggctacggcatgatgcggctgaccctgattctgaatcccctgaccaagcacatggcctatccatttctggtgctgagcctgtggggcatgattatgaccagcagcatctgcctgcggcagaccgatctgaagtccctgatcgcctacagctccatcagccacatggccctggtggtcaccgccatcctgattcagaccccttggagctttacaggcgccgtgatcctgatgattgcccacggcctgacaagcagcctgctgttttgtctggccaacagcaactacgagcggacccacagcagaatcatgatcctgtctcagggcctgcagaccctcctgcctcttatggctttttggtggctgctggcctctctggccaatctggcactgcctcctaccatcaatctgctgggcgagctgagcgtgctggtcaccacattcagctggtccaatatcaccctgctgctcaccggcctgaacatgctggttacagccctgtactccctgtacatgttcaccaccacacagtggggaagcctgacacaccacatcaacaatatgaagcccagcttcacccgcgagaacaccctgatgttcatgcatctgagccccattctgctgctgtccctgaatcctgatatcatcaccggcttctccagctga

SEQ ID NO: 8 - DNA, 1380 bp, synthetic construct
  source 1..1380: mol_type = other DNA
atgctgaagctgatcgtgcccaccatcatgctgctgcccctgacctggctgagcaagaagcacatgatctggatcaacaccaccacccacagcctgatcatcagcatcatccccctgctgttcttcaaccagatcaacaacaacctgttcagctgcagccccaccttcagcagcgaccccctgaccacccccctgctgatgctgaccacctggctgctgcccctgaccatcatggccagccagcgccacctgagcagcgagcccctgagccgcaagaagctgtacctgagcatgctgatcagcctgcagatcagcctgatcatgaccttcaccgccaccgagctgatcatgttctacatcttcttcgagaccaccctgatccccaccctggccatcatcacccgctggggcaaccagcccgagcgcctgaacgccggcacctacttcctgttctacaccctggtgggcagcctgcccctgctgatcgccctgatctacacccacaacaccctgggcagcctgaacatcctgctgctgaccctgaccgcccaggagctgagcaacagctgggccaacaacctgatgtggctggcctacaccatggccttcatggtgaagatgcccctgtacggcctgcacctgtggctgcccaaggcccacgtggaggcccccatcgccggcagcatggtgctggccgccgtgctgctgaagctgggcggctacggcatgatgcgcctgaccctgatcctgaaccccctgaccaagcacatggcctaccccttcctggtgctgagcctgtggggcatgatcatgaccagcagcatctgcctgcgccagaccgacctgaagagcctgatcgcctacagcagcatcagccacatggccctggtggtgaccgccatcctgatccagaccccctggagcttcaccggcgccgtgatcctgatgatcgcccacggcctgaccagcagcctgctgttctgcctggccaacagcaactacgagcgcacccacagccgcatcatgatcctgagccagggcctgcagaccctgctgcccctgatggccttctggtggctgctggccagcctggccaacctggccctgccccccaccatcaacctgctgggcgagctgagcgtgctggtgaccaccttcagctggagcaacatcaccctgctgctgaccggcctgaacatgctggtgaccgccctgtacagcctgtacatgttcaccaccacccagtggggcagcctgacccaccacatcaacaacatgaagcccagcttcacccgcgagaacaccctgatgttcatgcacctgagccccatcctgctgctgagcctgaaccccgacatcatcaccggcttcagcagctaa

SEQ ID NO: 9 - DNA, 525 bp, synthetic construct
  source 1..525: mol_type = other DNA
atgatgtatgctttgtttctgttgagtgtgggtttagtaatggggtttgtggggttttcttctaagccttctcctatttatgggggtttagtattgattgttagcggtgtggtcgggtgtgttattattctgaattttgggggaggttatatgggtttaatggtttttttaatttatttagggggaatgatggttgtctttggatatactacagcgatggctattgaggagtatcctgaggcatgggggtcaggggttgaggtcttggtgagtgttttagtggggttagcgatggaggtaggattggtgctgtgggtgaaagagtatgatggggtggtggttgtggtaaactttaatagtgtaggaagctggatgatttatgaaggagaggggtcagggttgattcgggaggatcctattggtgcgggggctttgtatgattatgggcgttggttagtagtagttactggttggacattgtttgttggtgtatatattgtaattgagattgctcgggggaattag

SEQ ID NO: 10 - DNA, 525 bp, synthetic construct
  source 1..525: mol_type = other DNA
atgatgtacgccctgttcctgctgagcgtgggcctggtgatgggcttcgtgggcttcagcagcaagcccagccccatctacggcggcctggtgctgatcgtgagcggcgtggtgggctgcgtgatcatcctgaacttcggcggcggctacatgggcctgatggtgttcctgatctacctgggcggcatgatggtggtgttcggctacaccaccgccatggccatcgaggagtaccccgaggcctggggcagcggcgtggaggtgctggtgagcgtgctggtgggcctggccatggaggtgggcctggtgctgtgggtgaaggagtacgacggcgtggtggtggtggtgaacttcaacagcgtgggcagctggatgatctacgagggcgagggcagcggcctgatccgcgaggaccccatcggcgccggcgccctgtacgactacggccgctggctggtggtggtgaccggctggaccctgttcgtgggcgtgtacatcgtgatcgagatcgcccgcggcaactaa

SEQ ID NO: 11 - DNA, 951 bp, synthetic construct
  source 1..951: mol_type = other DNA
atggccaacctcctactcctcattgtacccattctaatcgcaatggcattcctaatgcttaccgaacgaaaaattctaggctatatgcaactacgcaaaggccccaacgttgtaggcccctacgggctactacaacccttcgctgacgccataaaactcttcaccaaagagcccctaaaacccgccacatctaccatcaccctctacatcaccgccccgaccttagctctcaccatcgctcttctactatggacccccctccccatgcccaaccccctggtcaacctcaacctaggcctcctatttattctagccacctctagcctagccgtttactcaatcctctggtcagggtgggcatcaaactcaaactacgccctgatcggcgcactgcgagcagtagcccaaacaatctcatatgaagtcaccctagccatcattctactatcaacattactaatgagtggctcctttaacctctccacccttatcacaacacaagaacacctctggttactcctgccatcatggcccttggccatgatgtggtttatctccacactagcagagaccaaccgaacccccttcgaccttgccgaaggggagtccgaactagtctcaggcttcaacatcgaatacgccgcaggccccttcgccctattcttcatggccgaatacacaaacattattatgatgaacaccctcaccactacaatcttcctaggaacaacatatgacgcactctcccctgaactctacacaacatattttgtcaccaagaccctacttctaacctccctgttcttatggattcgaacagcatacccccgattccgctacgaccaactcatgcacctcctatggaaaaacttcctaccactcaccctagcattacttatgtggtatgtctccatgcccattacaatctccagcattccccctcaaacctaa

SEQ ID NO: 12 - DNA, 951 bp, synthetic construct
  source 1..951: mol_type = other DNA
atggccaacctgctgctgctgatcgtgcccatcctgatcgccatggccttcctgatgctgaccgagcgcaagatcctgggctacatgcagctgcgcaagggccccaacgtggtgggcccctacggcctgctgcagcccttcgccgacgccatcaagctgttcaccaaggagcccctgaagcccgccaccagcaccatcaccctgtacatcaccgcccccaccctggccctgaccatcgccctgctgctgtggacccccctgcccatgcccaaccccctggtgaacctgaacctgggcctgctgttcatcctggccaccagcagcctggccgtgtacagcatcctgtggagcggctgggccagcaacagcaactacgccctgatcggcgccctgcgcgccgtggcccagaccatcagctacgaggtgaccctggccatcatcctgctgagcaccctgctgatgagcggcagcttcaacctgagcaccctgatcaccacccaggagcacctgtggctgctgctgcccagctggcccctggccatgatgtggttcatcagcaccctggccgagaccaaccgcacccccttcgacctggccgagggcgagagcgagctggtgagcggcttcaacatcgagtacgccgccggccccttcgccctgttcttcatggccgagtacaccaacatcatcatgatgaacaccctgaccaccaccatcttcctgggcaccacctacgacgccctgagccccgagctgtacaccacctacttcgtgaccaagaccctgctgctgaccagcctgttcctgtggatccgcaccgcctacccccgcttccgctacgaccagctgatgcacctgctgtggaagaacttcctgcccctgaccctggccctgctgatgtggtacgtgagcatgcccatcaccatcagcagcatccccccccagacctaa

SEQ ID NO: 13 - DNA, 1425 bp, synthetic construct
  source 1..1425: mol_type = other DNA
gagcactgggacgcccaccgcccctttccctccgctgccaggcgagcatgttgtggtaattctggaacacaagaagagaaattgctgggtttagaacaagattataaacgaattcggtgctcagtgatcacttgacagttttttttttttttaaatattacccaaaatgctccccaaataagaaatgcatcagctcagtcagtgaatacaaaaaaggaattatttttccctttgagggtcttttatacatctctcctccaaccccaccctctattctgtttcttcctcctcacatgggggtacacatacacagcttcctcttttggttccatccttaccaccacaccacacgcacactccacatgcccagcagagtggcacttggtggccagaaagtgtgagcctcatgatctgctgtctgtagttctgtgagctcaggtccctcaaaggcctcggagcacccccttccttgtgactgagccagggcctgcatttttggttttccccaccccacacattctcaaccatagtccttctaacaataccaatagctaggacccggctgctgtgcactgggactggggattccacatgtttgccttgggagtctcaagctggactgccagcccctgtcctcccttcacccccattgcgtatgagcatttcagaactccaaggagtcacaggcatctttatagttcacgttaacatatagacactgttggaagcagttccttctaaaagggtagccctggacttaataccagccggatacctctggcccccaccccattactgtacctctggagtcactactgtgggtcgccactcctctgctacacagcacggctttttcaaggctgtattgagaagggaagttaggaagaagggtgtgctgggctaaccagcccacagagctcacattcctgtcccttgggtgaaaaatacatgtccatcctgatatctcctgaattcagaaattagcctccacatgtgcaatggctttaagagccagaagcagggttctgggaattttgcaagttacctgtggccaggtgtggtctcggttaccaaatacggttacctgcagctttttagtcctttgtgctcccacgggtctacagagtcccatctgcccaaaggtcttgaagcttgacaggatgttttcgattactcagtctcccagggcactactggtccgtaggattcgattggtcggggtaggagagttaaacaacatttaaacagagttctctcaaaaatgtctaaagggattgtaggtagataacatccaatcactgtttgcacttatctgaaatcttccctcttggctgcccccaggtatttactgtggagaacattgcataggaatgtctggaaaaagcttctacaacttgttacagccttcacatttgtagaagcttt

SEQ ID NO: 14 - DNA, 625 bp, synthetic construct
  source 1..625: mol_type = other DNA
gagcactgggacgcccaccgcccctttccctccgctgccaggcgagcatgttgtggtaattctggaacacaagaagagaaattgctgggtttagaacaagattataaacgaattcggtgctcagtgatcacttgacagttttttttttttttaaatattacccaaaatgctccccaaataagaaatgcatcagctcagtcagtgaatacaaaaaaggaattatttttccctttgagggtcttttatacatctctcctccaaccccaccctctattctgtttcttcctcctcacatgggggtacacatacacagcttcctcttttggttccatccttaccaccacaccacacgcacactccacatgcccagcagagtggcacttggtggccagaaagtgtgagcctcatgatctgctgtctgtagttctgtgagctcaggtccctcaaaggcctcggagcacccccttccttgtgactgagccagggcctgcatttttggttttccccaccccacacattctcaaccatagtccttctaacaataccaatagctaggacccggctgctgtgcactgggactggggattccacatgtttgccttgggagtctcaagctggactgcca

SEQ ID NO: 15 - DNA, 2889 bp, synthetic construct
  source 1..2889: mol_type = other DNA
atggccgcatctccgcacactctctcctcacgcctcctgacaggttgcgtaggaggctctgtctggtatcttgaaagaagaactatgctaaaactaatcgtcccaacaattatgttactaccactgacatggctttccaaaaaacacatgatttggatcaacacaaccacccacagcctaattattagcatcatccctctactattttttaaccaaatcaacaacaacctatttagctgttccccaaccttttcctccgaccccctaacaacccccctcctaatgctaactacctggctcctacccctcacaatcatggcaagccaacgccacttatccagtgaaccactatcacgaaaaaaactctacctctctatgctaatctccctacaaatctccttaattatgacattcacagccacagaactaatcatgttttatatcttcttcgaaaccacacttatccccaccttggctatcatcacccgatggggcaaccagccagaacgcctgaacgcaggcacatacttcctattctacaccctagtaggctcccttcccctactcatcgcactaatttacactcacaacaccctaggctcactaaacattctactactcactctcactgcccaagaactatcaaactcctgggccaacaacttaatgtggctagcttacacaatggcttttatggtaaagatgcctctttacggactccacttatggctccctaaagcccatgtcgaagcccccatcgctgggtcaatggtacttgccgcagtactcttaaaactaggcggctatggtatgatgcgcctcacactcattctcaaccccctgacaaaacacatggcctaccccttccttgtactatccctatggggcatgattatgacaagctccatctgcctacgacaaacagacctaaaatcgctcattgcatactcttcaatcagccacatggccctcgtagtaacagccattctcatccaaaccccctggagcttcaccggcgcagtcattctcatgatcgcccacgggcttacatcctcattactattctgcctagcaaactcaaactacgaacgcactcacagtcgcatcatgatcctctctcaaggacttcaaactctactcccactaatggctttttggtggcttctagcaagcctcgctaacctcgccttaccccccactattaacctactgggagaactctctgtgctagtaaccacgttctcctggtcaaatatcactctcctacttacaggactcaacatgctagtcacagccctatactccctctacatgtttaccacaacacaatggggctcactcacccaccacattaacaacatgaaaccctcattcacacgagaaaacaccctcatgttcatgcacctatcccccattctcctcctatccctcaaccccgacatcattaccgggttttcctcttaagagcactgggacgcccaccgcccctttccctccgctgccaggcgagcatgttgtggtaattctggaacacaagaagagaaattgctgggtttagaacaagattataaacgaattcggtgctcagtgatcacttgacagttttttttttttttaaatattacccaaaatgctccccaaataagaaatgcatcagctcagtcagtgaatacaaaaaaggaattatttttccctttgagggtcttttatacatctctcctccaaccccaccctctattctgtttcttcctcctcacatgggggtacacatacacagcttcctcttttggttccatccttaccaccacaccacacgcacactccacatgcccagcagagtggcacttggtggccagaaagtgtgagcctcatgatctgctgtctgtagttctgtgagctcaggtccctcaaaggcctcggagcacccccttccttgtgactgagccagggcctgcatttttggttttccccaccccacacattctcaaccatagtccttctaacaataccaatagctaggacccggctgctgtgcactgggactggggattccacatgtttgccttgggagtctcaagctggactgccagcccctgtcctcccttcacccccattgcgtatgagcatttcagaactccaaggagtcacaggcatctttatagttcacgttaacatatagacactgttggaagcagttccttctaaaagggtagccctggacttaataccagccggatacctctggcccccaccccattactgtacctctggagtcactactgtgggtcgccactcctctgctacacagcacggctttttcaaggctgtattgagaagggaagttaggaagaagggtgtgctgggctaaccagcccacagagctcacattcctgtcccttgggtgaaaaatacatgtccatcctgatatctcctgaattcagaaattagcctccacatgtgcaatggctttaagagccagaagcagggttctgggaattttgcaagttacctgtggccaggtgtggtctcggttaccaaatacggttacctgcagctttttagtcctttgtgctcccacgggtctacagagtcccatctgcccaaaggtcttgaagcttgacaggatgttttcgattactcagtctcccagggcactactggtccgtaggattcgattggtcggggtaggagagttaaacaacatttaaacagagttctctcaaaaatgtctaaagggattgtaggtagataacatccaatcactgtttgcacttatctgaaatcttccctcttggctgcccccaggtatttactgtggagaacattgcataggaatgtctggaaaaagcttctacaacttgttacagccttcacatttgtagaagcttt

SEQ ID NO: 16 - DNA, 2089 bp, synthetic construct
  source 1..2089: mol_type = other DNA
atggccgcatctccgcacactctctcctcacgcctcctgacaggttgcgtaggaggctctgtctggtatcttgaaagaagaactatgctaaaactaatcgtcccaacaattatgttactaccactgacatggctttccaaaaaacacatgatttggatcaacacaaccacccacagcctaattattagcatcatccctctactattttttaaccaaatcaacaacaacctatttagctgttccccaaccttttcctccgaccccctaacaacccccctcctaatgctaactacctggctcctacccctcacaatcatggcaagccaacgccacttatccagtgaaccactatcacgaaaaaaactctacctctctatgctaatctccctacaaatctccttaattatgacattcacagccacagaactaatcatgttttatatcttcttcgaaaccacacttatccccaccttggctatcatcacccgatggggcaaccagccagaacgcctgaacgcaggcacatacttcctattctacaccctagtaggctcccttcccctactcatcgcactaatttacactcacaacaccctaggctcactaaacattctactactcactctcactgcccaagaactatcaaactcctgggccaacaacttaatgtggctagcttacacaatggcttttatggtaaagatgcctctttacggactccacttatggctccctaaagcccatgtcgaagcccccatcgctgggtcaatggtacttgccgcagtactcttaaaactaggcggctatggtatgatgcgcctcacactcattctcaaccccctgacaaaacacatggcctaccccttccttgtactatccctatggggcatgattatgacaagctccatctgcctacgacaaacagacctaaaatcgctcattgcatactcttcaatcagccacatggccctcgtagtaacagccattctcatccaaaccccctggagcttcaccggcgcagtcattctcatgatcgcccacgggcttacatcctcattactattctgcctagcaaactcaaactacgaacgcactcacagtcgcatcatgatcctctctcaaggacttcaaactctactcccactaatggctttttggtggcttctagcaagcctcgctaacctcgccttaccccccactattaacctactgggagaactctctgtgctagtaaccacgttctcctggtcaaatatcactctcctacttacaggactcaacatgctagtcacagccctatactccctctacatgtttaccacaacacaatggggctcactcacccaccacattaacaacatgaaaccctcattcacacgagaaaacaccctcatgttcatgcacctatcccccattctcctcctatccctcaaccccgacatcattaccgggttttcctcttaagagcactgggacgcccaccgcccctttccctccgctgccaggcgagcatgttgtggtaattctggaacacaagaagagaaattgctgggtttagaacaagattataaacgaattcggtgctcagtgatcacttgacagttttttttttttttaaatattacccaaaatgctccccaaataagaaatgcatcagctcagtcagtgaatacaaaaaaggaattatttttccctttgagggtcttttatacatctctcctccaaccccaccctctattctgtttcttcctcctcacatgggggtacacatacacagcttcctcttttggttccatccttaccaccacaccacacgcacactccacatgcccagcagagtggcacttggtggccagaaagtgtgagcctcatgatctgctgtctgtagttctgtgagctcaggtccctcaaaggcctcggagcacccccttccttgtgactgagccagggcctgcatttttggttttccccaccccacacattctcaaccatagtccttctaacaataccaatagctaggacccggctgctgtgcactgggactggggattccacatgtttgccttgggagtctcaagctggactgcca

SEQ ID NO: 17 - DNA, 2889 bp, synthetic construct
  source 1..2889: mol_type = other DNA
atggccgcatctccgcacactctctcctcacgcctcctgacaggttgcgtaggaggctctgtctggtatcttgaaagaagaactatgctgaagctgatcgtgcccaccatcatgctgctgcctctgacctggctgagcaagaaacacatgatctggatcaacaccaccacgcacagcctgatcatcagcatcatccctctgctgttcttcaaccagatcaacaacaacctgttcagctgcagccccaccttcagcagcgaccctctgacaacacctctgctgatgctgaccacctggctgctgcccctcacaatcatggcctctcagagacacctgagcagcgagcccctgagccggaagaaactgtacctgagcatgctgatctccctgcagatctctctgatcatgaccttcaccgccaccgagctgatcatgttctacatctttttcgagacaacgctgatccccacactggccatcatcaccagatggggcaaccagcctgagagactgaacgccggcacctactttctgttctacaccctcgtgggcagcctgccactgctgattgccctgatctacacccacaacaccctgggctccctgaacatcctgctgctgacactgacagcccaagagctgagcaacagctgggccaacaatctgatgtggctggcctacacaatggccttcatggtcaagatgcccctgtacggcctgcacctgtggctgcctaaagctcatgtggaagcccctatcgccggctctatggtgctggctgcagtgctgctgaaactcggcggctacggcatgatgcggctgaccctgattctgaatcccctgaccaagcacatggcctatccatttctggtgctgagcctgtggggcatgattatgaccagcagcatctgcctgcggcagaccgatctgaagtccctgatcgcctacagctccatcagccacatggccctggtggtcaccgccatcctgattcagaccccttggagctttacaggcgccgtgatcctgatgattgcccacggcctgacaagcagcctgctgttttgtctggccaacagcaactacgagcggacccacagcagaatcatgatcctgtctcagggcctgcagaccctcctgcctcttatggctttttggtggctgctggcctctctggccaatctggcactgcctcctaccatcaatctgctgggcgagctgagcgtgctggtcaccacattcagctggtccaatatcaccctgctgctcaccggcctgaacatgctggttacagccctgtactccctgtacatgttcaccaccacacagtggggaagcctgacacaccacatcaacaatatgaagcccagcttcacccgcgagaacaccctgatgttcatgcatctgagccccattctgctgctgtccctgaatcctgatatcatcaccggcttctccagctgagagcactgggacgcccaccgcccctttccctccgctgccaggcgagcatgttgtggtaattctggaacacaagaagagaaattgctgggtttagaacaagattataaacgaattcggtgctcagtgatcacttgacagttttttttttttttaaatattacccaaaatgctccccaaataagaaatgcatcagctcagtcagtgaatacaaaaaaggaattatttttccctttgagggtcttttatacatctctcctccaaccccaccctctattctgtttcttcctcctcacatgggggtacacatacacagcttcctcttttggttccatccttaccaccacaccacacgcacactccacatgcccagcagagtggcacttggtggccagaaagtgtgagcctcatgatctgctgtctgtagttctgtgagctcaggtccctcaaaggcctcggagcacccccttccttgtgactgagccagggcctgcatttttggttttccccaccccacacattctcaaccatagtccttctaacaataccaatagctaggacccggctgctgtgcactgggactggggattccacatgtttgccttgggagtctcaagctggactgccagcccctgtcctcccttcacccccattgcgtatgagcatttcagaactccaaggagtcacaggcatctttatagttcacgttaacatatagacactgttggaagcagttccttctaaaagggtagccctggacttaataccagccggatacctctggcccccaccccattactgtacctctggagtcactactgtgggtcgccactcctctgctacacagcacggctttttcaaggctgtattgagaagggaagttaggaagaagggtgtgctgggctaaccagcccacagagctcacattcctgtcccttgggtgaaaaatacatgtccatcctgatatctcctgaattcagaaattagcctccacatgtgcaatggctttaagagccagaagcagggttctgggaattttgcaagttacctgtggccaggtgtggtctcggttaccaaatacggttacctgcagctttttagtcctttgtgctcccacgggtctacagagtcccatctgcccaaaggtcttgaagcttgacaggatgttttcgattactcagtctcccagggcactactggtccgtaggattcgattggtcggggtaggagagttaaacaacatttaaacagagttctctcaaaaatgtctaaagggattgtaggtagataacatccaatcactgtttgcacttatctgaaatcttccctcttggctgcccccaggtatttactgtggagaacattgcataggaatgtctggaaaaagcttctacaacttgttacagccttcacatttgtagaagcttt

SEQ ID NO: 18 - DNA, 2089 bp, synthetic construct
  source 1..2089: mol_type = other DNA
atggccgcatctccgcacactctctcctcacgcctcctgacaggttgcgtaggaggctctgtctggtatcttgaaagaagaactatgctgaagctgatcgtgcccaccatcatgctgctgcctctgacctggctgagcaagaaacacatgatctggatcaacaccaccacgcacagcctgatcatcagcatcatccctctgctgttcttcaaccagatcaacaacaacctgttcagctgcagccccaccttcagcagcgaccctctgacaacacctctgctgatgctgaccacctggctgctgcccctcacaatcatggcctctcagagacacctgagcagcgagcccctgagccggaagaaactgtacctgagcatgctgatctccctgcagatctctctgatcatgaccttcaccgccaccgagctgatcatgttctacatctttttcgagacaacgctgatccccacactggccatcatcaccagatggggcaaccagcctgagagactgaacgccggcacctactttctgttctacaccctcgtgggcagcctgccactgctgattgccctgatctacacccacaacaccctgggctccctgaacatcctgctgctgacactgacagcccaagagctgagcaacagctgggccaacaatctgatgtggctggcctacacaatggccttcatggtcaagatgcccctgtacggcctgcacctgtggctgcctaaagctcatgtggaagcccctatcgccggctctatggtgctggctgcagtgctgctgaaactcggcggctacggcatgatgcggctgaccctgattctgaatcccctgaccaagcacatggcctatccatttctggtgctgagcctgtggggcatgattatgaccagcagcatctgcctgcggcagaccgatctgaagtccctgatcgcctacagctccatcagccacatggccctggtggtcaccgccatcctgattcagaccccttggagctttacaggcgccgtgatcctgatgattgcccacggcctgacaagcagcctgctgttttgtctggccaacagcaactacgagcggacccacagcagaatcatgatcctgtctcagggcctgcagaccctcctgcctcttatggctttttggtggctgctggcctctctggccaatctggcactgcctcctaccatcaatctgctgggcgagctgagcgtgctggtcaccacattcagctggtccaatatcaccctgctgctcaccggcctgaacatgctggttacagccctgtactccctgtacatgttcaccaccacacagtggggaagcctgacacaccacatcaacaatatgaagcccagcttcacccgcgagaacaccctgatgttcatgcatctgagccccattctgctgctgtccctgaatcctgatatcatcaccggcttctccagctgagagcactgggacgcccaccgcccctttccctccgctgccaggcgagcatgttgtggtaattctggaacacaagaagagaaattgctgggtttagaacaagattataaacgaattcggtgctcagtgatcacttgacagttttttttttttttaaatattacccaaaatgctccccaaataagaaatgcatcagctcagtcagtgaatacaaaaaaggaattatttttccctttgagggtcttttatacatctctcctccaaccccaccctctattctgtttcttcctcctcacatgggggtacacatacacagcttcctcttttggttccatccttaccaccacaccacacgcacactccacatgcccagcagagtggcacttggtggccagaaagtgtgagcctcatgatctgctgtctgtagttctgtgagctcaggtccctcaaaggcctcggagcacccccttccttgtgactgagccagggcctgcatttttggttttccccaccccacacattctcaaccatagtccttctaacaataccaatagctaggacccggctgctgtgcactgggactggggattccacatgtttgccttgggagtctcaagctggactgcca

SEQ ID NO: 19 - DNA, 2889 bp, synthetic construct
  source 1..2889: mol_type = other DNA
atggccgcatctccgcacactctctcctcacgcctcctgacaggttgcgtaggaggctctgtctggtatcttgaaagaagaactatgctgaagctgatcgtgcccaccatcatgctgctgcccctgacctggctgagcaagaagcacatgatctggatcaacaccaccacccacagcctgatcatcagcatcatccccctgctgttcttcaaccagatcaacaacaacctgttcagctgcagccccaccttcagcagcgaccccctgaccacccccctgctgatgctgaccacctggctgctgcccctgaccatcatggccagccagcgccacctgagcagcgagcccctgagccgcaagaagctgtacctgagcatgctgatcagcctgcagatcagcctgatcatgaccttcaccgccaccgagctgatcatgttctacatcttcttcgagaccaccctgatccccaccctggccatcatcacccgctggggcaaccagcccgagcgcctgaacgccggcacctacttcctgttctacaccctggtgggcagcctgcccctgctgatcgccctgatctacacccacaacaccctgggcagcctgaacatcctgctgctgaccctgaccgcccaggagctgagcaacagctgggccaacaacctgatgtggctggcctacaccatggccttcatggtgaagatgcccctgtacggcctgcacctgtggctgcccaaggcccacgtggaggcccccatcgccggcagcatggtgctggccgccgtgctgctgaagctgggcggctacggcatgatgcgcctgaccctgatcctgaaccccctgaccaagcacatggcctaccccttcctggtgctgagcctgtggggcatgatcatgaccagcagcatctgcctgcgccagaccgacctgaagagcctgatcgcctacagcagcatcagccacatggccctggtggtgaccgccatcctgatccagaccccctggagcttcaccggcgccgtgatcctgatgatcgcccacggcctgaccagcagcctgctgttctgcctggccaacagcaactacgagcgcacccacagccgcatcatgatcctgagccagggcctgcagaccctgctgcccctgatggccttctggtggctgctggccagcctggccaacctggccctgccccccaccatcaacctgctgggcgagctgagcgtgctggtgaccaccttcagctggagcaacatcaccctgctgctgaccggcctgaacatgctggtgaccgccctgtacagcctgtacatgttcaccaccacccagtggggcagcctgacccaccacatcaacaacatgaagcccagcttcacccgcgagaacaccctgatgttcatgcacctgagccccatcctgctgctgagcctgaaccccgacatcatcaccggcttcagcagctaagagcactgggacgcccaccgcccctttccctccgctgccaggcgagcatgttgtggtaattctggaacacaagaagagaaattgctgggtttagaacaagattataaacgaattcggtgctcagtgatcacttgacagttttttttttttttaaatattacccaaaatgctccccaaataagaaatgcatcagctcagtcagtgaatacaaaaaaggaattatttttccctttgagggtcttttatacatctctcctccaaccccaccctctattctgtttcttcctcctcacatgggggtacacatacacagcttcctcttttggttccatccttaccaccacaccacacgcacactccacatgcccagcagagtggcacttggtggccagaaagtgtgagcctcatgatctgctgtctgtagttctgtgagctcaggtccctcaaaggcctcggagcacccccttccttgtgactgagccagggcctgcatttttggttttccccaccccacacattctcaaccatagtccttctaacaataccaatagctaggacccggctgctgtgcactgggactggggattccacatgtttgccttgggagtctcaagctggactgccagcccctgtcctcccttcacccccattgcgtatgagcatttcagaactccaaggagtcacaggcatctttatagttcacgttaacatatagacactgttggaagcagttccttctaaaagggtagccctggacttaataccagccggatacctctggcccccaccccattactgtacctctggagtcactactgtgggtcgccactcctctgctacacagcacggctttttcaaggctgtattgagaagggaagttaggaagaagggtgtgctgggctaaccagcccacagagctcacattcctgtcccttgggtgaaaaatacatgtccatcctgatatctcctgaattcagaaattagcctccacatgtgcaatggctttaagagccagaagcagggttctgggaattttgcaagttacctgtggccaggtgtggtctcggttaccaaatacggttacctgcagctttttagtcctttgtgctcccacgggtctacagagtcccatctgcccaaaggtcttgaagcttgacaggatgttttcgattactcagtctcccagggcactactggtccgtaggattcgattggtcggggtaggagagttaaacaacatttaaacagagttctctcaaaaatgtctaaagggattgtaggtagataacatccaatcactgtttgcacttatctgaaatcttccctcttggctgcccccaggtatttactgtggagaacattgcataggaatgtctggaaaaagcttctacaacttgttacagccttcacatttgtagaagcttt

SEQ ID NO: 20 - DNA, 2089 bp, synthetic construct
  source 1..2089: mol_type = other DNA
atggccgcatctccgcacactctctcctcacgcctcctgacaggttgcgtaggaggctctgtctggtatcttgaaagaagaactatgctgaagctgatcgtgcccaccatcatgctgctgcccctgacctggctgagcaagaagcacatgatctggatcaacaccaccacccacagcctgatcatcagcatcatccccctgctgttcttcaaccagatcaacaacaacctgttcagctgcagccccaccttcagcagcgaccccctgaccacccccctgctgatgctgaccacctggctgctgcccctgaccatcatggccagccagcgccacctgagcagcgagcccctgagccgcaagaagctgtacctgagcatgctgatcagcctgcagatcagcctgatcatgaccttcaccgccaccgagctgatcatgttctacatcttcttcgagaccaccctgatccccaccctggccatcatcacccgctggggcaaccagcccgagcgcctgaacgccggcacctacttcctgttctacaccctggtgggcagcctgcccctgctgatcgccctgatctacacccacaacaccctgggcagcctgaacatcctgctgctgaccctgaccgcccaggagctgagcaacagctgggccaacaacctgatgtggctggcctacaccatggccttcatggtgaagatgcccctgtacggcctgcacctgtggctgcccaaggcccacgtggaggcccccatcgccggcagcatggtgctggccgccgtgctgctgaagctgggcggctacggcatgatgcgcctgaccctgatcctgaaccccctgaccaagcacatggcctaccccttcctggtgctgagcctgtggggcatgatcatgaccagcagcatctgcctgcgccagaccgacctgaagagcctgatcgcctacagcagcatcagccacatggccctggtggtgaccgccatcctgatccagaccccctggagcttcaccggcgccgtgatcctgatgatcgcccacggcctgaccagcagcctgctgttctgcctggccaacagcaactacgagcgcacccacagccgcatcatgatcctgagccagggcctgcagaccctgctgcccctgatggccttctggtggctgctggccagcctggccaacctggccctgccccccaccatcaacctgctgggcgagctgagcgtgctggtgaccaccttcagctggagcaacatcaccctgctgctgaccggcctgaacatgctggtgaccgccctgtacagcctgtacatgttcaccaccacccagtggggcagcctgacccaccacatcaacaacatgaagcccagcttcacccgcgagaacaccctgatgttcatgcacctgagccccatcctgctgctgagcctgaaccccgacatcatcaccggcttcagcagctaagagcactgggacgcccaccgcccctttccctccgctgccaggcgagcatgttgtggtaattctggaacacaagaagagaaattgctgggtttagaacaagattataaacgaattcggtgctcagtgatcacttgacagttttttttttttttaaatattacccaaaatgctccccaaataagaaatgcatcagctcagtcagtgaatacaaaaaaggaattatttttccctttgagggtcttttatacatctctcctccaaccccaccctctattctgtttcttcctcctcacatgggggtacacatacacagcttcctcttttggttccatccttaccaccacaccacacgcacactccacatgcccagcagagtggcacttggtggccagaaagtgtgagcctcatgatctgctgtctgtagttctgtgagctcaggtccctcaaaggcctcggagcacccccttccttgtgactgagccagggcctgcatttttggttttccccaccccacacattctcaaccatagtccttctaacaataccaatagctaggacccggctgctgtgcactgggactggggattccacatgtttgccttgggagtctcaagctggactgcca

SEQ ID NO: 21 - DNA, 2034 bp, synthetic construct
  source 1..2034: mol_type = other DNA
atggccgcatctccgcacactctctcctcacgcctcctgacaggttgcgtaggaggctctgtctggtatcttgaaagaagaactatgatgtatgctttgtttctgttgagtgtgggtttagtaatggggtttgtggggttttcttctaagccttctcctatttatgggggtttagtattgattgttagcggtgtggtcgggtgtgttattattctgaattttgggggaggttatatgggtttaatggtttttttaatttatttagggggaatgatggttgtctttggatatactacagcgatggctattgaggagtatcctgaggcatgggggtcaggggttgaggtcttggtgagtgttttagtggggttagcgatggaggtaggattggtgctgtgggtgaaagagtatgatggggtggtggttgtggtaaactttaatagtgtaggaagctggatgatttatgaaggagaggggtcagggttgattcgggaggatcctattggtgcgggggctttgtatgattatgggcgttggttagtagtagttactggttggacattgtttgttggtgtatatattgtaattgagattgctcgggggaattaggagcactgggacgcccaccgcccctttccctccgctgccaggcgagcatgttgtggtaattctggaacacaagaagagaaattgctgggtttagaacaagattataaacgaattcggtgctcagtgatcacttgacagttttttttttttttaaatattacccaaaatgctccccaaataagaaatgcatcagctcagtcagtgaatacaaaaaaggaattatttttccctttgagggtcttttatacatctctcctccaaccccaccctctattctgtttcttcctcctcacatgggggtacacatacacagcttcctcttttggttccatccttaccaccacaccacacgcacactccacatgcccagcagagtggcacttggtggccagaaagtgtgagcctcatgatctgctgtctgtagttctgtgagctcaggtccctcaaaggcctcggagcacccccttccttgtgactgagccagggcctgcatttttggttttccccaccccacacattctcaaccatagtccttctaacaataccaatagctaggacccggctgctgtgcactgggactggggattccacatgtttgccttgggagtctcaagctggactgccagcccctgtcctcccttcacccccattgcgtatgagcatttcagaactccaaggagtcacaggcatctttatagttcacgttaacatatagacactgttggaagcagttccttctaaaagggtagccctggacttaataccagccggatacctctggcccccaccccattactgtacctctggagtcactactgtgggtcgccactcctctgctacacagcacggctttttcaaggctgtattgagaagggaagttaggaagaagggtgtgctgggctaaccagcccacagagctcacattcctgtcccttgggtgaaaaatacatgtccatcctgatatctcctgaattcagaaattagcctccacatgtgcaatggctttaagagccagaagcagggttctgggaattttgcaagttacctgtggccaggtgtggtctcggttaccaaatacggttacctgcagctttttagtcctttgtgctcccacgggtctacagagtcccatctgcccaaaggtcttgaagcttgacaggatgttttcgattactcagtctcccagggcactactggtccgtaggattcgattggtcggggtaggagagttaaacaacatttaaacagagttctctcaaaaatgtctaaagggattgtaggtagataacatccaatcactgtttgcacttatctgaaatcttccctcttggctgcccccaggtatttactgtggagaacattgcataggaatgtctggaaaaagcttctacaacttgttacagccttcacatttgtagaagcttt

SEQ ID NO: 22 - DNA, 1234 bp, synthetic construct
  source 1..1234: mol_type = other DNA
atggccgcatctccgcacactctctcctcacgcctcctgacaggttgcgtaggaggctctgtctggtatcttgaaagaagaactatgatgtatgctttgtttctgttgagtgtgggtttagtaatggggtttgtggggttttcttctaagccttctcctatttatgggggtttagtattgattgttagcggtgtggtcgggtgtgttattattctgaattttgggggaggttatatgggtttaatggtttttttaatttatttagggggaatgatggttgtctttggatatactacagcgatggctattgaggagtatcctgaggcatgggggtcaggggttgaggtcttggtgagtgttttagtggggttagcgatggaggtaggattggtgctgtgggtgaaagagtatgatggggtggtggttgtggtaaactttaatagtgtaggaagctggatgatttatgaaggagaggggtcagggttgattcgggaggatcctattggtgcgggggctttgtatgattatgggcgttggttagtagtagttactggttggacattgtttgttggtgtatatattgtaattgagattgctcgggggaattaggagcactgggacgcccaccgcccctttccctccgctgccaggcgagcatgttgtggtaattctggaacacaagaagagaaattgctgggtttagaacaagattataaacgaattcggtgctcagtgatcacttgacagttttttttttttttaaatattacccaaaatgctccccaaataagaaatgcatcagctcagtcagtgaatacaaaaaaggaattatttttccctttgagggtcttttatacatctctcctccaaccccaccctctattctgtttcttcctcctcacatgggggtacacatacacagcttcctcttttggttccatccttaccaccacaccacacgcacactccacatgcccagcagagtggcacttggtggccagaaagtgtgagcctcatgatctgctgtctgtagttctgtgagctcaggtccctcaaaggcctcggagcacccccttccttgtgactgagccagggcctgcatttttggttttccccaccccacacattctcaaccatagtccttctaacaataccaatagctaggacccggctgctgtgcactgggactggggattccacatgtttgccttgggagtctcaagctggactgcca

SEQ ID NO: 23 - DNA, 2034 bp, synthetic construct
  source 1..2034: mol_type = other DNA
atggccgcatctccgcacactctctcctcacgcctcctgacaggttgcgtaggaggctctgtctggtatcttgaaagaagaactatgatgtacgccctgttcctgctgagcgtgggcctggtgatgggcttcgtgggcttcagcagcaagcccagccccatctacggcggcctggtgctgatcgtgagcggcgtggtgggctgcgtgatcatcctgaacttcggcggcggctacatgggcctgatggtgttcctgatctacctgggcggcatgatggtggtgttcggctacaccaccgccatggccatcgaggagtaccccgaggcctggggcagcggcgtggaggtgctggtgagcgtgctggtgggcctggccatggaggtgggcctggtgctgtgggtgaaggagtacgacggcgtggtggtggtggtgaacttcaacagcgtgggcagctggatgatctacgagggcgagggcagcggcctgatccgcgaggaccccatcggcgccggcgccctgtacgactacggccgctggctggtggtggtgaccggctggaccctgttcgtgggcgtgtacatcgtgatcgagatcgcccgcggcaactaagagcactgggacgcccaccgcccctttccctccgctgccaggcgagcatgttgtggtaattctggaacacaagaagagaaattgctgggtttagaacaagattataaacgaattcggtgctcagtgatcacttgacagttttttttttttttaaatattacccaaaatgctccccaaataagaaatgcatcagctcagtcagtgaatacaaaaaaggaattatttttccctttgagggtcttttatacatctctcctccaaccccaccctctattctgtttcttcctcctcacatgggggtacacatacacagcttcctcttttggttccatccttaccaccacaccacacgcacactccacatgcccagcagagtggcacttggtggccagaaagtgtgagcctcatgatctgctgtctgtagttctgtgagctcaggtccctcaaaggcctcggagcacccccttccttgtgactgagccagggcctgcatttttggttttccccaccccacacattctcaaccatagtccttctaacaataccaatagctaggacccggctgctgtgcactgggactggggattccacatgtttgccttgggagtctcaagctggactgccagcccctgtcctcccttcacccccattgcgtatgagcatttcagaactccaaggagtcacaggcatctttatagttcacgttaacatatagacactgttggaagcagttccttctaaaagggtagccctggacttaataccagccggatacctctggcccccaccccattactgtacctctggagtcactactgtgggtcgccactcctctgctacacagcacggctttttcaaggctgtattgagaagggaagttaggaagaagggtgtgctgggctaaccagcccacagagctcacattcctgtcccttgggtgaaaaatacatgtccatcctgatatctcctgaattcagaaattagcctccacatgtgcaatggctttaagagccagaagcagggttctgggaattttgcaagttacctgtggccaggtgtggtctcggttaccaaatacggttacctgcagctttttagtcctttgtgctcccacgggtctacagagtcccatctgcccaaaggtcttgaagcttgacaggatgttttcgattactcagtctcccagggcactactggtccgtaggattcgattggtcggggtaggagagttaaacaacatttaaacagagttctctcaaaaatgtctaaagggattgtaggtagataacatccaatcactgtttgcacttatctgaaatcttccctcttggctgcccccaggtatttactgtggagaacattgcataggaatgtctggaaaaagcttctacaacttgttacagccttcacatttgtagaagcttt

SEQ ID NO: 24 - DNA, 1234 bp, synthetic construct
  source 1..1234: mol_type = other DNA
atggccgcatctccgcacactctctcctcacgcctcctgacaggttgcgtaggaggctctgtctggtatcttgaaagaagaactatgatgtacgccctgttcctgctgagcgtgggcctggtgatgggcttcgtgggcttcagcagcaagcccagccccatctacggcggcctggtgctgatcgtgagcggcgtggtgggctgcgtgatcatcctgaacttcggcggcggctacatgggcctgatggtgttcctgatctacctgggcggcatgatggtggtgttcggctacaccaccgccatggccatcgaggagtaccccgaggcctggggcagcggcgtggaggtgctggtgagcgtgctggtgggcctggccatggaggtgggcctggtgctgtgggtgaaggagtacgacggcgtggtggtggtggtgaacttcaacagcgtgggcagctggatgatctacgagggcgagggcagcggcctgatccgcgaggaccccatcggcgccggcgccctgtacgactacggccgctggctggtggtggtgaccggctggaccctgttcgtgggcgtgtacatcgtgatcgagatcgcccgcggcaactaagagcactgggacgcccaccgcccctttccctccgctgccaggcgagcatgttgtggtaattctggaacacaagaagagaaattgctgggtttagaacaagattataaacgaattcggtgctcagtgatcacttgacagttttttttttttttaaatattacccaaaatgctccccaaataagaaatgcatcagctcagtcagtgaatacaaaaaaggaattatttttccctttgagggtcttttatacatctctcctccaaccccaccctctattctgtttcttcctcctcacatgggggtacacatacacagcttcctcttttggttccatccttaccaccacaccacacgcacactccacatgcccagcagagtggcacttggtggccagaaagtgtgagcctcatgatctgctgtctgtagttctgtgagctcaggtccctcaaaggcctcggagcacccccttccttgtgactgagccagggcctgcatttttggttttccccaccccacacattctcaaccatagtccttctaacaataccaatagctaggacccggctgctgtgcactgggactggggattccacatgtttgccttgggagtctcaagctggactgcca

SEQ ID NO: 25 - DNA, 2460 bp, synthetic construct
  source 1..2460: mol_type = other DNA
atggccgcatctccgcacactctctcctcacgcctcctgacaggttgcgtaggaggctctgtctggtatcttgaaagaagaactatggccaacctcctactcctcattgtacccattctaatcgcaatggcattcctaatgcttaccgaacgaaaaattctaggctatatgcaactacgcaaaggccccaacgttgtaggcccctacgggctactacaacccttcgctgacgccataaaactcttcaccaaagagcccctaaaacccgccacatctaccatcaccctctacatcaccgccccgaccttagctctcaccatcgctcttctactatggacccccctccccatgcccaaccccctggtcaacctcaacctaggcctcctatttattctagccacctctagcctagccgtttactcaatcctctggtcagggtgggcatcaaactcaaactacgccctgatcggcgcactgcgagcagtagcccaaacaatctcatatgaagtcaccctagccatcattctactatcaacattactaatgagtggctcctttaacctctccacccttatcacaacacaagaacacctctggttactcctgccatcatggcccttggccatgatgtggtttatctccacactagcagagaccaaccgaacccccttcgaccttgccgaaggggagtccgaactagtctcaggcttcaacatcgaatacgccgcaggccccttcgccctattcttcatggccgaatacacaaacattattatgatgaacaccctcaccactacaatcttcctaggaacaacatatgacgcactctcccctgaactctacacaacatattttgtcaccaagaccctacttctaacctccctgttcttatggattcgaacagcatacccccgattccgctacgaccaactcatgcacctcctatggaaaaacttcctaccactcaccctagcattacttatgtggtatgtctccatgcccattacaatctccagcattccccctcaaacctaagagcactgggacgcccaccgcccctttccctccgctgccaggcgagcatgttgtggtaattctggaacacaagaagagaaattgctgggtttagaacaagattataaacgaattcggtgctcagtgatcacttgacagttttttttttttttaaatattacccaaaatgctccccaaataagaaatgcatcagctcagtcagtgaatacaaaaaaggaattatttttccctttgagggtcttttatacatctctcctccaaccccaccctctattctgtttcttcctcctcacatgggggtacacatacacagcttcctcttttggttccatccttaccaccacaccacacgcacactccacatgcccagcagagtggcacttggtggccagaaagtgtgagcctcatgatctgctgtctgtagttctgtgagctcaggtccctcaaaggcctcggagcacccccttccttgtgactgagccagggcctgcatttttggttttccccaccccacacattctcaaccatagtccttctaacaataccaatagctaggacccggctgctgtgcactgggactggggattccacatgtttgccttgggagtctcaagctggactgccagcccctgtcctcccttcacccccattgcgtatgagcatttcagaactccaaggagtcacaggcatctttatagttcacgttaacatatagacactgttggaagcagttccttctaaaagggtagccctggacttaataccagccggatacctctggcccccaccccattactgtacctctggagtcactactgtgggtcgccactcctctgctacacagcacggctttttcaaggctgtattgagaagggaagttaggaagaagggtgtgctgggctaaccagcccacagagctcacattcctgtcccttgggtgaaaaatacatgtccatcctgatatctcctgaattcagaaattagcctccacatgtgcaatggctttaagagccagaagcagggttctgggaattttgcaagttacctgtggccaggtgtggtctcggttaccaaatacggttacctgcagctttttagtcctttgtgctcccacgggtctacagagtcccatctgcccaaaggtcttgaagcttgacaggatgttttcgattactcagtctcccagggcactactggtccgtaggattcgattggtcggggtaggagagttaaacaacatttaaacagagttctctcaaaaatgtctaaagggattgtaggtagataacatccaatcactgtttgcacttatctgaaatcttccctcttggctgcccccaggtatttactgtggagaacattgcataggaatgtctggaaaaagcttctacaacttgttacagccttcacatttgtagaagcttt

SEQ ID NO: 26 - DNA, 1660 bp, synthetic construct
  source 1..1660: mol_type = other DNA
atggccgcatctccgcacactctctcctcacgcctcctgacaggttgcgtaggaggctctgtctggtatcttgaaagaagaactatggccaacctcctactcctcattgtacccattctaatcgcaatggcattcctaatgcttaccgaacgaaaaattctaggctatatgcaactacgcaaaggccccaacgttgtaggcccctacgggctactacaacccttcgctgacgccataaaactcttcaccaaagagcccctaaaacccgccacatctaccatcaccctctacatcaccgccccgaccttagctctcaccatcgctcttctactatggacccccctccccatgcccaaccccctggtcaacctcaacctaggcctcctatttattctagccacctctagcctagccgtttactcaatcctctggtcagggtgggcatcaaactcaaactacgccctgatcggcgcactgcgagcagtagcccaaacaatctcatatgaagtcaccctagccatcattctactatcaacattactaatgagtggctcctttaacctctccacccttatcacaacacaagaacacctctggttactcctgccatcatggcccttggccatgatgtggtttatctccacactagcagagaccaaccgaacccccttcgaccttgccgaaggggagtccgaactagtctcaggcttcaacatcgaatacgccgcaggccccttcgccctattcttcatggccgaatacacaaacattattatgatgaacaccctcaccactacaatcttcctaggaacaacatatgacgcactctcccctgaactctacacaacatattttgtcaccaagaccctacttctaacctccctgttcttatggattcgaacagcatacccccgattccgctacgaccaactcatgcacctcctatggaaaaacttcctaccactcaccctagcattacttatgtggtatgtctccatgcccattacaatctccagcattccccctcaaacctaagagcactgggacgcccaccgcccctttccctccgctgccaggcgagcatgttgtggtaattctggaacacaagaagagaaattgctgggtttagaacaagattataaacgaattcggtgctcagtgatcacttgacagttttttttttttttaaatattacccaaaatgctccccaaataagaaatgcatcagctcagtcagtgaatacaaaaaaggaattatttttccctttgagggtcttttatacatctctcctccaaccccaccctctattctgtttcttcctcctcacatgggggtacacatacacagcttcctcttttggttccatccttaccaccacaccacacgcacactccacatgcccagcagagtggcacttggtggccagaaagtgtgagcctcatgatctgctgtctgtagttctgtgagctcaggtccctcaaaggcctcggagcacccccttccttgtgactgagccagggcctgcatttttggttttccccaccccacacattctcaaccatagtccttctaacaataccaatagctaggacccggctgctgtgcactgggactggggattccacatgtttgccttgggagtctcaagctggactgcca

SEQ ID NO: 27 - DNA, 2460 bp, synthetic construct
  source 1..2460: mol_type = other DNA
atggccgcatctccgcacactctctcctcacgcctcctgacaggttgcgtaggaggctctgtctggtatcttgaaagaagaactatggccaacctgctgctgctgatcgtgcccatcctgatcgccatggccttcctgatgctgaccgagcgcaagatcctgggctacatgcagctgcgcaagggccccaacgtggtgggcccctacggcctgctgcagcccttcgccgacgccatcaagctgttcaccaaggagcccctgaagcccgccaccagcaccatcaccctgtacatcaccgcccccaccctggccctgaccatcgccctgctgctgtggacccccctgcccatgcccaaccccctggtgaacctgaacctgggcctgctgttcatcctggccaccagcagcctggccgtgtacagcatcctgtggagcggctgggccagcaacagcaactacgccctgatcggcgccctgcgcgccgtggcccagaccatcagctacgaggtgaccctggccatcatcctgctgagcaccctgctgatgagcggcagcttcaacctgagcaccctgatcaccacccaggagcacctgtggctgctgctgcccagctggcccctggccatgatgtggttcatcagcaccctggccgagaccaaccgcacccccttcgacctggccgagggcgagagcgagctggtgagcggcttcaacatcgagtacgccgccggccccttcgccctgttcttcatggccgagtacaccaacatcatcatgatgaacaccctgaccaccaccatcttcctgggcaccacctacgacgccctgagccccgagctgtacaccacctacttcgtgaccaagaccctgctgctgaccagcctgttcctgtggatccgcaccgcctacccccgcttccgctacgaccagctgatgcacctgctgtggaagaacttcctgcccctgaccctggccctgctgatgtggtacgtgagcatgcccatcaccatcagcagcatccccccccagacctaagagcactgggacgcccaccgcccctttccctccgctgccaggcgagcatgttgtggtaattctggaacacaagaagagaaattgctgggtttagaacaagattataaacgaattcggtgctcagtgatcacttgacagttttttttttttttaaatattacccaaaatgctccccaaataagaaatgcatcagctcagtcagtgaatacaaaaaaggaattatttttccctttgagggtcttttatacatctctcctccaaccccaccctctattctgtttcttcctcctcacatgggggtacacatacacagcttcctcttttggttccatccttaccaccacaccacacgcacactccacatgcccagcagagtggcacttggtggccagaaagtgtgagcctcatgatctgctgtctgtagttctgtgagctcaggtccctcaaaggcctcggagcacccccttccttgtgactgagccagggcctgcatttttggttttccccaccccacacattctcaaccatagtccttctaacaataccaatagctaggacccggctgctgtgcactgggactggggattccacatgtttgccttgggagtctcaagctggactgccagcccctgtcctcccttcacccccattgcgtatgagcatttcagaactccaaggagtcacaggcatctttatagttcacgttaacatatagacactgttggaagcagttccttctaaaagggtagccctggacttaataccagccggatacctctggcccccaccccattactgtacctctggagtcactactgtgggtcgccactcctctgctacacagcacggctttttcaaggctgtattgagaagggaagttaggaagaagggtgtgctgggctaaccagcccacagagctcacattcctgtcccttgggtgaaaaatacatgtccatcctgatatctcctgaattcagaaattagcctccacatgtgcaatggctttaagagccagaagcagggttctgggaattttgcaagttacctgtggccaggtgtggtctcggttaccaaatacggttacctgcagctttttagtcctttgtgctcccacgggtctacagagtcccatctgcccaaaggtcttgaagcttgacaggatgttttcgattactcagtctcccagggcactactggtccgtaggattcgattggtcggggtaggagagttaaacaacatttaaacagagttctctcaaaaatgtctaaagggattgtaggtagataacatccaatcactgtttgcacttatctgaaatcttccctcttggctgcccccaggtatttactgtggagaacattgcataggaatgtctggaaaaagcttctacaacttgttacagccttcacatttgtagaagcttt

SEQ ID NO: 28 - DNA, 1660 bp, synthetic construct
  source 1..1660: mol_type = other DNA
atggccgcatctccgcacactctctcctcacgcctcctgacaggttgcgtaggaggctctgtctggtatcttgaaagaagaactatggccaacctgctgctgctgatcgtgcccatcctgatcgccatggccttcctgatgctgaccgagcgcaagatcctgggctacatgcagctgcgcaagggccccaacgtggtgggcccctacggcctgctgcagcccttcgccgacgccatcaagctgttcaccaaggagcccctgaagcccgccaccagcaccatcaccctgtacatcaccgcccccaccctggccctgaccatcgccctgctgctgtggacccccctgcccatgcccaaccccctggtgaacctgaacctgggcctgctgttcatcctggccaccagcagcctggccgtgtacagcatcctgtggagcggctgggccagcaacagcaactacgccctgatcggcgccctgcgcgccgtggcccagaccatcagctacgaggtgaccctggccatcatcctgctgagcaccctgctgatgagcggcagcttcaacctgagcaccctgatcaccacccaggagcacctgtggctgctgctgcccagctggcccctggccatgatgtggttcatcagcaccctggccgagaccaaccgcacccccttcgacctggccgagggcgagagcgagctggtgagcggcttcaacatcgagtacgccgccggccccttcgccctgttcttcatggccgagtacaccaacatcatcatgatgaacaccctgaccaccaccatcttcctgggcaccacctacgacgccctgagccccgagctgtacaccacctacttcgtgaccaagaccctgctgctgaccagcctgttcctgtggatccgcaccgcctacccccgcttccgctacgaccagctgatgcacctgctgtggaagaacttcctgcccctgaccctggccctgctgatgtggtacgtgagcatgcccatcaccatcagcagcatccccccccagacctaagagcactgggacgcccaccgcccctttccctccgctgccaggcgagcatgttgtggtaattctggaacacaagaagagaaattgctgggtttagaacaagattataaacgaattcggtgctcagtgatcacttgacagttttttttttttttaaatattacccaaaatgctccccaaataagaaatgcatcagctcagtcagtgaatacaaaaaaggaattatttttccctttgagggtcttttatacatctctcctccaaccccaccctctattctgtttcttcctcctcacatgggggtacacatacacagcttcctcttttggttccatccttaccaccacaccacacgcacactccacatgcccagcagagtggcacttggtggccagaaagtgtgagcctcatgatctgctgtctgtagttctgtgagctcaggtccctcaaaggcctcggagcacccccttccttgtgactgagccagggcctgcatttttggttttccccaccccacacattctcaaccatagtccttctaacaataccaatagctaggacccggctgctgtgcactgggactggggattccacatgtttgccttgggagtctcaagctggactgcca

SEQ ID NO: 29 - DNA, 2889 bp, synthetic construct
  source 1..2889: mol_type = other DNA
atggccgcctctccacacacactgagtagcagactgctgaccggctgtgttggcggctctgtgtggtatctggaacggcggacaatgctaaaactaatcgtcccaacaattatgttactaccactgacatggctttccaaaaaacacatgatttggatcaacacaaccacccacagcctaattattagcatcatccctctactattttttaaccaaatcaacaacaacctatttagctgttccccaaccttttcctccgaccccctaacaacccccctcctaatgctaactacctggctcctacccctcacaatcatggcaagccaacgccacttatccagtgaaccactatcacgaaaaaaactctacctctctatgctaatctccctacaaatctccttaattatgacattcacagccacagaactaatcatgttttatatcttcttcgaaaccacacttatccccaccttggctatcatcacccgatggggcaaccagccagaacgcctgaacgcaggcacatacttcctattctacaccctagtaggctcccttcccctactcatcgcactaatttacactcacaacaccctaggctcactaaacattctactactcactctcactgcccaagaactatcaaactcctgggccaacaacttaatgtggctagcttacacaatggcttttatggtaaagatgcctctttacggactccacttatggctccctaaagcccatgtcgaagcccccatcgctgggtcaatggtacttgccgcagtactcttaaaactaggcggctatggtatgatgcgcctcacactcattctcaaccccctgacaaaacacatggcctaccccttccttgtactatccctatggggcatgattatgacaagctccatctgcctacgacaaacagacctaaaatcgctcattgcatactcttcaatcagccacatggccctcgtagtaacagccattctcatccaaaccccctggagcttcaccggcgcagtcattctcatgatcgcccacgggcttacatcctcattactattctgcctagcaaactcaaactacgaacgcactcacagtcgcatcatgatcctctctcaaggacttcaaactctactcccactaatggctttttggtggcttctagcaagcctcgctaacctcgccttaccccccactattaacctactgggagaactctctgtgctagtaaccacgttctcctggtcaaatatcactctcctacttacaggactcaacatgctagtcacagccctatactccctctacatgtttaccacaacacaatggggctcactcacccaccacattaacaacatgaaaccctcattcacacgagaaaacaccctcatgttcatgcacctatcccccattctcctcctatccctcaaccccgacatcattaccgggttttcctcttaagagcactgggacgcccaccgcccctttccctccgctgccaggcgagcatgttgtggtaattctggaacacaagaagagaaattgctgggtttagaacaagattataaacgaattcggtgctcagtgatcacttgacagttttttttttttttaaatattacccaaaatgctccccaaataagaaatgcatcagctcagtcagtgaatacaaaaaaggaattatttttccctttgagggtcttttatacatctctcctccaaccccaccctctattctgtttcttcctcctcacatgggggtacacatacacagcttcctcttttggttccatccttaccaccacaccacacgcacactccacatgcccagcagagtggcacttggtggccagaaagtgtgagcctcatgatctgctgtctgtagttctgtgagctcaggtccctcaaaggcctcggagcacccccttccttgtgactgagccagggcctgcatttttggttttccccaccccacacattctcaaccatagtccttctaacaataccaatagctaggacccggctgctgtgcactgggactggggattccacatgtttgccttgggagtctcaagctggactgccagcccctgtcctcccttcacccccattgcgtatgagcatttcagaactccaaggagtcacaggcatctttatagttcacgttaacatatagacactgttggaagcagttccttctaaaagggtagccctggacttaataccagccggatacctctggcccccaccccattactgtacctctggagtcactactgtgggtcgccactcctctgctacacagcacggctttttcaaggctgtattgagaagggaagttaggaagaagggtgtgctgggctaaccagcccacagagctcacattcctgtcccttgggtgaaaaatacatgtccatcctgatatctcctgaattcagaaattagcctccacatgtgcaatggctttaagagccagaagcagggttctgggaattttgcaagttacctgtggccaggtgtggtctcggttaccaaatacggttacctgcagctttttagtcctttgtgctcccacgggtctacagagtcccatctgcccaaaggtcttgaagcttgacaggatgttttcgattactcagtctcccagggcactactggtccgtaggattcgattggtcggggtaggagagttaaacaacatttaaacagagttctctcaaaaatgtctaaagggattgtaggtagataacatccaatcactgtttgcacttatctgaaatcttccctcttggctgcccccaggtatttactgtggagaacattgcataggaatgtctggaaaaagcttctacaacttgttacagccttcacatttgtagaagcttt

SEQ ID NO: 30 - DNA, 2089 bp, synthetic construct
  source 1..2089: mol_type = other DNA
atggccgcctctccacacacactgagtagcagactgctgaccggctgtgttggcggctctgtgtggtatctggaacggcggacaatgctaaaactaatcgtcccaacaattatgttactaccactgacatggctttccaaaaaacacatgatttggatcaacacaaccacccacagcctaattattagcatcatccctctactattttttaaccaaatcaacaacaacctatttagctgttccccaaccttttcctccgaccccctaacaacccccctcctaatgctaactacctggctcctacccctcacaatcatggcaagccaacgccacttatccagtgaaccactatcacgaaaaaaactctacctctctatgctaatctccctacaaatctccttaattatgacattcacagccacagaactaatcatgttttatatcttcttcgaaaccacacttatccccaccttggctatcatcacccgatggggcaaccagccagaacgcctgaacgcaggcacatacttcctattctacaccctagtaggctcccttcccctactcatcgcactaatttacactcacaacaccctaggctcactaaacattctactactcactctcactgcccaagaactatcaaactcctgggccaacaacttaatgtggctagcttacacaatggcttttatggtaaagatgcctctttacggactccacttatggctccctaaagcccatgtcgaagcccccatcgctgggtcaatggtacttgccgcagtactcttaaaactaggcggctatggtatgatgcgcctcacactcattctcaaccccctgacaaaacacatggcctaccccttccttgtactatccctatggggcatgattatgacaagctccatctgcctacgacaaacagacctaaaatcgctcattgcatactcttcaatcagccacatggccctcgtagtaacagccattctcatccaaaccccctggagcttcaccggcgcagtcattctcatgatcgcccacgggcttacatcctcattactattctgcctagcaaactcaaactacgaacgcactcacagtcgcatcatgatcctctctcaaggacttcaaactctactcccactaatggctttttggtggcttctagcaagcctcgctaacctcgccttaccccccactattaacctactgggagaactctctgtgctagtaaccacgttctcctggtcaaatatcactctcctacttacaggactcaacatgctagtcacagccctatactccctctacatgtttaccacaacacaatggggctcactcacccaccacattaacaacatgaaaccctcattcacacgagaaaacaccctcatgttcatgcacctatcccccattctcctcctatccctcaaccccgacatcattaccgggttttcctcttaagagcactgggacgcccaccgcccctttccctccgctgccaggcgagcatgttgtggtaattctggaacacaagaagagaaattgctgggtttagaacaagattataaacgaattcggtgctcagtgatcacttgacagttttttttttttttaaatattacccaaaatgctccccaaataagaaatgcatcagctcagtcagtgaatacaaaaaaggaattatttttccctttgagggtcttttatacatctctcctccaaccccaccctctattctgtttcttcctcctcacatgggggtacacatacacagcttcctcttttggttccatccttaccaccacaccacacgcacactccacatgcccagcagagtggcacttggtggccagaaagtgtgagcctcatgatctgctgtctgtagttctgtgagctcaggtccctcaaaggcctcggagcacccccttccttgtgactgagccagggcctgcatttttggttttccccaccccacacattctcaaccatagtccttctaacaataccaatagctaggacccggctgctgtgcactgggactggggattccacatgtttgccttgggagtctcaagctggactgcca

SEQ ID NO: 31 - DNA, 2889 bp, synthetic construct
  source 1..2889: mol_type = other DNA
atggccgcctctccacacacactgagtagcagactgctgaccggctgtgttggcggctctgtgtggtatctggaacggcggacaatgctgaagctgatcgtgcccaccatcatgctgctgcctctgacctggctgagcaagaaacacatgatctggatcaacaccaccacgcacagcctgatcatcagcatcatccctctgctgttcttcaaccagatcaacaacaacctgttcagctgcagccccaccttcagcagcgaccctctgacaacacctctgctgatgctgaccacctggctgctgcccctcacaatcatggcctctcagagacacctgagcagcgagcccctgagccggaagaaactgtacctgagcatgctgatctccctgcagatctctctgatcatgaccttcaccgccaccgagctgatcatgttctacatctttttcgagacaacgctgatccccacactggccatcatcaccagatggggcaaccagcctgagagactgaacgccggcacctactttctgttctacaccctcgtgggcagcctgccactgctgattgccctgatctacacccacaacaccctgggctccctgaacatcctgctgctgacactgacagcccaagagctgagcaacagctgggccaacaatctgatgtggctggcctacacaatggccttcatggtcaagatgcccctgtacggcctgcacctgtggctgcctaaagctcatgtggaagcccctatcgccggctctatggtgctggctgcagtgctgctgaaactcggcggctacggcatgatgcggctgaccctgattctgaatcccctgaccaagcacatggcctatccatttctggtgctgagcctgtggggcatgattatgaccagcagcatctgcctgcggcagaccgatctgaagtccctgatcgcctacagctccatcagccacatggccctggtggtcaccgccatcctgattcagaccccttggagctttacaggcgccgtgatcctgatgattgcccacggcctgacaagcagcctgctgttttgtctggccaacagcaactacgagcggacccacagcagaatcatgatcctgtctcagggcctgcagaccctcctgcctcttatggctttttggtggctgctggcctctctggccaatctggcactgcctcctaccatcaatctgctgggcgagctgagcgtgctggtcaccacattcagctggtccaatatcaccctgctgctcaccggcctgaacatgctggttacagccctgtactccctgtacatgttcaccaccacacagtggggaagcctgacacaccacatcaacaatatgaagcccagcttcacccgcgagaacaccctgatgttcatgcatctgagccccattctgctgctgtccctgaatcctgatatcatcaccggcttctccagctgagagcactgggacgcccaccgcccctttccctccgctgccaggcgagcatgttgtggtaattctggaacacaagaagagaaattgctgggtttagaacaagattataaacgaattcggtgctcagtgatcacttgacagttttttttttttttaaatattacccaaaatgctccccaaataagaaatgcatcagctcagtcagtgaatacaaaaaaggaattatttttccctttgagggtcttttatacatctctcctccaaccccaccctctattctgtttcttcctcctcacatgggggtacacatacacagcttcctcttttggttccatccttaccaccacaccacacgcacactccacatgcccagcagagtggcacttggtggccagaaagtgtgagcctcatgatctgctgtctgtagttctgtgagctcaggtccctcaaaggcctcggagcacccccttccttgtgactgagccagggcctgcatttttggttttccccaccccacacattctcaaccatagtccttctaacaataccaatagctaggacccggctgctgtgcactgggactggggattccacatgtttgccttgggagtctcaagctggactgccagcccctgtcctcccttcacccccattgcgtatgagcatttcagaactccaaggagtcacaggcatctttatagttcacgttaacatatagacactgttggaagcagttccttctaaaagggtagccctggacttaataccagccggatacctctggcccccaccccattactgtacctctggagtcactactgtgggtcgccactcctctgctacacagcacggctttttcaaggctgtattgagaagggaagttaggaagaagggtgtgctgggctaaccagcccacagagctcacattcctgtcccttgggtgaaaaatacatgtccatcctgatatctcctgaattcagaaattagcctccacatgtgcaatggctttaagagccagaagcagggttctgggaattttgcaagttacctgtggccaggtgtggtctcggttaccaaatacggttacctgcagctttttagtcctttgtgctcccacgggtctacagagtcccatctgcccaaaggtcttgaagcttgacaggatgttttcgattactcagtctcccagggcactactggtccgtaggattcgattggtcggggtaggagagttaaacaacatttaaacagagttctctcaaaaatgtctaaagggattgtaggtagataacatccaatcactgtttgcacttatctgaaatcttccctcttggctgcccccaggtatttactgtggagaacattgcataggaatgtctggaaaaagcttctacaacttgttacagccttcacatttgtagaagcttt

SEQ ID NO: 32 - DNA, 2089 bp, synthetic construct
  source 1..2089: mol_type = other DNA
atggccgcctctccacacacactgagtagcagactgctgaccggctgtgttggcggctctgtgtggtatctggaacggcggacaatgctgaagctgatcgtgcccaccatcatgctgctgcctctgacctggctgagcaagaaacacatgatctggatcaacaccaccacgcacagcctgatcatcagcatcatccctctgctgttcttcaaccagatcaacaacaacctgttcagctgcagccccaccttcagcagcgaccctctgacaacacctctgctgatgctgaccacctggctgctgcccctcacaatcatggcctctcagagacacctgagcagcgagcccctgagccggaagaaactgtacctgagcatgctgatctccctgcagatctctctgatcatgaccttcaccgccaccgagctgatcatgttctacatctttttcgagacaacgctgatccccacactggccatcatcaccagatggggcaaccagcctgagagactgaacgccggcacctactttctgttctacaccctcgtgggcagcctgccactgctgattgccctgatctacacccacaacaccctgggctccctgaacatcctgctgctgacactgacagcccaagagctgagcaacagctgggccaacaatctgatgtggctggcctacacaatggccttcatggtcaagatgcccctgtacggcctgcacctgtggctgcctaaagctcatgtggaagcccctatcgccggctctatggtgctggctgcagtgctgctgaaactcggcggctacggcatgatgcggctgaccctgattctgaatcccctgaccaagcacatggcctatccatttctggtgctgagcctgtggggcatgattatgaccagcagcatctgcctgcggcagaccgatctgaagtccctgatcgcctacagctccatcagccacatggccctggtggtcaccgccatcctgattcagaccccttggagctttacaggcgccgtgatcctgatgattgcccacggcctgacaagcagcctgctgttttgtctggccaacagcaactacgagcggacccacagcagaatcatgatcctgtctcagggcctgcagaccctcctgcctcttatggctttttggtggctgctggcctctctggccaatctggcactgcctcctaccatcaatctgctgggcgagctgagcgtgctggtcaccacattcagctggtccaatatcaccctgctgctcaccggcctgaacatgctggttacagccctgtactccctgtacatgttcaccaccacacagtggggaagcctgacacaccacatcaacaatatgaagcccagcttcacccgcgagaacaccctgatgttcatgcatctgagccccattctgctgctgtccctgaatcctgatatcatcaccggcttctccagctgagagcactgggacgcccaccgcccctttccctccgctgccaggcgagcatgttgtggtaattctggaacacaagaagagaaattgctgggtttagaacaagattataaacgaattcggtgctcagtgatcacttgacagttttttttttttttaaatattacccaaaatgctccccaaataagaaatgcatcagctcagtcagtgaatacaaaaaaggaattatttttccctttgagggtcttttatacatctctcctccaaccccaccctctattctgtttcttcctcctcacatgggggtacacatacacagcttcctcttttggttccatccttaccaccacaccacacgcacactccacatgcccagcagagtggcacttggtggccagaaagtgtgagcctcatgatctgctgtctgtagttctgtgagctcaggtccctcaaaggcctcggagcacccccttccttgtgactgagccagggcctgcatttttggttttccccaccccacacattctcaaccatagtccttctaacaataccaatagctaggacccggctgctgtgcactgggactggggattccacatgtttgccttgggagtctcaagctggactgcca

SEQ ID NO: 33 - DNA, 2889 bp, synthetic construct
  source 1..2889: mol_type = other DNA
atggccgcctctccacacacactgagtagcagactgctgaccggctgtgttggcggctctgtgtggtatctggaacggcggacaatgctgaagctgatcgtgcccaccatcatgctgctgcccctgacctggctgagcaagaagcacatgatctggatcaacaccaccacccacagcctgatcatcagcatcatccccctgctgttcttcaaccagatcaacaacaacctgttcagctgcagccccaccttcagcagcgaccccctgaccacccccctgctgatgctgaccacctggctgctgcccctgaccatcatggccagccagcgccacctgagcagcgagcccctgagccgcaagaagctgtacctgagcatgctgatcagcctgcagatcagcctgatcatgaccttcaccgccaccgagctgatcatgttctacatcttcttcgagaccaccctgatccccaccctggccatcatcacccgctggggcaaccagcccgagcgcctgaacgccggcacctacttcctgttctacaccctggtgggcagcctgcccctgctgatcgccctgatctacacccacaacaccctgggcagcctgaacatcctgctgctgaccctgaccgcccaggagctgagcaacagctgggccaacaacctgatgtggctggcctacaccatggccttcatggtgaagatgcccctgtacggcctgcacctgtggctgcccaaggcccacgtggaggcccccatcgccggcagcatggtgctggccgccgtgctgctgaagctgggcggctacggcatgatgcgcctgaccctgatcctgaaccccctgaccaagcacatggcctaccccttcctggtgctgagcctgtggggcatgatcatgaccagcagcatctgcctgcgccagaccgacctgaagagcctgatcgcctacagcagcatcagccacatggccctggtggtgaccgccatcctgatccagaccccctggagcttcaccggcgccgtgatcctgatgatcgcccacggcctgaccagcagcctgctgttctgcctggccaacagcaactacgagcgcacccacagccgcatcatgatcctgagccagggcctgcagaccctgctgcccctgatggccttctggtggctgctggccagcctggccaacctggccctgccccccaccatcaacctgctgggcgagctgagcgtgctggtgaccaccttcagctggagcaacatcaccctgctgctgaccggcctgaacatgctggtgaccgccctgtacagcctgtacatgttcaccaccacccagtggggcagcctgacccaccacatcaacaacatgaagcccagcttcacccgcgagaacaccctgatgttcatgcacctgagccccatcctgctgctgagcctgaaccccgacatcatcaccggcttcagcagctaagagcactgggacgcccaccgcccctttccctccgctgccaggcgagcatgttgtggtaattctggaacacaagaagagaaattgctgggtttagaacaagattataaacgaattcggtgctcagtgatcacttgacagttttttttttttttaaatattacccaaaatgctccccaaataagaaatgcatcagctcagtcagtgaatacaaaaaaggaattatttttccctttgagggtcttttatacatctctcctccaaccccaccctctattctgtttcttcctcctcacatgggggtacacatacacagcttcctcttttggttccatccttaccaccacaccacacgcacactccacatgcccagcagagtggcacttggtggccagaaagtgtgagcctcatgatctgctgtctgtagttctgtgagctcaggtccctcaaaggcctcggagcacccccttccttgtgactgagccagggcctgcatttttggttttccccaccccacacattctcaaccatagtccttctaacaataccaatagctaggacccggctgctgtgcactgggactggggattccacatgtttgccttgggagtctcaagctggactgccagcccctgtcctcccttcacccccattgcgtatgagcatttcagaactccaaggagtcacaggcatctttatagttcacgttaacatatagacactgttggaagcagttccttctaaaagggtagccctggacttaataccagccggatacctctggcccccaccccattactgtacctctggagtcactactgtgggtcgccactcctctgctacacagcacggctttttcaaggctgtattgagaagggaagttaggaagaagggtgtgctgggctaaccagcccacagagctcacattcctgtcccttgggtgaaaaatacatgtccatcctgatatctcctgaattcagaaattagcctccacatgtgcaatggctttaagagccagaagcagggttctgggaattttgcaagttacctgtggccaggtgtggtctcggttaccaaatacggttacctgcagctttttagtcctttgtgctcccacgggtctacagagtcccatctgcccaaaggtcttgaagcttgacaggatgttttcgattactcagtctcccagggcactactggtccgtaggattcgattggtcggggtaggagagttaaacaacatttaaacagagttctctcaaaaatgtctaaagggattgtaggtagataacatccaatcactgtttgcacttatctgaaatcttccctcttggctgcccccaggtatttactgtggagaacattgcataggaatgtctggaaaaagcttctacaacttgttacagccttcacatttgtagaagcttt

SEQ ID NO: 34 - DNA, 2089 bp, synthetic construct
  source 1..2089: mol_type = other DNA
atggccgcctctccacacacactgagtagcagactgctgaccggctgtgttggcggctctgtgtggtatctggaacggcggacaatgctgaagctgatcgtgcccaccatcatgctgctgcccctgacctggctgagcaagaagcacatgatctggatcaacaccaccacccacagcctgatcatcagcatcatccccctgctgttcttcaaccagatcaacaacaacctgttcagctgcagccccaccttcagcagcgaccccctgaccacccccctgctgatgctgaccacctggctgctgcccctgaccatcatggccagccagcgccacctgagcagcgagcccctgagccgcaagaagctgtacctgagcatgctgatcagcctgcagatcagcctgatcatgaccttcaccgccaccgagctgatcatgttctacatcttcttcgagaccaccctgatccccaccctggccatcatcacccgctggggcaaccagcccgagcgcctgaacgccggcacctacttcctgttctacaccctggtgggcagcctgcccctgctgatcgccctgatctacacccacaacaccctgggcagcctgaacatcctgctgctgaccctgaccgcccaggagctgagcaacagctgggccaacaacctgatgtggctggcctacaccatggccttcatggtgaagatgcccctgtacggcctgcacctgtggctgcccaaggcccacgtggaggcccccatcgccggcagcatggtgctggccgccgtgctgctgaagctgggcggctacggcatgatgcgcctgaccctgatcctgaaccccctgaccaagcacatggcctaccccttcctggtgctgagcctgtggggcatgatcatgaccagcagcatctgcctgcgccagaccgacctgaagagcctgatcgcctacagcagcatcagccacatggccctggtggtgaccgccatcctgatccagaccccctggagcttcaccggcgccgtgatcctgatgatcgcccacggcctgaccagcagcctgctgttctgcctggccaacagcaactacgagcgcacccacagccgcatcatgatcctgagccagggcctgcagaccctgctgcccctgatggccttctggtggctgctggccagcctggccaacctggccctgccccccaccatcaacctgctgggcgagctgagcgtgctggtgaccaccttcagctggagcaacatcaccctgctgctgaccggcctgaacatgctggtgaccgccctgtacagcctgtacatgttcaccaccacccagtggggcagcctgacccaccacatcaacaacatgaagcccagcttcacccgcgagaacaccctgatgttcatgcacctgagccccatcctgctgctgagcctgaaccccgacatcatcaccggcttcagcagctaagagcactgggacgcccaccgcccctttccctccgctgccaggcgagcatgttgtggtaattctggaacacaagaagagaaattgctgggtttagaacaagattataaacgaattcggtgctcagtgatcacttgacagttttttttttttttaaatattacccaaaatgctccccaaataagaaatgcatcagctcagtcagtgaatacaaaaaaggaattatttttccctttgagggtcttttatacatctctcctccaaccccaccctctattctgtttcttcctcctcacatgggggtacacatacacagcttcctcttttggttccatccttaccaccacaccacacgcacactccacatgcccagcagagtggcacttggtggccagaaagtgtgagcctcatgatctgctgtctgtagttctgtgagctcaggtccctcaaaggcctcggagcacccccttccttgtgactgagccagggcctgcatttttggttttccccaccccacacattctcaaccatagtccttctaacaataccaatagctaggacccggctgctgtgcactgggactggggattccacatgtttgccttgggagtctcaagctggactgcca

SEQ ID NO: 35 - DNA, 2034 bp, synthetic construct
  source 1..2034: mol_type = other DNA
atggccgcctctccacacacactgagtagcagactgctgaccggctgtgttggcggctctgtgtggtatctggaacggcggacaatgatgtatgctttgtttctgttgagtgtgggtttagtaatggggtttgtggggttttcttctaagccttctcctatttatgggggtttagtattgattgttagcggtgtggtcgggtgtgttattattctgaattttgggggaggttatatgggtttaatggtttttttaatttatttagggggaatgatggttgtctttggatatactacagcgatggctattgaggagtatcctgaggcatgggggtcaggggttgaggtcttggtgagtgttttagtggggttagcgatggaggtaggattggtgctgtgggtgaaagagtatgatggggtggtggttgtggtaaactttaatagtgtaggaagctggatgatttatgaaggagaggggtcagggttgattcgggaggatcctattggtgcgggggctttgtatgattatgggcgttggttagtagtagttactggttggacattgtttgttggtgtatatattgtaattgagattgctcgggggaattaggagcactgggacgcccaccgcccctttccctccgctgccaggcgagcatgttgtggtaattctggaacacaagaagagaaattgctgggtttagaacaagattataaacgaattcggtgctcagtgatcacttgacagttttttttttttttaaatattacccaaaatgctccccaaataagaaatgcatcagctcagtcagtgaatacaaaaaaggaattatttttccctttgagggtcttttatacatctctcctccaaccccaccctctattctgtttcttcctcctcacatgggggtacacatacacagcttcctcttttggttccatccttaccaccacaccacacgcacactccacatgcccagcagagtggcacttggtggccagaaagtgtgagcctcatgatctgctgtctgtagttctgtgagctcaggtccctcaaaggcctcggagcacccccttccttgtgactgagccagggcctgcatttttggttttccccaccccacacattctcaaccatagtccttctaacaataccaatagctaggacccggctgctgtgcactgggactggggattccacatgtttgccttgggagtctcaagctggactgccagcccctgtcctcccttcacccccattgcgtatgagcatttcagaactccaaggagtcacaggcatctttatagttcacgttaacatatagacactgttggaagcagttccttctaaaagggtagccctggacttaataccagccggatacctctggcccccaccccattactgtacctctggagtcactactgtgggtcgccactcctctgctacacagcacggctttttcaaggctgtattgagaagggaagttaggaagaagggtgtgctgggctaaccagcccacagagctcacattcctgtcccttgggtgaaaaatacatgtccatcctgatatctcctgaattcagaaattagcctccacatgtgcaatggctttaagagccagaagcagggttctgggaattttgcaagttacctgtggccaggtgtggtctcggttaccaaatacggttacctgcagctttttagtcctttgtgctcccacgggtctacagagtcccatctgcccaaaggtcttgaagcttgacaggatgttttcgattactcagtctcccagggcactactggtccgtaggattcgattggtcggggtaggagagttaaacaacatttaaacagagttctctcaaaaatgtctaaagggattgtaggtagataacatccaatcactgtttgcacttatctgaaatcttccctcttggctgcccccaggtatttactgtggagaacattgcataggaatgtctggaaaaagcttctacaacttgttacagccttcacatttgtagaagcttt

SEQ ID NO: 36 - DNA, 1234 bp, synthetic construct
  source 1..1234: mol_type = other DNA
atggccgcctctccacacacactgagtagcagactgctgaccggctgtgttggcggctctgtgtggtatctggaacggcggacaatgatgtatgctttgtttctgttgagtgtgggtttagtaatggggtttgtggggttttcttctaagccttctcctatttatgggggtttagtattgattgttagcggtgtggtcgggtgtgttattattctgaattttgggggaggttatatgggtttaatggtttttttaatttatttagggggaatgatggttgtctttggatatactacagcgatggctattgaggagtatcctgaggcatgggggtcaggggttgaggtcttggtgagtgttttagtggggttagcgatggaggtaggattggtgctgtgggtgaaagagtatgatggggtggtggttgtggtaaactttaatagtgtaggaagctggatgatttatgaaggagaggggtcagggttgattcgggaggatcctattggtgcgggggctttgtatgattatgggcgttggttagtagtagttactggttggacattgtttgttggtgtatatattgtaattgagattgctcgggggaattaggagcactgggacgcccaccgcccctttccctccgctgccaggcgagcatgttgtggtaattctggaacacaagaagagaaattgctgggtttagaacaagattataaacgaattcggtgctcagtgatcacttgacagttttttttttttttaaatattacccaaaatgctccccaaataagaaatgcatcagctcagtcagtgaatacaaaaaaggaattatttttccctttgagggtcttttatacatctctcctccaaccccaccctctattctgtttcttcctcctcacatgggggtacacatacacagcttcctcttttggttccatccttaccaccacaccacacgcacactccacatgcccagcagagtggcacttggtggccagaaagtgtgagcctcatgatctgctgtctgtagttctgtgagctcaggtccctcaaaggcctcggagcacccccttccttgtgactgagccagggcctgcatttttggttttccccaccccacacattctcaaccatagtccttctaacaataccaatagctaggacccggctgctgtgcactgggactggggattccacatgtttgccttgggagtctcaagctggactgcca

SEQ ID NO: 37 - DNA, 2034 bp, synthetic construct
  source 1..2034: mol_type = other DNA
atggccgcctctccacacacactgagtagcagactgctgaccggctgtgttggcggctctgtgtggtatctggaacggcggacaatgatgtacgccctgttcctgctgagcgtgggcctggtgatgggcttcgtgggcttcagcagcaagcccagccccatctacggcggcctggtgctgatcgtgagcggcgtggtgggctgcgtgatcatcctgaacttcggcggcggctacatgggcctgatggtgttcctgatctacctgggcggcatgatggtggtgttcggctacaccaccgccatggccatcgaggagtaccccgaggcctggggcagcggcgtggaggtgctggtgagcgtgctggtgggcctggccatggaggtgggcctggtgctgtgggtgaaggagtacgacggcgtggtggtggtggtgaacttcaacagcgtgggcagctggatgatctacgagggcgagggcagcggcctgatccgcgaggaccccatcggcgccggcgccctgtacgactacggccgctggctggtggtggtgaccggctggaccctgttcgtgggcgtgtacatcgtgatcgagatcgcccgcggcaactaagagcactgggacgcccaccgcccctttccctccgctgccaggcgagcatgttgtggtaattctggaacacaagaagagaaattgctgggtttagaacaagattataaacgaattcggtgctcagtgatcacttgacagttttttttttttttaaatattacccaaaatgctccccaaataagaaatgcatcagctcagtcagtgaatacaaaaaaggaattatttttccctttgagggtcttttatacatctctcctccaaccccaccctctattctgtttcttcctcctcacatgggggtacacatacacagcttcctcttttggttccatccttaccaccacaccacacgcacactccacatgcccagcagagtggcacttggtggccagaaagtgtgagcctcatgatctgctgtctgtagttctgtgagctcaggtccctcaaaggcctcggagcacccccttccttgtgactgagccagggcctgcatttttggttttccccaccccacacattctcaaccatagtccttctaacaataccaatagctaggacccggctgctgtgcactgggactggggattccacatgtttgccttgggagtctcaagctggactgccagcccctgtcctcccttcacccccattgcgtatgagcatttcagaactccaaggagtcacaggcatctttatagttcacgttaacatatagacactgttggaagcagttccttctaaaagggtagccctggacttaataccagccggatacctctggcccccaccccattactgtacctctggagtcactactgtgggtcgccactcctctgctacacagcacggctttttcaaggctgtattgagaagggaagttaggaagaagggtgtgctgggctaaccagcccacagagctcacattcctgtcccttgggtgaaaaatacatgtccatcctgatatctcctgaattcagaaattagcctccacatgtgcaatggctttaagagccagaagcagggttctgggaattttgcaagttacctgtggccaggtgtggtctcggttaccaaatacggttacctgcagctttttagtcctttgtgctcccacgggtctacagagtcccatctgcccaaaggtcttgaagcttgacaggatgttttcgattactcagtctcccagggcactactggtccgtaggattcgattggtcggggtaggagagttaaacaacatttaaacagagttctctcaaaaatgtctaaagggattgtaggtagataacatccaatcactgtttgcacttatctgaaatcttccctcttggctgcccccaggtatttactgtggagaacattgcataggaatgtctggaaaaagcttctacaacttgttacagccttcacatttgtagaagcttt

SEQ ID NO: 38 - DNA, 1234 bp, synthetic construct
  source 1..1234: mol_type = other DNA
atggccgcctctccacacacactgagtagcagactgctgaccggctgtgttggcggctctgtgtggtatctggaacggcggacaatgatgtacgccctgttcctgctgagcgtgggcctggtgatgggcttcgtgggcttcagcagcaagcccagccccatctacggcggcctggtgctgatcgtgagcggcgtggtgggctgcgtgatcatcctgaacttcggcggcggctacatgggcctgatggtgttcctgatctacctgggcggcatgatggtggtgttcggctacaccaccgccatggccatcgaggagtaccccgaggcctggggcagcggcgtggaggtgctggtgagcgtgctggtgggcctggccatggaggtgggcctggtgctgtgggtgaaggagtacgacggcgtggtggtggtggtgaacttcaacagcgtgggcagctggatgatctacgagggcgagggcagcggcctgatccgcgaggaccccatcggcgccggcgccctgtacgactacggccgctggctggtggtggtgaccggctggaccctgttcgtgggcgtgtacatcgtgatcgagatcgcccgcggcaactaagagcactgggacgcccaccgcccctttccctccgctgccaggcgagcatgttgtggtaattctggaacacaagaagagaaattgctgggtttagaacaagattataaacgaattcggtgctcagtgatcacttgacagttttttttttttttaaatattacccaaaatgctccccaaataagaaatgcatcagctcagtcagtgaatacaaaaaaggaattatttttccctttgagggtcttttatacatctctcctccaaccccaccctctattctgtttcttcctcctcacatgggggtacacatacacagcttcctcttttggttccatccttaccaccacaccacacgcacactccacatgcccagcagagtggcacttggtggccagaaagtgtgagcctcatgatctgctgtctgtagttctgtgagctcaggtccctcaaaggcctcggagcacccccttccttgtgactgagccagggcctgcatttttggttttccccaccccacacattctcaaccatagtccttctaacaataccaatagctaggacccggctgctgtgcactgggactggggattccacatgtttgccttgggagtctcaagctggactgcca

SEQ ID NO: 39 - DNA, 2460 bp, synthetic construct
  source 1..2460: mol_type = other DNA
atggccgcctctccacacacactgagtagcagactgctgaccggctgtgttggcggctctgtgtggtatctggaacggcggacaatggccaacctcctactcctcattgtacccattctaatcgcaatggcattcctaatgcttaccgaacgaaaaattctaggctatatgcaactacgcaaaggccccaacgttgtaggcccctacgggctactacaacccttcgctgacgccataaaactcttcaccaaagagcccctaaaacccgccacatctaccatcaccctctacatcaccgccccgaccttagctctcaccatcgctcttctactatggacccccctccccatgcccaaccccctggtcaacctcaacctaggcctcctatttattctagccacctctagcctagccgtttactcaatcctctggtcagggtgggcatcaaactcaaactacgccctgatcggcgcactgcgagcagtagcccaaacaatctcatatgaagtcaccctagccatcattctactatcaacattactaatgagtggctcctttaacctctccacccttatcacaacacaagaacacctctggttactcctgccatcatggcccttggccatgatgtggtttatctccacactagcagagaccaaccgaacccccttcgaccttgccgaaggggagtccgaactagtctcaggcttcaacatcgaatacgccgcaggccccttcgccctattcttcatggccgaatacacaaacattattatgatgaacaccctcaccactacaatcttcctaggaacaacatatgacgcactctcccctgaactctacacaacatattttgtcaccaagaccctacttctaacctccctgttcttatggattcgaacagcatacccccgattccgctacgaccaactcatgcacctcctatggaaaaacttcctaccactcaccctagcattacttatgtggtatgtctccatgcccattacaatctccagcattccccctcaaacctaagagcactgggacgcccaccgcccctttccctccgctgccaggcgagcatgttgtggtaattctggaacacaagaagagaaattgctgggtttagaacaagattataaacgaattcggtgctcagtgatcacttgacagttttttttttttttaaatattacccaaaatgctccccaaataagaaatgcatcagctcagtcagtgaatacaaaaaaggaattatttttccctttgagggtcttttatacatctctcctccaaccccaccctctattctgtttcttcctcctcacatgggggtacacatacacagcttcctcttttggttccatccttaccaccacaccacacgcacactccacatgcccagcagagtggcacttggtggccagaaagtgtgagcctcatgatctgctgtctgtagttctgtgagctcaggtccctcaaaggcctcggagcacccccttccttgtgactgagccagggcctgcatttttggttttccccaccccacacattctcaaccatagtccttctaacaataccaatagctaggacccggctgctgtgcactgggactggggattccacatgtttgccttgggagtctcaagctggactgccagcccctgtcctcccttcacccccattgcgtatgagcatttcagaactccaaggagtcacaggcatctttatagttcacgttaacatatagacactgttggaagcagttccttctaaaagggtagccctggacttaataccagccggatacctctggcccccaccccattactgtacctctggagtcactactgtgggtcgccactcctctgctacacagcacggctttttcaaggctgtattgagaagggaagttaggaagaagggtgtgctgggctaaccagcccacagagctcacattcctgtcccttgggtgaaaaatacatgtccatcctgatatctcctgaattcagaaattagcctccacatgtgcaatggctttaagagccagaagcagggttctgggaattttgcaagttacctgtggccaggtgtggtctcggttaccaaatacggttacctgcagctttttagtcctttgtgctcccacgggtctacagagtcccatctgcccaaaggtcttgaagcttgacaggatgttttcgattactcagtctcccagggcactactggtccgtaggattcgattggtcggggtaggagagttaaacaacatttaaacagagttctctcaaaaatgtctaaagggattgtaggtagataacatccaatcactgtttgcacttatctgaaatcttccctcttggctgcccccaggtatttactgtggagaacattgcataggaatgtctggaaaaagcttctacaacttgttacagccttcacatttgtagaagcttt

SEQ ID NO: 40 - DNA, 1660 bp, synthetic construct
  source 1..1660: mol_type = other DNA
atggccgcctctccacacacactgagtagcagactgctgaccggctgtgttggcggctctgtgtggtatctggaacggcggacaatggccaacctcctactcctcattgtacccattctaatcgcaatggcattcctaatgcttaccgaacgaaaaattctaggctatatgcaactacgcaaaggccccaacgttgtaggcccctacgggctactacaacccttcgctgacgccataaaactcttcaccaaagagcccctaaaacccgccacatctaccatcaccctctacatcaccgccccgaccttagctctcaccatcgctcttctactatggacccccctccccatgcccaaccccctggtcaacctcaacctaggcctcctatttattctagccacctctagcctagccgtttactcaatcctctggtcagggtgggcatcaaactcaaactacgccctgatcggcgcactgcgagcagtagcccaaacaatctcatatgaagtcaccctagccatcattctactatcaacattactaatgagtggctcctttaacctctccacccttatcacaacacaagaacacctctggttactcctgccatcatggcccttggccatgatgtggtttatctccacactagcagagaccaaccgaacccccttcgaccttgccgaaggggagtccgaactagtctcaggcttcaacatcgaatacgccgcaggccccttcgccctattcttcatggccgaatacacaaacattattatgatgaacaccctcaccactacaatcttcctaggaacaacatatgacgcactctcccctgaactctacacaacatattttgtcaccaagaccctacttctaacctccctgttcttatggattcgaacagcatacccccgattccgctacgaccaactcatgcacctcctatggaaaaacttcctaccactcaccctagcattacttatgtggtatgtctccatgcccattacaatctccagcattccccctcaaacctaagagcactgggacgcccaccgcccctttccctccgctgccaggcgagcatgttgtggtaattctggaacacaagaagagaaattgctgggtttagaacaagattataaacgaattcggtgctcagtgatcacttgacagttttttttttttttaaatattacccaaaatgctccccaaataagaaatgcatcagctcagtcagtgaatacaaaaaaggaattatttttccctttgagggtcttttatacatctctcctccaaccccaccctctattctgtttcttcctcctcacatgggggtacacatacacagcttcctcttttggttccatccttaccaccacaccacacgcacactccacatgcccagcagagtggcacttggtggccagaaagtgtgagcctcatgatctgctgtctgtagttctgtgagctcaggtccctcaaaggcctcggagcacccccttccttgtgactgagccagggcctgcatttttggttttccccaccccacacattctcaaccatagtccttctaacaataccaatagctaggacccggctgctgtgcactgggactggggattccacatgtttgccttgggagtctcaagctggactgcca

SEQ ID NO: 41 - DNA, 2460 bp, synthetic construct
  source 1..2460: mol_type = other DNA
atggccgcctctccacacacactgagtagcagactgctgaccggctgtgttggcggctctgtgtggtatctggaacggcggacaatggccaacctgctgctgctgatcgtgcccatcctgatcgccatggccttcctgatgctgaccgagcgcaagatcctgggctacatgcagctgcgcaagggccccaacgtggtgggcccctacggcctgctgcagcccttcgccgacgccatcaagctgttcaccaaggagcccctgaagcccgccaccagcaccatcaccctgtacatcaccgcccccaccctggccctgaccatcgccctgctgctgtggacccccctgcccatgcccaaccccctggtgaacctgaacctgggcctgctgttcatcctggccaccagcagcctggccgtgtacagcatcctgtggagcggctgggccagcaacagcaactacgccctgatcggcgccctgcgcgccgtggcccagaccatcagctacgaggtgaccctggccatcatcctgctgagcaccctgctgatgagcggcagcttcaacctgagcaccctgatcaccacccaggagcacctgtggctgctgctgcccagctggcccctggccatgatgtggttcatcagcaccctggccgagaccaaccgcacccccttcgacctggccgagggcgagagcgagctggtgagcggcttcaacatcgagtacgccgccggccccttcgccctgttcttcatggccgagtacaccaacatcatcatgatgaacaccctgaccaccaccatcttcctgggcaccacctacgacgccctgagccccgagctgtacaccacctacttcgtgaccaagaccctgctgctgaccagcctgttcctgtggatccgcaccgcctacccccgcttccgctacgaccagctgatgcacctgctgtggaagaacttcctgcccctgaccctggccctgctgatgtggtacgtgagcatgcccatcaccatcagcagcatccccccccagacctaagagcactgggacgcccaccgcccctttccctccgctgccaggcgagcatgttgtggtaattctggaacacaagaagagaaattgctgggtttagaacaagattataaacgaattcggtgctcagtgatcacttgacagttttttttttttttaaatattacccaaaatgctccccaaataagaaatgcatcagctcagtcagtgaatacaaaaaaggaattatttttccctttgagggtcttttatacatctctcctccaaccccaccctctattctgtttcttcctcctcacatgggggtacacatacacagcttcctcttttggttccatccttaccaccacaccacacgcacactccacatgcccagcagagtggcacttggtggccagaaagtgtgagcctcatgatctgctgtctgtagttctgtgagctcaggtccctcaaaggcctcggagcacccccttccttgtgactgagccagggcctgcatttttggttttccccaccccacacattctcaaccatagtccttctaacaataccaatagctaggacccggctgctgtgcactgggactggggattccacatgtttgccttgggagtctcaagctggactgccagcccctgtcctcccttcacccccattgcgtatgagcatttcagaactccaaggagtcacaggcatctttatagttcacgttaacatatagacactgttggaagcagttccttctaaaagggtagccctggacttaataccagccggatacctctggcccccaccccattactgtacctctggagtcactactgtgggtcgccactcctctgctacacagcacggctttttcaaggctgtattgagaagggaagttaggaagaagggtgtgctgggctaaccagcccacagagctcacattcctgtcccttgggtgaaaaatacatgtccatcctgatatctcctgaattcagaaattagcctccacatgtgcaatggctttaagagccagaagcagggttctgggaattttgcaagttacctgtggccaggtgtggtctcggttaccaaatacggttacctgcagctttttagtcctttgtgctcccacgggtctacagagtcccatctgcccaaaggtcttgaagcttgacaggatgttttcgattactcagtctcccagggcactactggtccgtaggattcgattggtcggggtaggagagttaaacaacatttaaacagagttctctcaaaaatgtctaaagggattgtaggtagataacatccaatcactgtttgcacttatctgaaatcttccctcttggctgcccccaggtatttactgtggagaacattgcataggaatgtctggaaaaagcttctacaacttgttacagccttcacatttgtagaagcttt

SEQ ID NO: 42 - DNA, 1660 bp, synthetic construct
  source 1..1660: mol_type = other DNA
atggccgcctctccacacacactgagtagcagactgctgaccggctgtgttggcggctctgtgtggtatctggaacggcggacaatggccaacctgctgctgctgatcgtgcccatcctgatcgccatggccttcctgatgctgaccgagcgcaagatcctgggctacatgcagctgcgcaagggccccaacgtggtgggcccctacggcctgctgcagcccttcgccgacgccatcaagctgttcaccaaggagcccctgaagcccgccaccagcaccatcaccctgtacatcaccgcccccaccctggccctgaccatcgccctgctgctgtggacccccctgcccatgcccaaccccctggtgaacctgaacctgggcctgctgttcatcctggccaccagcagcctggccgtgtacagcatcctgtggagcggctgggccagcaacagcaactacgccctgatcggcgccctgcgcgccgtggcccagaccatcagctacgaggtgaccctggccatcatcctgctgagcaccctgctgatgagcggcagcttcaacctgagcaccctgatcaccacccaggagcacctgtggctgctgctgcccagctggcccctggccatgatgtggttcatcagcaccctggccgagaccaaccgcacccccttcgacctggccgagggcgagagcgagctggtgagcggcttcaacatcgagtacgccgccggccccttcgccctgttcttcatggccgagtacaccaacatcatcatgatgaacaccctgaccaccaccatcttcctgggcaccacctacgacgccctgagccccgagctgtacaccacctacttcgtgaccaagaccctgctgctgaccagcctgttcctgtggatccgcaccgcctacccccgcttccgctacgaccagctgatgcacctgctgtggaagaacttcctgcccctgaccctggccctgctgatgtggtacgtgagcatgcccatcaccatcagcagcatccccccccagacctaagagcactgggacgcccaccgcccctttccctccgctgccaggcgagcatgttgtggtaattctggaacacaagaagagaaattgctgggtttagaacaagattataaacgaattcggtgctcagtgatcacttgacagttttttttttttttaaatattacccaaaatgctccccaaataagaaatgcatcagctcagtcagtgaatacaaaaaaggaattatttttccctttgagggtcttttatacatctctcctccaaccccaccctctattctgtttcttcctcctcacatgggggtacacatacacagcttcctcttttggttccatccttaccaccacaccacacgcacactccacatgcccagcagagtggcacttggtggccagaaagtgtgagcctcatgatctgctgtctgtagttctgtgagctcaggtccctcaaaggcctcggagcacccccttccttgtgactgagccagggcctgcatttttggttttccccaccccacacattctcaaccatagtccttctaacaataccaatagctaggacccggctgctgtgcactgggactggggattccacatgtttgccttgggagtctcaagctggactgcca

SEQ ID NO: 43 - DNA, 2889 bp, synthetic construct
  source 1..2889: mol_type = other DNA
atggccgccagcccccacaccctgagcagccgcctgctgaccggctgcgtgggcggcagcgtgtggtacctggagcgccgcaccatgctaaaactaatcgtcccaacaattatgttactaccactgacatggctttccaaaaaacacatgatttggatcaacacaaccacccacagcctaattattagcatcatccctctactattttttaaccaaatcaacaacaacctatttagctgttccccaaccttttcctccgaccccctaacaacccccctcctaatgctaactacctggctcctacccctcacaatcatggcaagccaacgccacttatccagtgaaccactatcacgaaaaaaactctacctctctatgctaatctccctacaaatctccttaattatgacattcacagccacagaactaatcatgttttatatcttcttcgaaaccacacttatccccaccttggctatcatcacccgatggggcaaccagccagaacgcctgaacgcaggcacatacttcctattctacaccctagtaggctcccttcccctactcatcgcactaatttacactcacaacaccctaggctcactaaacattctactactcactctcactgcccaagaactatcaaactcctgggccaacaacttaatgtggctagcttacacaatggcttttatggtaaagatgcctctttacggactccacttatggctccctaaagcccatgtcgaagcccccatcgctgggtcaatggtacttgccgcagtactcttaaaactaggcggctatggtatgatgcgcctcacactcattctcaaccccctgacaaaacacatggcctaccccttccttgtactatccctatggggcatgattatgacaagctccatctgcctacgacaaacagacctaaaatcgctcattgcatactcttcaatcagccacatggccctcgtagtaacagccattctcatccaaaccccctggagcttcaccggcgcagtcattctcatgatcgcccacgggcttacatcctcattactattctgcctagcaaactcaaactacgaacgcactcacagtcgcatcatgatcctctctcaaggacttcaaactctactcccactaatggctttttggtggcttctagcaagcctcgctaacctcgccttaccccccactattaacctactgggagaactctctgtgctagtaaccacgttctcctggtcaaatatcactctcctacttacaggactcaacatgctagtcacagccctatactccctctacatgtttaccacaacacaatggggctcactcacccaccacattaacaacatgaaaccctcattcacacgagaaaacaccctcatgttcatgcacctatcccccattctcctcctatccctcaaccccgacatcattaccgggttttcctcttaagagcactgggacgcccaccgcccctttccctccgctgccaggcgagcatgttgtggtaattctggaacacaagaagagaaattgctgggtttagaacaagattataaacgaattcggtgctcagtgatcacttgacagttttttttttttttaaatattacccaaaatgctccccaaataagaaatgcatcagctcagtcagtgaatacaaaaaaggaattatttttccctttgagggtcttttatacatctctcctccaaccccaccctctattctgtttcttcctcctcacatgggggtacacatacacagcttcctcttttggttccatccttaccaccacaccacacgcacactccacatgcccagcagagtggcacttggtggccagaaagtgtgagcctcatgatctgctgtctgtagttctgtgagctcaggtccctcaaaggcctcggagcacccccttccttgtgactgagccagggcctgcatttttggttttccccaccccacacattctcaaccatagtccttctaacaataccaatagctaggacccggctgctgtgcactgggactggggattccacatgtttgccttgggagtctcaagctggactgccagcccctgtcctcccttcacccccattgcgtatgagcatttcagaactccaaggagtcacaggcatctttatagttcacgttaacatatagacactgttggaagcagttccttctaaaagggtagccctggacttaataccagccggatacctctggcccccaccccattactgtacctctggagtcactactgtgggtcgccactcctctgctacacagcacggctttttcaaggctgtattgagaagggaagttaggaagaagggtgtgctgggctaaccagcccacagagctcacattcctgtcccttgggtgaaaaatacatgtccatcctgatatctcctgaattcagaaattagcctccacatgtgcaatggctttaagagccagaagcagggttctgggaattttgcaagttacctgtggccaggtgtggtctcggttaccaaatacggttacctgcagctttttagtcctttgtgctcccacgggtctacagagtcccatctgcccaaaggtcttgaagcttgacaggatgttttcgattactcagtctcccagggcactactggtccgtaggattcgattggtcggggtaggagagttaaacaacatttaaacagagttctctcaaaaatgtctaaagggattgtaggtagataacatccaatcactgtttgcacttatctgaaatcttccctcttggctgcccccaggtatttactgtggagaacattgcataggaatgtctggaaaaagcttctacaacttgttacagccttcacatttgtagaagcttt

SEQ ID NO: 44 - DNA, 2089 bp, synthetic construct
  source 1..2089: mol_type = other DNA
atggccgccagcccccacaccctgagcagccgcctgctgaccggctgcgtgggcggcagcgtgtggtacctggagcgccgcaccatgctaaaactaatcgtcccaacaattatgttactaccactgacatggctttccaaaaaacacatgatttggatcaacacaaccacccacagcctaattattagcatcatccctctactattttttaaccaaatcaacaacaacctatttagctgttccccaaccttttcctccgaccccctaacaacccccctcctaatgctaactacctggctcctacccctcacaatcatggcaagccaacgccacttatccagtgaaccactatcacgaaaaaaactctacctctctatgctaatctccctacaaatctccttaattatgacattcacagccacagaactaatcatgttttatatcttcttcgaaaccacacttatccccaccttggctatcatcacccgatggggcaaccagccagaacgcctgaacgcaggcacatacttcctattctacaccctagtaggctcccttcccctactcatcgcactaatttacactcacaacaccctaggctcactaaacattctactactcactctcactgcccaagaactatcaaactcctgggccaacaacttaatgtggctagcttacacaatggcttttatggtaaagatgcctctttacggactccacttatggctccctaaagcccatgtcgaagcccccatcgctgggtcaatggtacttgccgcagtactcttaaaactaggcggctatggtatgatgcgcctcacactcattctcaaccccctgacaaaacacatggcctaccccttccttgtactatccctatggggcatgattatgacaagctccatctgcctacgacaaacagacctaaaatcgctcattgcatactcttcaatcagccacatggccctcgtagtaacagccattctcatccaaaccccctggagcttcaccggcgcagtcattctcatgatcgcccacgggcttacatcctcattactattctgcctagcaaactcaaactacgaacgcactcacagtcgcatcatgatcctctctcaaggacttcaaactctactcccactaatggctttttggtggcttctagcaagcctcgctaacctcgccttaccccccactattaacctactgggagaactctctgtgctagtaaccacgttctcctggtcaaatatcactctcctacttacaggactcaacatgctagtcacagccctatactccctctacatgtttaccacaacacaatggggctcactcacccaccacattaacaacatgaaaccctcattcacacgagaaaacaccctcatgttcatgcacctatcccccattctcctcctatccctcaaccccgacatcattaccgggttttcctcttaagagcactgggacgcccaccgcccctttccctccgctgccaggcgagcatgttgtggtaattctggaacacaagaagagaaattgctgggtttagaacaagattataaacgaattcggtgctcagtgatcacttgacagttttttttttttttaaatattacccaaaatgctccccaaataagaaatgcatcagctcagtcagtgaatacaaaaaaggaattatttttccctttgagggtcttttatacatctctcctccaaccccaccctctattctgtttcttcctcctcacatgggggtacacatacacagcttcctcttttggttccatccttaccaccacaccacacgcacactccacatgcccagcagagtggcacttggtggccagaaagtgtgagcctcatgatctgctgtctgtagttctgtgagctcaggtccctcaaaggcctcggagcacccccttccttgtgactgagccagggcctgcatttttggttttccccaccccacacattctcaaccatagtccttctaacaataccaatagctaggacccggctgctgtgcactgggactggggattccacatgtttgccttgggagtctcaagctggactgcca

SEQ ID NO: 45 - DNA, 2889 bp, synthetic construct
  source 1..2889: mol_type = other DNA
atggccgccagcccccacaccctgagcagccgcctgctgaccggctgcgtgggcggcagcgtgtggtacctggagcgccgcaccatgctgaagctgatcgtgcccaccatcatgctgctgcctctgacctggctgagcaagaaacacatgatctggatcaacaccaccacgcacagcctgatcatcagcatcatccctctgctgttcttcaaccagatcaacaacaacctgttcagctgcagccccaccttcagcagcgaccctctgacaacacctctgctgatgctgaccacctggctgctgcccctcacaatcatggcctctcagagacacctgagcagcgagcccctgagccggaagaaactgtacctgagcatgctgatctccctgcagatctctctgatcatgaccttcaccgccaccgagctgatcatgttctacatctttttcgagacaacgctgatccccacactggccatcatcaccagatggggcaaccagcctgagagactgaacgccggcacctactttctgttctacaccctcgtgggcagcctgccactgctgattgccctgatctacacccacaacaccctgggctccctgaacatcctgctgctgacactgacagcccaagagctgagcaacagctgggccaacaatctgatgtggctggcctacacaatggccttcatggtcaagatgcccctgtacggcctgcacctgtggctgcctaaagctcatgtggaagcccctatcgccggctctatggtgctggctgcagtgctgctgaaactcggcggctacggcatgatgcggctgaccctgattctgaatcccctgaccaagcacatggcctatccatttctggtgctgagcctgtggggcatgattatgaccagcagcatctgcctgcggcagaccgatctgaagtccctgatcgcctacagctccatcagccacatggccctggtggtcaccgccatcctgattcagaccccttggagctttacaggcgccgtgatcctgatgattgcccacggcctgacaagcagcctgctgttttgtctggccaacagcaactacgagcggacccacagcagaatcatgatcctgtctcagggcctgcagaccctcctgcctcttatggctttttggtggctgctggcctctctggccaatctggcactgcctcctaccatcaatctgctgggcgagctgagcgtgctggtcaccacattcagctggtccaatatcaccctgctgctcaccggcctgaacatgctggttacagccctgtactccctgtacatgttcaccaccacacagtggggaagcctgacacaccacatcaacaatatgaagcccagcttcacccgcgagaacaccctgatgttcatgcatctgagccccattctgctgctgtccctgaatcctgatatcatcaccggcttctccagctgagagcactgggacgcccaccgcccctttccctccgctgccaggcgagcatgttgtggtaattctggaacacaagaagagaaattgctgggtttagaacaagattataaacgaattcggtgctcagtgatcacttgacagttttttttttttttaaatattacccaaaatgctccccaaataagaaatgcatcagctcagtcagtgaatacaaaaaaggaattatttttccctttgagggtcttttatacatctctcctccaaccccaccctctattctgtttcttcctcctcacatgggggtacacatacacagcttcctcttttggttccatccttaccaccacaccacacgcacactccacatgcccagcagagtggcacttggtggccagaaagtgtgagcctcatgatctgctgtctgtagttctgtgagctcaggtccctcaaaggcctcggagcacccccttccttgtgactgagccagggcctgcatttttggttttccccaccccacacattctcaaccatagtccttctaacaataccaatagctaggacccggctgctgtgcactgggactggggattccacatgtttgccttgggagtctcaagctggactgccagcccctgtcctcccttcacccccattgcgtatgagcatttcagaactccaaggagtcacaggcatctttatagttcacgttaacatatagacactgttggaagcagttccttctaaaagggtagccctggacttaataccagccggatacctctggcccccaccccattactgtacctctggagtcactactgtgggtcgccactcctctgctacacagcacggctttttcaaggctgtattgagaagggaagttaggaagaagggtgtgctgggctaaccagcccacagagctcacattcctgtcccttgggtgaaaaatacatgtccatcctgatatctcctgaattcagaaattagcctccacatgtgcaatggctttaagagccagaagcagggttctgggaattttgcaagttacctgtggccaggtgtggtctcggttaccaaatacggttacctgcagctttttagtcctttgtgctcccacgggtctacagagtcccatctgcccaaaggtcttgaagcttgacaggatgttttcgattactcagtctcccagggcactactggtccgtaggattcgattggtcggggtaggagagttaaacaacatttaaacagagttctctcaaaaatgtctaaagggattgtaggtagataacatccaatcactgtttgcacttatctgaaatcttccctcttggctgcccccaggtatttactgtggagaacattgcataggaatgtctggaaaaagcttctacaacttgttacagccttcacatttgtagaagcttt

SEQ ID NO: 46 - DNA, 2089 bp, synthetic construct
  source 1..2089: mol_type = other DNA
atggccgccagcccccacaccctgagcagccgcctgctgaccggctgcgtgggcggcagcgtgtggtacctggagcgccgcaccatgctgaagctgatcgtgcccaccatcatgctgctgcctctgacctggctgagcaagaaacacatgatctggatcaacaccaccacgcacagcctgatcatcagcatcatccctctgctgttcttcaaccagatcaacaacaacctgttcagctgcagccccaccttcagcagcgaccctctgacaacacctctgctgatgctgaccacctggctgctgcccctcacaatcatggcctctcagagacacctgagcagcgagcccctgagccggaagaaactgtacctgagcatgctgatctccctgcagatctctctgatcatgaccttcaccgccaccgagctgatcatgttctacatctttttcgagacaacgctgatccccacactggccatcatcaccagatggggcaaccagcctgagagactgaacgccggcacctactttctgttctacaccctcgtgggcagcctgccactgctgattgccctgatctacacccacaacaccctgggctccctgaacatcctgctgctgacactgacagcccaagagctgagcaacagctgggccaacaatctgatgtggctggcctacacaatggccttcatggtcaagatgcccctgtacggcctgcacctgtggctgcctaaagctcatgtggaagcccctatcgccggctctatggtgctggctgcagtgctgctgaaactcggcggctacggcatgatgcggctgaccctgattctgaatcccctgaccaagcacatggcctatccatttctggtgctgagcctgtggggcatgattatgaccagcagcatctgcctgcggcagaccgatctgaagtccctgatcgcctacagctccatcagccacatggccctggtggtcaccgccatcctgattcagaccccttggagctttacaggcgccgtgatcctgatgattgcccacggcctgacaagcagcctgctgttttgtctggccaacagcaactacgagcggacccacagcagaatcatgatcctgtctcagggcctgcagaccctcctgcctcttatggctttttggtggctgctggcctctctggccaatctggcactgcctcctaccatcaatctgctgggcgagctgagcgtgctggtcaccacattcagctggtccaatatcaccctgctgctcaccggcctgaacatgctggttacagccctgtactccctgtacatgttcaccaccacacagtggggaagcctgacacaccacatcaacaatatgaagcccagcttcacccgcgagaacaccctgatgttcatgcatctgagccccattctgctgctgtccctgaatcctgatatcatcaccggcttctccagctgagagcactgggacgcccaccgcccctttccctccgctgccaggcgagcatgttgtggtaattctggaacacaagaagagaaattgctgggtttagaacaagattataaacgaattcggtgctcagtgatcacttgacagttttttttttttttaaatattacccaaaatgctccccaaataagaaatgcatcagctcagtcagtgaatacaaaaaaggaattatttttccctttgagggtcttttatacatctctcctccaaccccaccctctattctgtttcttcctcctcacatgggggtacacatacacagcttcctcttttggttccatccttaccaccacaccacacgcacactccacatgcccagcagagtggcacttggtggccagaaagtgtgagcctcatgatctgctgtctgtagttctgtgagctcaggtccctcaaaggcctcggagcacccccttccttgtgactgagccagggcctgcatttttggttttccccaccccacacattctcaaccatagtccttctaacaataccaatagctaggacccggctgctgtgcactgggactggggattccacatgtttgccttgggagtctcaagctggactgcca

SEQ ID NO: 47 - DNA, 2889 bp, synthetic construct
  source 1..2889: mol_type = other DNA
atggccgccagcccccacaccctgagcagccgcctgctgaccggctgcgtgggcggcagcgtgtggtacctggagcgccgcaccatgctgaagctgatcgtgcccaccatcatgctgctgcccctgacctggctgagcaagaagcacatgatctggatcaacaccaccacccacagcctgatcatcagcatcatccccctgctgttcttcaaccagatcaacaacaacctgttcagctgcagccccaccttcagcagcgaccccctgaccacccccctgctgatgctgaccacctggctgctgcccctgaccatcatggccagccagcgccacctgagcagcgagcccctgagccgcaagaagctgtacctgagcatgctgatcagcctgcagatcagcctgatcatgaccttcaccgccaccgagctgatcatgttctacatcttcttcgagaccaccctgatccccaccctggccatcatcacccgctggggcaaccagcccgagcgcctgaacgccggcacctacttcctgttctacaccctggtgggcagcctgcccctgctgatcgccctgatctacacccacaacaccctgggcagcctgaacatcctgctgctgaccctgaccgcccaggagctgagcaacagctgggccaacaacctgatgtggctggcctacaccatggccttcatggtgaagatgcccctgtacggcctgcacctgtggctgcccaaggcccacgtggaggcccccatcgccggcagcatggtgctggccgccgtgctgctgaagctgggcggctacggcatgatgcgcctgaccctgatcctgaaccccctgaccaagcacatggcctaccccttcctggtgctgagcctgtggggcatgatcatgaccagcagcatctgcctgcgccagaccgacctgaagagcctgatcgcctacagcagcatcagccacatggccctggtggtgaccgccatcctgatccagaccccctggagcttcaccggcgccgtgatcctgatgatcgcccacggcctgaccagcagcctgctgttctgcctggccaacagcaactacgagcgcacccacagccgcatcatgatcctgagccagggcctgcagaccctgctgcccctgatggccttctggtggctgctggccagcctggccaacctggccctgccccccaccatcaacctgctgggcgagctgagcgtgctggtgaccaccttcagctggagcaacatcaccctgctgctgaccggcctgaacatgctggtgaccgccctgtacagcctgtacatgttcaccaccacccagtggggcagcctgacccaccacatcaacaacatgaagcccagcttcacccgcgagaacaccctgatgttcatgcacctgagccccatcctgctgctgagcctgaaccccgacatcatcaccggcttcagcagctaagagcactgggacgcccaccgcccctttccctccgctgccaggcgagcatgttgtggtaattctggaacacaagaagagaaattgctgggtttagaacaagattataaacgaattcggtgctcagtgatcacttgacagttttttttttttttaaatattacccaaaatgctccccaaataagaaatgcatcagctcagtcagtgaatacaaaaaaggaattatttttccctttgagggtcttttatacatctctcctccaaccccaccctctattctgtttcttcctcctcacatgggggtacacatacacagcttcctcttttggttccatccttaccaccacaccacacgcacactccacatgcccagcagagtggcacttggtggccagaaagtgtgagcctcatgatctgctgtctgtagttctgtgagctcaggtccctcaaaggcctcggagcacccccttccttgtgactgagccagggcctgcatttttggttttccccaccccacacattctcaaccatagtccttctaacaataccaatagctaggacccggctgctgtgcactgggactggggattccacatgtttgccttgggagtctcaagctggactgccagcccctgtcctcccttcacccccattgcgtatgagcatttcagaactccaaggagtcacaggcatctttatagttcacgttaacatatagacactgttggaagcagttccttctaaaagggtagccctggacttaataccagccggatacctctggcccccaccccattactgtacctctggagtcactactgtgggtcgccactcctctgctacacagcacggctttttcaaggctgtattgagaagggaagttaggaagaagggtgtgctgggctaaccagcccacagagctcacattcctgtcccttgggtgaaaaatacatgtccatcctgatatctcctgaattcagaaattagcctccacatgtgcaatggctttaagagccagaagcagggttctgggaattttgcaagttacctgtggccaggtgtggtctcggttaccaaatacggttacctgcagctttttagtcctttgtgctcccacgggtctacagagtcccatctgcccaaaggtcttgaagcttgacaggatgttttcgattactcagtctcccagggcactactggtccgtaggattcgattggtcggggtaggagagttaaacaacatttaaacagagttctctcaaaaatgtctaaagggattgtaggtagataacatccaatcactgtttgcacttatctgaaatcttccctcttggctgcccccaggtatttactgtggagaacattgcataggaatgtctggaaaaagcttctacaacttgttacagccttcacatttgtagaagcttt

SEQ ID NO: 48 - DNA, 2089 bp, synthetic construct
  source 1..2089: mol_type = other DNA
atggccgccagcccccacaccctgagcagccgcctgctgaccggctgcgtgggcggcagcgtgtggtacctggagcgccgcaccatgctgaagctgatcgtgcccaccatcatgctgctgcccctgacctggctgagcaagaagcacatgatctggatcaacaccaccacccacagcctgatcatcagcatcatccccctgctgttcttcaaccagatcaacaacaacctgttcagctgcagccccaccttcagcagcgaccccctgaccacccccctgctgatgctgaccacctggctgctgcccctgaccatcatggccagccagcgccacctgagcagcgagcccctgagccgcaagaagctgtacctgagcatgctgatcagcctgcagatcagcctgatcatgaccttcaccgccaccgagctgatcatgttctacatcttcttcgagaccaccctgatccccaccctggccatcatcacccgctggggcaaccagcccgagcgcctgaacgccggcacctacttcctgttctacaccctggtgggcagcctgcccctgctgatcgccctgatctacacccacaacaccctgggcagcctgaacatcctgctgctgaccctgaccgcccaggagctgagcaacagctgggccaacaacctgatgtggctggcctacaccatggccttcatggtgaagatgcccctgtacggcctgcacctgtggctgcccaaggcccacgtggaggcccccatcgccggcagcatggtgctggccgccgtgctgctgaagctgggcggctacggcatgatgcgcctgaccctgatcctgaaccccctgaccaagcacatggcctaccccttcctggtgctgagcctgtggggcatgatcatgaccagcagcatctgcctgcgccagaccgacctgaagagcctgatcgcctacagcagcatcagccacatggccctggtggtgaccgccatcctgatccagaccccctggagcttcaccggcgccgtgatcctgatgatcgcccacggcctgaccagcagcctgctgttctgcctggccaacagcaactacgagcgcacccacagccgcatcatgatcctgagccagggcctgcagaccctgctgcccctgatggccttctggtggctgctggccagcctggccaacctggccctgccccccaccatcaacctgctgggcgagctgagcgtgctggtgaccaccttcagctggagcaacatcaccctgctgctgaccggcctgaacatgctggtgaccgccctgtacagcctgtacatgttcaccaccacccagtggggcagcctgacccaccacatcaacaacatgaagcccagcttcacccgcgagaacaccctgatgttcatgcacctgagccccatcctgctgctgagcctgaaccccgacatcatcaccggcttcagcagctaagagcactgggacgcccaccgcccctttccctccgctgccaggcgagcatgttgtggtaattctggaacacaagaagagaaattgctgggtttagaacaagattataaacgaattcggtgctcagtgatcacttgacagttttttttttttttaaatattacccaaaatgctccccaaataagaaatgcatcagctcagtcagtgaatacaaaaaaggaattatttttccctttgagggtcttttatacatctctcctccaaccccaccctctattctgtttcttcctcctcacatgggggtacacatacacagcttcctcttttggttccatccttaccaccacaccacacgcacactccacatgcccagcagagtggcacttggtggccagaaagtgtgagcctcatgatctgctgtctgtagttctgtgagctcaggtccctcaaaggcctcggagcacccccttccttgtgactgagccagggcctgcatttttggttttccccaccccacacattctcaaccatagtccttctaacaataccaatagctaggacccggctgctgtgcactgggactggggattccacatgtttgccttgggagtctcaagctggactgcca

SEQ ID NO: 49 - DNA, 2034 bp, synthetic construct
  source 1..2034: mol_type = other DNA
atggccgccagcccccacaccctgagcagccgcctgctgaccggctgcgtgggcggcagcgtgtggtacctggagcgccgcaccatgatgtatgctttgtttctgttgagtgtgggtttagtaatggggtttgtggggttttcttctaagccttctcctatttatgggggtttagtattgattgttagcggtgtggtcgggtgtgttattattctgaattttgggggaggttatatgggtttaatggtttttttaatttatttagggggaatgatggttgtctttggatatactacagcgatggctattgaggagtatcctgaggcatgggggtcaggggttgaggtcttggtgagtgttttagtggggttagcgatggaggtaggattggtgctgtgggtgaaagagtatgatggggtggtggttgtggtaaactttaatagtgtaggaagctggatgatttatgaaggagaggggtcagggttgattcgggaggatcctattggtgcgggggctttgtatgattatgggcgttggttagtagtagttactggttggacattgtttgttggtgtatatattgtaattgagattgctcgggggaattaggagcactgggacgcccaccgcccctttccctccgctgccaggcgagcatgttgtggtaattctggaacacaagaagagaaattgctgggtttagaacaagattataaacgaattcggtgctcagtgatcacttgacagttttttttttttttaaatattacccaaaatgctccccaaataagaaatgcatcagctcagtcagtgaatacaaaaaaggaattatttttccctttgagggtcttttatacatctctcctccaaccccaccctctattctgtttcttcctcctcacatgggggtacacatacacagcttcctcttttggttccatccttaccaccacaccacacgcacactccacatgcccagcagagtggcacttggtggccagaaagtgtgagcctcatgatctgctgtctgtagttctgtgagctcaggtccctcaaaggcctcggagcacccccttccttgtgactgagccagggcctgcatttttggttttccccaccccacacattctcaaccatagtccttctaacaataccaatagctaggacccggctgctgtgcactgggactggggattccacatgtttgccttgggagtctcaagctggactgccagcccctgtcctcccttcacccccattgcgtatgagcatttcagaactccaaggagtcacaggcatctttatagttcacgttaacatatagacactgttggaagcagttccttctaaaagggtagccctggacttaataccagccggatacctctggcccccaccccattactgtacctctggagtcactactgtgggtcgccactcctctgctacacagcacggctttttcaaggctgtattgagaagggaagttaggaagaagggtgtgctgggctaaccagcccacagagctcacattcctgtcccttgggtgaaaaatacatgtccatcctgatatctcctgaattcagaaattagcctccacatgtgcaatggctttaagagccagaagcagggttctgggaattttgcaagttacctgtggccaggtgtggtctcggttaccaaatacggttacctgcagctttttagtcctttgtgctcccacgggtctacagagtcccatctgcccaaaggtcttgaagcttgacaggatgttttcgattactcagtctcccagggcactactggtccgtaggattcgattggtcggggtaggagagttaaacaacatttaaacagagttctctcaaaaatgtctaaagggattgtaggtagataacatccaatcactgtttgcacttatctgaaatcttccctcttggctgcccccaggtatttactgtggagaacattgcataggaatgtctggaaaaagcttctacaacttgttacagccttcacatttgtagaagcttt

SEQ ID NO: 50 - DNA, 1234 bp, synthetic construct
  source 1..1234: mol_type = other DNA
atggccgccagcccccacaccctgagcagccgcctgctgaccggctgcgtgggcggcagcgtgtggtacctggagcgccgcaccatgatgtatgctttgtttctgttgagtgtgggtttagtaatggggtttgtggggttttcttctaagccttctcctatttatgggggtttagtattgattgttagcggtgtggtcgggtgtgttattattctgaattttgggggaggttatatgggtttaatggtttttttaatttatttagggggaatgatggttgtctttggatatactacagcgatggctattgaggagtatcctgaggcatgggggtcaggggttgaggtcttggtgagtgttttagtggggttagcgatggaggtaggattggtgctgtgggtgaaagagtatgatggggtggtggttgtggtaaactttaatagtgtaggaagctggatgatttatgaaggagaggggtcagggttgattcgggaggatcctattggtgcgggggctttgtatgattatgggcgttggttagtagtagttactggttggacattgtttgttggtgtatatattgtaattgagattgctcgggggaattaggagcactgggacgcccaccgcccctttccctccgctgccaggcgagcatgttgtggtaattctggaacacaagaagagaaattgctgggtttagaacaagattataaacgaattcggtgctcagtgatcacttgacagttttttttttttttaaatattacccaaaatgctccccaaataagaaatgcatcagctcagtcagtgaatacaaaaaaggaattatttttccctttgagggtcttttatacatctctcctccaaccccaccctctattctgtttcttcctcctcacatgggggtacacatacacagcttcctcttttggttccatccttaccaccacaccacacgcacactccacatgcccagcagagtggcacttggtggccagaaagtgtgagcctcatgatctgctgtctgtagttctgtgagctcaggtccctcaaaggcctcggagcacccccttccttgtgactgagccagggcctgcatttttggttttccccaccccacacattctcaaccatagtccttctaacaataccaatagctaggacccggctgctgtgcactgggactggggattccacatgtttgccttgggagtctcaagctggactgcca

SEQ ID NO: 51 - DNA, 2034 bp, synthetic construct
  source 1..2034: mol_type = other DNA
atggccgccagcccccacaccctgagcagccgcctgctgaccggctgcgtgggcggcagcgtgtggtacctggagcgccgcaccatgatgtacgccctgttcctgctgagcgtgggcctggtgatgggcttcgtgggcttcagcagcaagcccagccccatctacggcggcctggtgctgatcgtgagcggcgtggtgggctgcgtgatcatcctgaacttcggcggcggctacatgggcctgatggtgttcctgatctacctgggcggcatgatggtggtgttcggctacaccaccgccatggccatcgaggagtaccccgaggcctggggcagcggcgtggaggtgctggtgagcgtgctggtgggcctggccatggaggtgggcctggtgctgtgggtgaaggagtacgacggcgtggtggtggtggtgaacttcaacagcgtgggcagctggatgatctacgagggcgagggcagcggcctgatccgcgaggaccccatcggcgccggcgccctgtacgactacggccgctggctggtggtggtgaccggctggaccctgttcgtgggcgtgtacatcgtgatcgagatcgcccgcggcaactaagagcactgggacgcccaccgcccctttccctccgctgccaggcgagcatgttgtggtaattctggaacacaagaagagaaattgctgggtttagaacaagattataaacgaattcggtgctcagtgatcacttgacagttttttttttttttaaatattacccaaaatgctccccaaataagaaatgcatcagctcagtcagtgaatacaaaaaaggaattatttttccctttgagggtcttttatacatctctcctccaaccccaccctctattctgtttcttcctcctcacatgggggtacacatacacagcttcctcttttggttccatccttaccaccacaccacacgcacactccacatgcccagcagagtggcacttggtggccagaaagtgtgagcctcatgatctgctgtctgtagttctgtgagctcaggtccctcaaaggcctcggagcacccccttccttgtgactgagccagggcctgcatttttggttttccccaccccacacattctcaaccatagtccttctaacaataccaatagctaggacccggctgctgtgcactgggactggggattccacatgtttgccttgggagtctcaagctggactgccagcccctgtcctcccttcacccccattgcgtatgagcatttcagaactccaaggagtcacaggcatctttatagttcacgttaacatatagacactgttggaagcagttccttctaaaagggtagccctggacttaataccagccggatacctctggcccccaccccattactgtacctctggagtcactactgtgggtcgccactcctctgctacacagcacggctttttcaaggctgtattgagaagggaagttaggaagaagggtgtgctgggctaaccagcccacagagctcacattcctgtcccttgggtgaaaaatacatgtccatcctgatatctcctgaattcagaaattagcctccacatgtgcaatggctttaagagccagaagcagggttctgggaattttgcaagttacctgtggccaggtgtggtctcggttaccaaatacggttacctgcagctttttagtcctttgtgctcccacgggtctacagagtcccatctgcccaaaggtcttgaagcttgacaggatgttttcgattactcagtctcccagggcactactggtccgtaggattcgattggtcggggtaggagagttaaacaacatttaaacagagttctctcaaaaatgtctaaagggattgtaggtagataacatccaatcactgtttgcacttatctgaaatcttccctcttggctgcccccaggtatttactgtggagaacattgcataggaatgtctggaaaaagcttctacaacttgttacagccttcacatttgtagaagcttt

SEQ ID NO: 52 - DNA, 1234 bp, synthetic construct
  source 1..1234: mol_type = other DNA
atggccgccagcccccacaccctgagcagccgcctgctgaccggctgcgtgggcggcagcgtgtggtacctggagcgccgcaccatgatgtacgccctgttcctgctgagcgtgggcctggtgatgggcttcgtgggcttcagcagcaagcccagccccatctacggcggcctggtgctgatcgtgagcggcgtggtgggctgcgtgatcatcctgaacttcggcggcggctacatgggcctgatggtgttcctgatctacctgggcggcatgatggtggtgttcggctacaccaccgccatggccatcgaggagtaccccgaggcctggggcagcggcgtggaggtgctggtgagcgtgctggtgggcctggccatggaggtgggcctggtgctgtgggtgaaggagtacgacggcgtggtggtggtggtgaacttcaacagcgtgggcagctggatgatctacgagggcgagggcagcggcctgatccgcgaggaccccatcggcgccggcgccctgtacgactacggccgctggctggtggtggtgaccggctggaccctgttcgtgggcgtgtacatcgtgatcgagatcgcccgcggcaactaagagcactgggacgcccaccgcccctttccctccgctgccaggcgagcatgttgtggtaattctggaacacaagaagagaaattgctgggtttagaacaagattataaacgaattcggtgctcagtgatcacttgacagttttttttttttttaaatattacccaaaatgctccccaaataagaaatgcatcagctcagtcagtgaatacaaaaaaggaattatttttccctttgagggtcttttatacatctctcctccaaccccaccctctattctgtttcttcctcctcacatgggggtacacatacacagcttcctcttttggttccatccttaccaccacaccacacgcacactccacatgcccagcagagtggcacttggtggccagaaagtgtgagcctcatgatctgctgtctgtagttctgtgagctcaggtccctcaaaggcctcggagcacccccttccttgtgactgagccagggcctgcatttttggttttccccaccccacacattctcaaccatagtccttctaacaataccaatagctaggacccggctgctgtgcactgggactggggattccacatgtttgccttgggagtctcaagctggactgcca

SEQ ID NO: 53 - DNA, 2460 bp, synthetic construct
  source 1..2460: mol_type = other DNA
atggccgccagcccccacaccctgagcagccgcctgctgaccggctgcgtgggcggcagcgtgtggtacctggagcgccgcaccatggccaacctcctactcctcattgtacccattctaatcgcaatggcattcctaatgcttaccgaacgaaaaattctaggctatatgcaactacgcaaaggccccaacgttgtaggcccctacgggctactacaacccttcgctgacgccataaaactcttcaccaaagagcccctaaaacccgccacatctaccatcaccctctacatcaccgccccgaccttagctctcaccatcgctcttctactatggacccccctccccatgcccaaccccctggtcaacctcaacctaggcctcctatttattctagccacctctagcctagccgtttactcaatcctctggtcagggtgggcatcaaactcaaactacgccctgatcggcgcactgcgagcagtagcccaaacaatctcatatgaagtcaccctagccatcattctactatcaacattactaatgagtggctcctttaacctctccacccttatcacaacacaagaacacctctggttactcctgccatcatggcccttggccatgatgtggtttatctccacactagcagagaccaaccgaacccccttcgaccttgccgaaggggagtccgaactagtctcaggcttcaacatcgaatacgccgcaggccccttcgccctattcttcatggccgaatacacaaacattattatgatgaacaccctcaccactacaatcttcctaggaacaacatatgacgcactctcccctgaactctacacaacatattttgtcaccaagaccctacttctaacctccctgttcttatggattcgaacagcatacccccgattccgctacgaccaactcatgcacctcctatggaaaaacttcctaccactcaccctagcattacttatgtggtatgtctccatgcccattacaatctccagcattccccctcaaacctaagagcactgggacgcccaccgcccctttccctccgctgccaggcgagcatgttgtggtaattctggaacacaagaagagaaattgctgggtttagaacaagattataaacgaattcggtgctcagtgatcacttgacagttttttttttttttaaatattacccaaaatgctccccaaataagaaatgcatcagctcagtcagtgaatacaaaaaaggaattatttttccctttgagggtcttttatacatctctcctccaaccccaccctctattctgtttcttcctcctcacatgggggtacacatacacagcttcctcttttggttccatccttaccaccacaccacacgcacactccacatgcccagcagagtggcacttggtggccagaaagtgtgagcctcatgatctgctgtctgtagttctgtgagctcaggtccctcaaaggcctcggagcacccccttccttgtgactgagccagggcctgcatttttggttttccccaccccacacattctcaaccatagtccttctaacaataccaatagctaggacccggctgctgtgcactgggactggggattccacatgtttgccttgggagtctcaagctggactgccagcccctgtcctcccttcacccccattgcgtatgagcatttcagaactccaaggagtcacaggcatctttatagttcacgttaacatatagacactgttggaagcagttccttctaaaagggtagccctggacttaataccagccggatacctctggcccccaccccattactgtacctctggagtcactactgtgggtcgccactcctctgctacacagcacggctttttcaaggctgtattgagaagggaagttaggaagaagggtgtgctgggctaaccagcccacagagctcacattcctgtcccttgggtgaaaaatacatgtccatcctgatatctcctgaattcagaaattagcctccacatgtgcaatggctttaagagccagaagcagggttctgggaattttgcaagttacctgtggccaggtgtggtctcggttaccaaatacggttacctgcagctttttagtcctttgtgctcccacgggtctacagagtcccatctgcccaaaggtcttgaagcttgacaggatgttttcgattactcagtctcccagggcactactggtccgtaggattcgattggtcggggtaggagagttaaacaacatttaaacagagttctctcaaaaatgtctaaagggattgtaggtagataacatccaatcactgtttgcacttatctgaaatcttccctcttggctgcccccaggtatttactgtggagaacattgcataggaatgtctggaaaaagcttctacaacttgttacagccttcacatttgtagaagcttt

SEQ ID NO: 54 - DNA, 1660 bp, synthetic construct
  source 1..1660: mol_type = other DNA
atggccgccagcccccacaccctgagcagccgcctgctgaccggctgcgtgggcggcagcgtgtggtacctggagcgccgcaccatggccaacctcctactcctcattgtacccattctaatcgcaatggcattcctaatgcttaccgaacgaaaaattctaggctatatgcaactacgcaaaggccccaacgttgtaggcccctacgggctactacaacccttcgctgacgccataaaactcttcaccaaagagcccctaaaacccgccacatctaccatcaccctctacatcaccgccccgaccttagctctcaccatcgctcttctactatggacccccctccccatgcccaaccccctggtcaacctcaacctaggcctcctatttattctagccacctctagcctagccgtttactcaatcctctggtcagggtgggcatcaaactcaaactacgccctgatcggcgcactgcgagcagtagcccaaacaatctcatatgaagtcaccctagccatcattctactatcaacattactaatgagtggctcctttaacctctccacccttatcacaacacaagaacacctctggttactcctgccatcatggcccttggccatgatgtggtttatctccacactagcagagaccaaccgaacccccttcgaccttgccgaaggggagtccgaactagtctcaggcttcaacatcgaatacgccgcaggccccttcgccctattcttcatggccgaatacacaaacattattatgatgaacaccctcaccactacaatcttcctaggaacaacatatgacgcactctcccctgaactctacacaacatattttgtcaccaagaccctacttctaacctccctgttcttatggattcgaacagcatacccccgattccgctacgaccaactcatgcacctcctatggaaaaacttcctaccactcaccctagcattacttatgtggtatgtctccatgcccattacaatctccagcattccccctcaaacctaagagcactgggacgcccaccgcccctttccctccgctgccaggcgagcatgttgtggtaattctggaacacaagaagagaaattgctgggtttagaacaagattataaacgaattcggtgctcagtgatcacttgacagttttttttttttttaaatattacccaaaatgctccccaaataagaaatgcatcagctcagtcagtgaatacaaaaaaggaattatttttccctttgagggtcttttatacatctctcctccaaccccaccctctattctgtttcttcctcctcacatgggggtacacatacacagcttcctcttttggttccatccttaccaccacaccacacgcacactccacatgcccagcagagtggcacttggtggccagaaagtgtgagcctcatgatctgctgtctgtagttctgtgagctcaggtccctcaaaggcctcggagcacccccttccttgtgactgagccagggcctgcatttttggttttccccaccccacacattctcaaccatagtccttctaacaataccaatagctaggacccggctgctgtgcactgggactggggattccacatgtttgccttgggagtctcaagctggactgcca

SEQ ID NO: 55 - DNA, 2460 bp, synthetic construct
  source 1..2460: mol_type = other DNA
atggccgccagcccccacaccctgagcagccgcctgctgaccggctgcgtgggcggcagcgtgtggtacctggagcgccgcaccatggccaacctgctgctgctgatcgtgcccatcctgatcgccatggccttcctgatgctgaccgagcgcaagatcctgggctacatgcagctgcgcaagggccccaacgtggtgggcccctacggcctgctgcagcccttcgccgacgccatcaagctgttcaccaaggagcccctgaagcccgccaccagcaccatcaccctgtacatcaccgcccccaccctggccctgaccatcgccctgctgctgtggacccccctgcccatgcccaaccccctggtgaacctgaacctgggcctgctgttcatcctggccaccagcagcctggccgtgtacagcatcctgtggagcggctgggccagcaacagcaactacgccctgatcggcgccctgcgcgccgtggcccagaccatcagctacgaggtgaccctggccatcatcctgctgagcaccctgctgatgagcggcagcttcaacctgagcaccctgatcaccacccaggagcacctgtggctgctgctgcccagctggcccctggccatgatgtggttcatcagcaccctggccgagaccaaccgcacccccttcgacctggccgagggcgagagcgagctggtgagcggcttcaacatcgagtacgccgccggccccttcgccctgttcttcatggccgagtacaccaacatcatcatgatgaacaccctgaccaccaccatcttcctgggcaccacctacgacgccctgagccccgagctgtacaccacctacttcgtgaccaagaccctgctgctgaccagcctgttcctgtggatccgcaccgcctacccccgcttccgctacgaccagctgatgcacctgctgtggaagaacttcctgcccctgaccctggccctgctgatgtggtacgtgagcatgcccatcaccatcagcagcatccccccccagacctaagagcactgggacgcccaccgcccctttccctccgctgccaggcgagcatgttgtggtaattctggaacacaagaagagaaattgctgggtttagaacaagattataaacgaattcggtgctcagtgatcacttgacagttttttttttttttaaatattacccaaaatgctccccaaataagaaatgcatcagctcagtcagtgaatacaaaaaaggaattatttttccctttgagggtcttttatacatctctcctccaaccccaccctctattctgtttcttcctcctcacatgggggtacacatacacagcttcctcttttggttccatccttaccaccacaccacacgcacactccacatgcccagcagagtggcacttggtggccagaaagtgtgagcctcatgatctgctgtctgtagttctgtgagctcaggtccctcaaaggcctcggagcacccccttccttgtgactgagccagggcctgcatttttggttttccccaccccacacattctcaaccatagtccttctaacaataccaatagctaggacccggctgctgtgcactgggactggggattccacatgtttgccttgggagtctcaagctggactgccagcccctgtcctcccttcacccccattgcgtatgagcatttcagaactccaaggagtcacaggcatctttatagttcacgttaacatatagacactgttggaagcagttccttctaaaagggtagccctggacttaataccagccggatacctctggcccccaccccattactgtacctctggagtcactactgtgggtcgccactcctctgctacacagcacggctttttcaaggctgtattgagaagggaagttaggaagaagggtgtgctgggctaaccagcccacagagctcacattcctgtcccttgggtgaaaaatacatgtccatcctgatatctcctgaattcagaaattagcctccacatgtgcaatggctttaagagccagaagcagggttctgggaattttgcaagttacctgtggccaggtgtggtctcggttaccaaatacggttacctgcagctttttagtcctttgtgctcccacgggtctacagagtcccatctgcccaaaggtcttgaagcttgacaggatgttttcgattactcagtctcccagggcactactggtccgtaggattcgattggtcggggtaggagagttaaacaacatttaaacagagttctctcaaaaatgtctaaagggattgtaggtagataacatccaatcactgtttgcacttatctgaaatcttccctcttggctgcccccaggtatttactgtggagaacattgcataggaatgtctggaaaaagcttctacaacttgttacagccttcacatttgtagaagcttt

SEQ ID NO: 56 - DNA, 1660 bp, synthetic construct
  source 1..1660: mol_type = other DNA
atggccgccagcccccacaccctgagcagccgcctgctgaccggctgcgtgggcggcagcgtgtggtacctggagcgccgcaccatggccaacctgctgctgctgatcgtgcccatcctgatcgccatggccttcctgatgctgaccgagcgcaagatcctgggctacatgcagctgcgcaagggccccaacgtggtgggcccctacggcctgctgcagcccttcgccgacgccatcaagctgttcaccaaggagcccctgaagcccgccaccagcaccatcaccctgtacatcaccgcccccaccctggccctgaccatcgccctgctgctgtggacccccctgcccatgcccaaccccctggtgaacctgaacctgggcctgctgttcatcctggccaccagcagcctggccgtgtacagcatcctgtggagcggctgggccagcaacagcaactacgccctgatcggcgccctgcgcgccgtggcccagaccatcagctacgaggtgaccctggccatcatcctgctgagcaccctgctgatgagcggcagcttcaacctgagcaccctgatcaccacccaggagcacctgtggctgctgctgcccagctggcccctggccatgatgtggttcatcagcaccctggccgagaccaaccgcacccccttcgacctggccgagggcgagagcgagctggtgagcggcttcaacatcgagtacgccgccggccccttcgccctgttcttcatggccgagtacaccaacatcatcatgatgaacaccctgaccaccaccatcttcctgggcaccacctacgacgccctgagccccgagctgtacaccacctacttcgtgaccaagaccctgctgctgaccagcctgttcctgtggatccgcaccgcctacccccgcttccgctacgaccagctgatgcacctgctgtggaagaacttcctgcccctgaccctggccctgctgatgtggtacgtgagcatgcccatcaccatcagcagcatccccccccagacctaagagcactgggacgcccaccgcccctttccctccgctgccaggcgagcatgttgtggtaattctggaacacaagaagagaaattgctgggtttagaacaagattataaacgaattcggtgctcagtgatcacttgacagttttttttttttttaaatattacccaaaatgctccccaaataagaaatgcatcagctcagtcagtgaatacaaaaaaggaattatttttccctttgagggtcttttatacatctctcctccaaccccaccctctattctgtttcttcctcctcacatgggggtacacatacacagcttcctcttttggttccatccttaccaccacaccacacgcacactccacatgcccagcagagtggcacttggtggccagaaagtgtgagcctcatgatctgctgtctgtagttctgtgagctcaggtccctcaaaggcctcggagcacccccttccttgtgactgagccagggcctgcatttttggttttccccaccccacacattctcaaccatagtccttctaacaataccaatagctaggacccggctgctgtgcactgggactggggattccacatgtttgccttgggagtctcaagctggactgcca

SEQ ID NO: 57 - DNA, 2892 bp, synthetic construct
  source 1..2892: mol_type = other DNA
atgtccgtcctgacgcgcctgctgctgcggggcttgacacggctcggctcggcggctccagtgcggcgcgccagaatccattcgttgatgctaaaactaatcgtcccaacaattatgttactaccactgacatggctttccaaaaaacacatgatttggatcaacacaaccacccacagcctaattattagcatcatccctctactattttttaaccaaatcaacaacaacctatttagctgttccccaaccttttcctccgaccccctaacaacccccctcctaatgctaactacctggctcctacccctcacaatcatggcaagccaacgccacttatccagtgaaccactatcacgaaaaaaactctacctctctatgctaatctccctacaaatctccttaattatgacattcacagccacagaactaatcatgttttatatcttcttcgaaaccacacttatccccaccttggctatcatcacccgatggggcaaccagccagaacgcctgaacgcaggcacatacttcctattctacaccctagtaggctcccttcccctactcatcgcactaatttacactcacaacaccctaggctcactaaacattctactactcactctcactgcccaagaactatcaaactcctgggccaacaacttaatgtggctagcttacacaatggcttttatggtaaagatgcctctttacggactccacttatggctccctaaagcccatgtcgaagcccccatcgctgggtcaatggtacttgccgcagtactcttaaaactaggcggctatggtatgatgcgcctcacactcattctcaaccccctgacaaaacacatggcctaccccttccttgtactatccctatggggcatgattatgacaagctccatctgcctacgacaaacagacctaaaatcgctcattgcatactcttcaatcagccacatggccctcgtagtaacagccattctcatccaaaccccctggagcttcaccggcgcagtcattctcatgatcgcccacgggcttacatcctcattactattctgcctagcaaactcaaactacgaacgcactcacagtcgcatcatgatcctctctcaaggacttcaaactctactcccactaatggctttttggtggcttctagcaagcctcgctaacctcgccttaccccccactattaacctactgggagaactctctgtgctagtaaccacgttctcctggtcaaatatcactctcctacttacaggactcaacatgctagtcacagccctatactccctctacatgtttaccacaacacaatggggctcactcacccaccacattaacaacatgaaaccctcattcacacgagaaaacaccctcatgttcatgcacctatcccccattctcctcctatccctcaaccccgacatcattaccgggttttcctcttaagagcactgggacgcccaccgcccctttccctccgctgccaggcgagcatgttgtggtaattctggaacacaagaagagaaattgctgggtttagaacaagattataaacgaattcggtgctcagtgatcacttgacagttttttttttttttaaatattacccaaaatgctccccaaataagaaatgcatcagctcagtcagtgaatacaaaaaaggaattatttttccctttgagggtcttttatacatctctcctccaaccccaccctctattctgtttcttcctcctcacatgggggtacacatacacagcttcctcttttggttccatccttaccaccacaccacacgcacactccacatgcccagcagagtggcacttggtggccagaaagtgtgagcctcatgatctgctgtctgtagttctgtgagctcaggtccctcaaaggcctcggagcacccccttccttgtgactgagccagggcctgcatttttggttttccccaccccacacattctcaaccatagtccttctaacaataccaatagctaggacccggctgctgtgcactgggactggggattccacatgtttgccttgggagtctcaagctggactgccagcccctgtcctcccttcacccccattgcgtatgagcatttcagaactccaaggagtcacaggcatctttatagttcacgttaacatatagacactgttggaagcagttccttctaaaagggtagccctggacttaataccagccggatacctctggcccccaccccattactgtacctctggagtcactactgtgggtcgccactcctctgctacacagcacggctttttcaaggctgtattgagaagggaagttaggaagaagggtgtgctgggctaaccagcccacagagctcacattcctgtcccttgggtgaaaaatacatgtccatcctgatatctcctgaattcagaaattagcctccacatgtgcaatggctttaagagccagaagcagggttctgggaattttgcaagttacctgtggccaggtgtggtctcggttaccaaatacggttacctgcagctttttagtcctttgtgctcccacgggtctacagagtcccatctgcccaaaggtcttgaagcttgacaggatgttttcgattactcagtctcccagggcactactggtccgtaggattcgattggtcggggtaggagagttaaacaacatttaaacagagttctctcaaaaatgtctaaagggattgtaggtagataacatccaatcactgtttgcacttatctgaaatcttccctcttggctgcccccaggtatttactgtggagaacattgcataggaatgtctggaaaaagcttctacaacttgttacagccttcacatttgtagaagcttt

SEQ ID NO: 58 - DNA, 2092 bp, synthetic construct
  source 1..2092: mol_type = other DNA
atgtccgtcctgacgcgcctgctgctgcggggcttgacacggctcggctcggcggctccagtgcggcgcgccagaatccattcgttgatgctaaaactaatcgtcccaacaattatgttactaccactgacatggctttccaaaaaacacatgatttggatcaacacaaccacccacagcctaattattagcatcatccctctactattttttaaccaaatcaacaacaacctatttagctgttccccaaccttttcctccgaccccctaacaacccccctcctaatgctaactacctggctcctacccctcacaatcatggcaagccaacgccacttatccagtgaaccactatcacgaaaaaaactctacctctctatgctaatctccctacaaatctccttaattatgacattcacagccacagaactaatcatgttttatatcttcttcgaaaccacacttatccccaccttggctatcatcacccgatggggcaaccagccagaacgcctgaacgcaggcacatacttcctattctacaccctagtaggctcccttcccctactcatcgcactaatttacactcacaacaccctaggctcactaaacattctactactcactctcactgcccaagaactatcaaactcctgggccaacaacttaatgtggctagcttacacaatggcttttatggtaaagatgcctctttacggactccacttatggctccctaaagcccatgtcgaagcccccatcgctgggtcaatggtacttgccgcagtactcttaaaactaggcggctatggtatgatgcgcctcacactcattctcaaccccctgacaaaacacatggcctaccccttccttgtactatccctatggggcatgattatgacaagctccatctgcctacgacaaacagacctaaaatcgctcattgcatactcttcaatcagccacatggccctcgtagtaacagccattctcatccaaaccccctggagcttcaccggcgcagtcattctcatgatcgcccacgggcttacatcctcattactattctgcctagcaaactcaaactacgaacgcactcacagtcgcatcatgatcctctctcaaggacttcaaactctactcccactaatggctttttggtggcttctagcaagcctcgctaacctcgccttaccccccactattaacctactgggagaactctctgtgctagtaaccacgttctcctggtcaaatatcactctcctacttacaggactcaacatgctagtcacagccctatactccctctacatgtttaccacaacacaatggggctcactcacccaccacattaacaacatgaaaccctcattcacacgagaaaacaccctcatgttcatgcacctatcccccattctcctcctatccctcaaccccgacatcattaccgggttttcctcttaagagcactgggacgcccaccgcccctttccctccgctgccaggcgagcatgttgtggtaattctggaacacaagaagagaaattgctgggtttagaacaagattataaacgaattcggtgctcagtgatcacttgacagttttttttttttttaaatattacccaaaatgctccccaaataagaaatgcatcagctcagtcagtgaatacaaaaaaggaattatttttccctttgagggtcttttatacatctctcctccaaccccaccctctattctgtttcttcctcctcacatgggggtacacatacacagcttcctcttttggttccatccttaccaccacaccacacgcacactccacatgcccagcagagtggcacttggtggccagaaagtgtgagcctcatgatctgctgtctgtagttctgtgagctcaggtccctcaaaggcctcggagcacccccttccttgtgactgagccagggcctgcatttttggttttccccaccccacacattctcaaccatagtccttctaacaataccaatagctaggacccggctgctgtgcactgggactggggattccacatgtttgccttgggagtctcaagctggactgcca

SEQ ID NO: 59 - DNA, 2892 bp, synthetic construct
  source 1..2892: mol_type = other DNA
atgtccgtcctgacgcgcctgctgctgcggggcttgacacggctcggctcggcggctccagtgcggcgcgccagaatccattcgttgatgctgaagctgatcgtgcccaccatcatgctgctgcctctgacctggctgagcaagaaacacatgatctggatcaacaccaccacgcacagcctgatcatcagcatcatccctctgctgttcttcaaccagatcaacaacaacctgttcagctgcagccccaccttcagcagcgaccctctgacaacacctctgctgatgctgaccacctggctgctgcccctcacaatcatggcctctcagagacacctgagcagcgagcccctgagccggaagaaactgtacctgagcatgctgatctccctgcagatctctctgatcatgaccttcaccgccaccgagctgatcatgttctacatctttttcgagacaacgctgatccccacactggccatcatcaccagatggggcaaccagcctgagagactgaacgccggcacctactttctgttctacaccctcgtgggcagcctgccactgctgattgccctgatctacacccacaacaccctgggctccctgaacatcctgctgctgacactgacagcccaagagctgagcaacagctgggccaacaatctgatgtggctggcctacacaatggccttcatggtcaagatgcccctgtacggcctgcacctgtggctgcctaaagctcatgtggaagcccctatcgccggctctatggtgctggctgcagtgctgctgaaactcggcggctacggcatgatgcggctgaccctgattctgaatcccctgaccaagcacatggcctatccatttctggtgctgagcctgtggggcatgattatgaccagcagcatctgcctgcggcagaccgatctgaagtccctgatcgcctacagctccatcagccacatggccctggtggtcaccgccatcctgattcagaccccttggagctttacaggcgccgtgatcctgatgattgcccacggcctgacaagcagcctgctgttttgtctggccaacagcaactacgagcggacccacagcagaatcatgatcctgtctcagggcctgcagaccctcctgcctcttatggctttttggtggctgctggcctctctggccaatctggcactgcctcctaccatcaatctgctgggcgagctgagcgtgctggtcaccacattcagctggtccaatatcaccctgctgctcaccggcctgaacatgctggttacagccctgtactccctgtacatgttcaccaccacacagtggggaagcctgacacaccacatcaacaatatgaagcccagcttcacccgcgagaacaccctgatgttcatgcatctgagccccattctgctgctgtccctgaatcctgatatcatcaccggcttctccagctgagagcactgggacgcccaccgcccctttccctccgctgccaggcgagcatgttgtggtaattctggaacacaagaagagaaattgctgggtttagaacaagattataaacgaattcggtgctcagtgatcacttgacagttttttttttttttaaatattacccaaaatgctccccaaataagaaatgcatcagctcagtcagtgaatacaaaaaaggaattatttttccctttgagggtcttttatacatctctcctccaaccccaccctctattctgtttcttcctcctcacatgggggtacacatacacagcttcctcttttggttccatccttaccaccacaccacacgcacactccacatgcccagcagagtggcacttggtggccagaaagtgtgagcctcatgatctgctgtctgtagttctgtgagctcaggtccctcaaaggcctcggagcacccccttccttgtgactgagccagggcctgcatttttggttttccccaccccacacattctcaaccatagtccttctaacaataccaatagctaggacccggctgctgtgcactgggactggggattccacatgtttgccttgggagtctcaagctggactgccagcccctgtcctcccttcacccccattgcgtatgagcatttcagaactccaaggagtcacaggcatctttatagttcacgttaacatatagacactgttggaagcagttccttctaaaagggtagccctggacttaataccagccggatacctctggcccccaccccattactgtacctctggagtcactactgtgggtcgccactcctctgctacacagcacggctttttcaaggctgtattgagaagggaagttaggaagaagggtgtgctgggctaaccagcccacagagctcacattcctgtcccttgggtgaaaaatacatgtccatcctgatatctcctgaattcagaaattagcctccacatgtgcaatggctttaagagccagaagcagggttctgggaattttgcaagttacctgtggccaggtgtggtctcggttaccaaatacggttacctgcagctttttagtcctttgtgctcccacgggtctacagagtcccatctgcccaaaggtcttgaagcttgacaggatgttttcgattactcagtctcccagggcactactggtccgtaggattcgattggtcggggtaggagagttaaacaacatttaaacagagttctctcaaaaatgtctaaagggattgtaggtagataacatccaatcactgtttgcacttatctgaaatcttccctcttggctgcccccaggtatttactgtggagaacattgcataggaatgtctggaaaaagcttctacaacttgttacagccttcacatttgtagaagcttt

SEQ ID NO: 60 - DNA, 2092 bp, synthetic construct
  source 1..2092: mol_type = other DNA
atgtccgtcctgacgcgcctgctgctgcggggcttgacacggctcggctcggcggctccagtgcggcgcgccagaatccattcgttgatgctgaagctgatcgtgcccaccatcatgctgctgcctctgacctggctgagcaagaaacacatgatctggatcaacaccaccacgcacagcctgatcatcagcatcatccctctgctgttcttcaaccagatcaacaacaacctgttcagctgcagccccaccttcagcagcgaccctctgacaacacctctgctgatgctgaccacctggctgctgcccctcacaatcatggcctctcagagacacctgagcagcgagcccctgagccggaagaaactgtacctgagcatgctgatctccctgcagatctctctgatcatgaccttcaccgccaccgagctgatcatgttctacatctttttcgagacaacgctgatccccacactggccatcatcaccagatggggcaaccagcctgagagactgaacgccggcacctactttctgttctacaccctcgtgggcagcctgccactgctgattgccctgatctacacccacaacaccctgggctccctgaacatcctgctgctgacactgacagcccaagagctgagcaacagctgggccaacaatctgatgtggctggcctacacaatggccttcatggtcaagatgcccctgtacggcctgcacctgtggctgcctaaagctcatgtggaagcccctatcgccggctctatggtgctggctgcagtgctgctgaaactcggcggctacggcatgatgcggctgaccctgattctgaatcccctgaccaagcacatggcctatccatttctggtgctgagcctgtggggcatgattatgaccagcagcatctgcctgcggcagaccgatctgaagtccctgatcgcctacagctccatcagccacatggccctggtggtcaccgccatcctgattcagaccccttggagctttacaggcgccgtgatcctgatgattgcccacggcctgacaagcagcctgctgttttgtctggccaacagcaactacgagcggacccacagcagaatcatgatcctgtctcagggcctgcagaccctcctgcctcttatggctttttggtggctgctggcctctctggccaatctggcactgcctcctaccatcaatctgctgggcgagctgagcgtgctggtcaccacattcagctggtccaatatcaccctgctgctcaccggcctgaacatgctggttacagccctgtactccctgtacatgttcaccaccacacagtggggaagcctgacacaccacatcaacaatatgaagcccagcttcacccgcgagaacaccctgatgttcatgcatctgagccccattctgctgctgtccctgaatcctgatatcatcaccggcttctccagctgagagcactgggacgcccaccgcccctttccctccgctgccaggcgagcatgttgtggtaattctggaacacaagaagagaaattgctgggtttagaacaagattataaacgaattcggtgctcagtgatcacttgacagttttttttttttttaaatattacccaaaatgctccccaaataagaaatgcatcagctcagtcagtgaatacaaaaaaggaattatttttccctttgagggtcttttatacatctctcctccaaccccaccctctattctgtttcttcctcctcacatgggggtacacatacacagcttcctcttttggttccatccttaccaccacaccacacgcacactccacatgcccagcagagtggcacttggtggccagaaagtgtgagcctcatgatctgctgtctgtagttctgtgagctcaggtccctcaaaggcctcggagcacccccttccttgtgactgagccagggcctgcatttttggttttccccaccccacacattctcaaccatagtccttctaacaataccaatagctaggacccggctgctgtgcactgggactggggattccacatgtttgccttgggagtctcaagctggactgcca

SEQ ID NO: 61 - DNA, 2892 bp, synthetic construct
  source 1..2892: mol_type = other DNA
atgtccgtcctgacgcgcctgctgctgcggggcttgacacggctcggctcggcggctccagtgcggcgcgccagaatccattcgttgatgctgaagctgatcgtgcccaccatcatgctgctgcccctgacctggctgagcaagaagcacatgatctggatcaacaccaccacccacagcctgatcatcagcatcatccccctgctgttcttcaaccagatcaacaacaacctgttcagctgcagccccaccttcagcagcgaccccctgaccacccccctgctgatgctgaccacctggctgctgcccctgaccatcatggccagccagcgccacctgagcagcgagcccctgagccgcaagaagctgtacctgagcatgctgatcagcctgcagatcagcctgatcatgaccttcaccgccaccgagctgatcatgttctacatcttcttcgagaccaccctgatccccaccctggccatcatcacccgctggggcaaccagcccgagcgcctgaacgccggcacctacttcctgttctacaccctggtgggcagcctgcccctgctgatcgccctgatctacacccacaacaccctgggcagcctgaacatcctgctgctgaccctgaccgcccaggagctgagcaacagctgggccaacaacctgatgtggctggcctacaccatggccttcatggtgaagatgcccctgtacggcctgcacctgtggctgcccaaggcccacgtggaggcccccatcgccggcagcatggtgctggccgccgtgctgctgaagctgggcggctacggcatgatgcgcctgaccctgatcctgaaccccctgaccaagcacatggcctaccccttcctggtgctgagcctgtggggcatgatcatgaccagcagcatctgcctgcgccagaccgacctgaagagcctgatcgcctacagcagcatcagccacatggccctggtggtgaccgccatcctgatccagaccccctggagcttcaccggcgccgtgatcctgatgatcgcccacggcctgaccagcagcctgctgttctgcctggccaacagcaactacgagcgcacccacagccgcatcatgatcctgagccagggcctgcagaccctgctgcccctgatggccttctggtggctgctggccagcctggccaacctggccctgccccccaccatcaacctgctgggcgagctgagcgtgctggtgaccaccttcagctggagcaacatcaccctgctgctgaccggcctgaacatgctggtgaccgccctgtacagcctgtacatgttcaccaccacccagtggggcagcctgacccaccacatcaacaacatgaagcccagcttcacccgcgagaacaccctgatgttcatgcacctgagccccatcctgctgctgagcctgaaccccgacatcatcaccggcttcagcagctaagagcactgggacgcccaccgcccctttccctccgctgccaggcgagcatgttgtggtaattctggaacacaagaagagaaattgctgggtttagaacaagattataaacgaattcggtgctcagtgatcacttgacagttttttttttttttaaatattacccaaaatgctccccaaataagaaatgcatcagctcagtcagtgaatacaaaaaaggaattatttttccctttgagggtcttttatacatctctcctccaaccccaccctctattctgtttcttcctcctcacatgggggtacacatacacagcttcctcttttggttccatccttaccaccacaccacacgcacactccacatgcccagcagagtggcacttggtggccagaaagtgtgagcctcatgatctgctgtctgtagttctgtgagctcaggtccctcaaaggcctcggagcacccccttccttgtgactgagccagggcctgcatttttggttttccccaccccacacattctcaaccatagtccttctaacaataccaatagctaggacccggctgctgtgcactgggactggggattccacatgtttgccttgggagtctcaagctggactgccagcccctgtcctcccttcacccccattgcgtatgagcatttcagaactccaaggagtcacaggcatctttatagttcacgttaacatatagacactgttggaagcagttccttctaaaagggtagccctggacttaataccagccggatacctctggcccccaccccattactgtacctctggagtcactactgtgggtcgccactcctctgctacacagcacggctttttcaaggctgtattgagaagggaagttaggaagaagggtgtgctgggctaaccagcccacagagctcacattcctgtcccttgggtgaaaaatacatgtccatcctgatatctcctgaattcagaaattagcctccacatgtgcaatggctttaagagccagaagcagggttctgggaattttgcaagttacctgtggccaggtgtggtctcggttaccaaatacggttacctgcagctttttagtcctttgtgctcccacgggtctacagagtcccatctgcccaaaggtcttgaagcttgacaggatgttttcgattactcagtctcccagggcactactggtccgtaggattcgattggtcggggtaggagagttaaacaacatttaaacagagttctctcaaaaatgtctaaagggattgtaggtagataacatccaatcactgtttgcacttatctgaaatcttccctcttggctgcccccaggtatttactgtggagaacattgcataggaatgtctggaaaaagcttctacaacttgttacagccttcacatttgtagaagcttt

SEQ ID NO: 62 - DNA, 2092 bp, synthetic construct
  source 1..2092: mol_type = other DNA
atgtccgtcctgacgcgcctgctgctgcggggcttgacacggctcggctcggcggctccagtgcggcgcgccagaatccattcgttgatgctgaagctgatcgtgcccaccatcatgctgctgcccctgacctggctgagcaagaagcacatgatctggatcaacaccaccacccacagcctgatcatcagcatcatccccctgctgttcttcaaccagatcaacaacaacctgttcagctgcagccccaccttcagcagcgaccccctgaccacccccctgctgatgctgaccacctggctgctgcccctgaccatcatggccagccagcgccacctgagcagcgagcccctgagccgcaagaagctgtacctgagcatgctgatcagcctgcagatcagcctgatcatgaccttcaccgccaccgagctgatcatgttctacatcttcttcgagaccaccctgatccccaccctggccatcatcacccgctggggcaaccagcccgagcgcctgaacgccggcacctacttcctgttctacaccctggtgggcagcctgcccctgctgatcgccctgatctacacccacaacaccctgggcagcctgaacatcctgctgctgaccctgaccgcccaggagctgagcaacagctgggccaacaacctgatgtggctggcctacaccatggccttcatggtgaagatgcccctgtacggcctgcacctgtggctgcccaaggcccacgtggaggcccccatcgccggcagcatggtgctggccgccgtgctgctgaagctgggcggctacggcatgatgcgcctgaccctgatcctgaaccccctgaccaagcacatggcctaccccttcctggtgctgagcctgtggggcatgatcatgaccagcagcatctgcctgcgccagaccgacctgaagagcctgatcgcctacagcagcatcagccacatggccctggtggtgaccgccatcctgatccagaccccctggagcttcaccggcgccgtgatcctgatgatcgcccacggcctgaccagcagcctgctgttctgcctggccaacagcaactacgagcgcacccacagccgcatcatgatcctgagccagggcctgcagaccctgctgcccctgatggccttctggtggctgctggccagcctggccaacctggccctgccccccaccatcaacctgctgggcgagctgagcgtgctggtgaccaccttcagctggagcaacatcaccctgctgctgaccggcctgaacatgctggtgaccgccctgtacagcctgtacatgttcaccaccacccagtggggcagcctgacccaccacatcaacaacatgaagcccagcttcacccgcgagaacaccctgatgttcatgcacctgagccccatcctgctgctgagcctgaaccccgacatcatcaccggcttcagcagctaagagcactgggacgcccaccgcccctttccctccgctgccaggcgagcatgttgtggtaattctggaacacaagaagagaaattgctgggtttagaacaagattataaacgaattcggtgctcagtgatcacttgacagttttttttttttttaaatattacccaaaatgctccccaaataagaaatgcatcagctcagtcagtgaatacaaaaaaggaattatttttccctttgagggtcttttatacatctctcctccaaccccaccctctattctgtttcttcctcctcacatgggggtacacatacacagcttcctcttttggttccatccttaccaccacaccacacgcacactccacatgcccagcagagtggcacttggtggccagaaagtgtgagcctcatgatctgctgtctgtagttctgtgagctcaggtccctcaaaggcctcggagcacccccttccttgtgactgagccagggcctgcatttttggttttccccaccccacacattctcaaccatagtccttctaacaataccaatagctaggacccggctgctgtgcactgggactggggattccacatgtttgccttgggagtctcaagctggactgcca

SEQ ID NO: 63 - DNA, 2037 bp, synthetic construct
  source 1..2037: mol_type = other DNA
atgtccgtcctgacgcgcctgctgctgcggggcttgacacggctcggctcggcggctccagtgcggcgcgccagaatccattcgttgatgatgtatgctttgtttctgttgagtgtgggtttagtaatggggtttgtggggttttcttctaagccttctcctatttatgggggtttagtattgattgttagcggtgtggtcgggtgtgttattattctgaattttgggggaggttatatgggtttaatggtttttttaatttatttagggggaatgatggttgtctttggatatactacagcgatggctattgaggagtatcctgaggcatgggggtcaggggttgaggtcttggtgagtgttttagtggggttagcgatggaggtaggattggtgctgtgggtgaaagagtatgatggggtggtggttgtggtaaactttaatagtgtaggaagctggatgatttatgaaggagaggggtcagggttgattcgggaggatcctattggtgcgggggctttgtatgattatgggcgttggttagtagtagttactggttggacattgtttgttggtgtatatattgtaattgagattgctcgggggaattaggagcactgggacgcccaccgcccctttccctccgctgccaggcgagcatgttgtggtaattctggaacacaagaagagaaattgctgggtttagaacaagattataaacgaattcggtgctcagtgatcacttgacagttttttttttttttaaatattacccaaaatgctccccaaataagaaatgcatcagctcagtcagtgaatacaaaaaaggaattatttttccctttgagggtcttttatacatctctcctccaaccccaccctctattctgtttcttcctcctcacatgggggtacacatacacagcttcctcttttggttccatccttaccaccacaccacacgcacactccacatgcccagcagagtggcacttggtggccagaaagtgtgagcctcatgatctgctgtctgtagttctgtgagctcaggtccctcaaaggcctcggagcacccccttccttgtgactgagccagggcctgcatttttggttttccccaccccacacattctcaaccatagtccttctaacaataccaatagctaggacccggctgctgtgcactgggactggggattccacatgtttgccttgggagtctcaagctggactgccagcccctgtcctcccttcacccccattgcgtatgagcatttcagaactccaaggagtcacaggcatctttatagttcacgttaacatatagacactgttggaagcagttccttctaaaagggtagccctggacttaataccagccggatacctctggcccccaccccattactgtacctctggagtcactactgtgggtcgccactcctctgctacacagcacggctttttcaaggctgtattgagaagggaagttaggaagaagggtgtgctgggctaaccagcccacagagctcacattcctgtcccttgggtgaaaaatacatgtccatcctgatatctcctgaattcagaaattagcctccacatgtgcaatggctttaagagccagaagcagggttctgggaattttgcaagttacctgtggccaggtgtggtctcggttaccaaatacggttacctgcagctttttagtcctttgtgctcccacgggtctacagagtcccatctgcccaaaggtcttgaagcttgacaggatgttttcgattactcagtctcccagggcactactggtccgtaggattcgattggtcggggtaggagagttaaacaacatttaaacagagttctctcaaaaatgtctaaagggattgtaggtagataacatccaatcactgtttgcacttatctgaaatcttccctcttggctgcccccaggtatttactgtggagaacattgcataggaatgtctggaaaaagcttctacaacttgttacagccttcacatttgtagaagcttt

SEQ ID NO: 64 - DNA, 1237 bp, synthetic construct
  source 1..1237: mol_type = other DNA
atgtccgtcctgacgcgcctgctgctgcggggcttgacacggctcggctcggcggctccagtgcggcgcgccagaatccattcgttgatgatgtatgctttgtttctgttgagtgtgggtttagtaatggggtttgtggggttttcttctaagccttctcctatttatgggggtttagtattgattgttagcggtgtggtcgggtgtgttattattctgaattttgggggaggttatatgggtttaatggtttttttaatttatttagggggaatgatggttgtctttggatatactacagcgatggctattgaggagtatcctgaggcatgggggtcaggggttgaggtcttggtgagtgttttagtggggttagcgatggaggtaggattggtgctgtgggtgaaagagtatgatggggtggtggttgtggtaaactttaatagtgtaggaagctggatgatttatgaaggagaggggtcagggttgattcgggaggatcctattggtgcgggggctttgtatgattatgggcgttggttagtagtagttactggttggacattgtttgttggtgtatatattgtaattgagattgctcgggggaattaggagcactgggacgcccaccgcccctttccctccgctgccaggcgagcatgttgtggtaattctggaacacaagaagagaaattgctgggtttagaacaagattataaacgaattcggtgctcagtgatcacttgacagttttttttttttttaaatattacccaaaatgctccccaaataagaaatgcatcagctcagtcagtgaatacaaaaaaggaattatttttccctttgagggtcttttatacatctctcctccaaccccaccctctattctgtttcttcctcctcacatgggggtacacatacacagcttcctcttttggttccatccttaccaccacaccacacgcacactccacatgcccagcagagtggcacttggtggccagaaagtgtgagcctcatgatctgctgtctgtagttctgtgagctcaggtccctcaaaggcctcggagcacccccttccttgtgactgagccagggcctgcatttttggttttccccaccccacacattctcaaccatagtccttctaacaataccaatagctaggacccggctgctgtgcactgggactggggattccacatgtttgccttgggagtctcaagctggactgcca

SEQ ID NO: 65 - DNA, 2037 bp, synthetic construct
  source 1..2037: mol_type = other DNA
atgtccgtcctgacgcgcctgctgctgcggggcttgacacggctcggctcggcggctccagtgcggcgcgccagaatccattcgttgatgatgtacgccctgttcctgctgagcgtgggcctggtgatgggcttcgtgggcttcagcagcaagcccagccccatctacggcggcctggtgctgatcgtgagcggcgtggtgggctgcgtgatcatcctgaacttcggcggcggctacatgggcctgatggtgttcctgatctacctgggcggcatgatggtggtgttcggctacaccaccgccatggccatcgaggagtaccccgaggcctggggcagcggcgtggaggtgctggtgagcgtgctggtgggcctggccatggaggtgggcctggtgctgtgggtgaaggagtacgacggcgtggtggtggtggtgaacttcaacagcgtgggcagctggatgatctacgagggcgagggcagcggcctgatccgcgaggaccccatcggcgccggcgccctgtacgactacggccgctggctggtggtggtgaccggctggaccctgttcgtgggcgtgtacatcgtgatcgagatcgcccgcggcaactaagagcactgggacgcccaccgcccctttccctccgctgccaggcgagcatgttgtggtaattctggaacacaagaagagaaattgctgggtttagaacaagattataaacgaattcggtgctcagtgatcacttgacagttttttttttttttaaatattacccaaaatgctccccaaataagaaatgcatcagctcagtcagtgaatacaaaaaaggaattatttttccctttgagggtcttttatacatctctcctccaaccccaccctctattctgtttcttcctcctcacatgggggtacacatacacagcttcctcttttggttccatccttaccaccacaccacacgcacactccacatgcccagcagagtggcacttggtggccagaaagtgtgagcctcatgatctgctgtctgtagttctgtgagctcaggtccctcaaaggcctcggagcacccccttccttgtgactgagccagggcctgcatttttggttttccccaccccacacattctcaaccatagtccttctaacaataccaatagctaggacccggctgctgtgcactgggactggggattccacatgtttgccttgggagtctcaagctggactgccagcccctgtcctcccttcacccccattgcgtatgagcatttcagaactccaaggagtcacaggcatctttatagttcacgttaacatatagacactgttggaagcagttccttctaaaagggtagccctggacttaataccagccggatacctctggcccccaccccattactgtacctctggagtcactactgtgggtcgccactcctctgctacacagcacggctttttcaaggctgtattgagaagggaagttaggaagaagggtgtgctgggctaaccagcccacagagctcacattcctgtcccttgggtgaaaaatacatgtccatcctgatatctcctgaattcagaaattagcctccacatgtgcaatggctttaagagccagaagcagggttctgggaattttgcaagttacctgtggccaggtgtggtctcggttaccaaatacggttacctgcagctttttagtcctttgtgctcccacgggtctacagagtcccatctgcccaaaggtcttgaagcttgacaggatgttttcgattactcagtctcccagggcactactggtccgtaggattcgattggtcggggtaggagagttaaacaacatttaaacagagttctctcaaaaatgtctaaagggattgtaggtagataacatccaatcactgtttgcacttatctgaaatcttccctcttggctgcccccaggtatttactgtggagaacattgcataggaatgtctggaaaaagcttctacaacttgttacagccttcacatttgtagaagcttt

SEQ ID NO: 66 - DNA, 1237 bp, synthetic construct
  source 1..1237: mol_type = other DNA
atgtccgtcctgacgcgcctgctgctgcggggcttgacacggctcggctcggcggctccagtgcggcgcgccagaatccattcgttgatgatgtacgccctgttcctgctgagcgtgggcctggtgatgggcttcgtgggcttcagcagcaagcccagccccatctacggcggcctggtgctgatcgtgagcggcgtggtgggctgcgtgatcatcctgaacttcggcggcggctacatgggcctgatggtgttcctgatctacctgggcggcatgatggtggtgttcggctacaccaccgccatggccatcgaggagtaccccgaggcctggggcagcggcgtggaggtgctggtgagcgtgctggtgggcctggccatggaggtgggcctggtgctgtgggtgaaggagtacgacggcgtggtggtggtggtgaacttcaacagcgtgggcagctggatgatctacgagggcgagggcagcggcctgatccgcgaggaccccatcggcgccggcgccctgtacgactacggccgctggctggtggtggtgaccggctggaccctgttcgtgggcgtgtacatcgtgatcgagatcgcccgcggcaactaagagcactgggacgcccaccgcccctttccctccgctgccaggcgagcatgttgtggtaattctggaacacaagaagagaaattgctgggtttagaacaagattataaacgaattcggtgctcagtgatcacttgacagttttttttttttttaaatattacccaaaatgctccccaaataagaaatgcatcagctcagtcagtgaatacaaaaaaggaattatttttccctttgagggtcttttatacatctctcctccaaccccaccctctattctgtttcttcctcctcacatgggggtacacatacacagcttcctcttttggttccatccttaccaccacaccacacgcacactccacatgcccagcagagtggcacttggtggccagaaagtgtgagcctcatgatctgctgtctgtagttctgtgagctcaggtccctcaaaggcctcggagcacccccttccttgtgactgagccagggcctgcatttttggttttccccaccccacacattctcaaccatagtccttctaacaataccaatagctaggacccggctgctgtgcactgggactggggattccacatgtttgccttgggagtctcaagctggactgcca

SEQ ID NO: 67 - DNA, 2463 bp, synthetic construct
  source 1..2463: mol_type = other DNA
atgtccgtcctgacgcgcctgctgctgcggggcttgacacggctcggctcggcggctccagtgcggcgcgccagaatccattcgttgatggccaacctcctactcctcattgtacccattctaatcgcaatggcattcctaatgcttaccgaacgaaaaattctaggctatatgcaactacgcaaaggccccaacgttgtaggcccctacgggctactacaacccttcgctgacgccataaaactcttcaccaaagagcccctaaaacccgccacatctaccatcaccctctacatcaccgccccgaccttagctctcaccatcgctcttctactatggacccccctccccatgcccaaccccctggtcaacctcaacctaggcctcctatttattctagccacctctagcctagccgtttactcaatcctctggtcagggtgggcatcaaactcaaactacgccctgatcggcgcactgcgagcagtagcccaaacaatctcatatgaagtcaccctagccatcattctactatcaacattactaatgagtggctcctttaacctctccacccttatcacaacacaagaacacctctggttactcctgccatcatggcccttggccatgatgtggtttatctccacactagcagagaccaaccgaacccccttcgaccttgccgaaggggagtccgaactagtctcaggcttcaacatcgaatacgccgcaggccccttcgccctattcttcatggccgaatacacaaacattattatgatgaacaccctcaccactacaatcttcctaggaacaacatatgacgcactctcccctgaactctacacaacatattttgtcaccaagaccctacttctaacctccctgttcttatggattcgaacagcatacccccgattccgctacgaccaactcatgcacctcctatggaaaaacttcctaccactcaccctagcattacttatgtggtatgtctccatgcccattacaatctccagcattccccctcaaacctaagagcactgggacgcccaccgcccctttccctccgctgccaggcgagcatgttgtggtaattctggaacacaagaagagaaattgctgggtttagaacaagattataaacgaattcggtgctcagtgatcacttgacagttttttttttttttaaatattacccaaaatgctccccaaataagaaatgcatcagctcagtcagtgaatacaaaaaaggaattatttttccctttgagggtcttttatacatctctcctccaaccccaccctctattctgtttcttcctcctcacatgggggtacacatacacagcttcctcttttggttccatccttaccaccacaccacacgcacactccacatgcccagcagagtggcacttggtggccagaaagtgtgagcctcatgatctgctgtctgtagttctgtgagctcaggtccctcaaaggcctcggagcacccccttccttgtgactgagccagggcctgcatttttggttttccccaccccacacattctcaaccatagtccttctaacaataccaatagctaggacccggctgctgtgcactgggactggggattccacatgtttgccttgggagtctcaagctggactgccagcccctgtcctcccttcacccccattgcgtatgagcatttcagaactccaaggagtcacaggcatctttatagttcacgttaacatatagacactgttggaagcagttccttctaaaagggtagccctggacttaataccagccggatacctctggcccccaccccattactgtacctctggagtcactactgtgggtcgccactcctctgctacacagcacggctttttcaaggctgtattgagaagggaagttaggaagaagggtgtgctgggctaaccagcccacagagctcacattcctgtcccttgggtgaaaaatacatgtccatcctgatatctcctgaattcagaaattagcctccacatgtgcaatggctttaagagccagaagcagggttctgggaattttgcaagttacctgtggccaggtgtggtctcggttaccaaatacggttacctgcagctttttagtcctttgtgctcccacgggtctacagagtcccatctgcccaaaggtcttgaagcttgacaggatgttttcgattactcagtctcccagggcactactggtccgtaggattcgattggtcggggtaggagagttaaacaacatttaaacagagttctctcaaaaatgtctaaagggattgtaggtagataacatccaatcactgtttgcacttatctgaaatcttccctcttggctgcccccaggtatttactgtggagaacattgcataggaatgtctggaaaaagcttctacaacttgttacagccttcacatttgtagaagcttt

SEQ ID NO: 68 - DNA, 1663 bp, synthetic construct
  source 1..1663: mol_type = other DNA
atgtccgtcctgacgcgcctgctgctgcggggcttgacacggctcggctcggcggctccagtgcggcgcgccagaatccattcgttgatggccaacctcctactcctcattgtacccattctaatcgcaatggcattcctaatgcttaccgaacgaaaaattctaggctatatgcaactacgcaaaggccccaacgttgtaggcccctacgggctactacaacccttcgctgacgccataaaactcttcaccaaagagcccctaaaacccgccacatctaccatcaccctctacatcaccgccccgaccttagctctcaccatcgctcttctactatggacccccctccccatgcccaaccccctggtcaacctcaacctaggcctcctatttattctagccacctctagcctagccgtttactcaatcctctggtcagggtgggcatcaaactcaaactacgccctgatcggcgcactgcgagcagtagcccaaacaatctcatatgaagtcaccctagccatcattctactatcaacattactaatgagtggctcctttaacctctccacccttatcacaacacaagaacacctctggttactcctgccatcatggcccttggccatgatgtggtttatctccacactagcagagaccaaccgaacccccttcgaccttgccgaaggggagtccgaactagtctcaggcttcaacatcgaatacgccgcaggccccttcgccctattcttcatggccgaatacacaaacattattatgatgaacaccctcaccactacaatcttcctaggaacaacatatgacgcactctcccctgaactctacacaacatattttgtcaccaagaccctacttctaacctccctgttcttatggattcgaacagcatacccccgattccgctacgaccaactcatgcacctcctatggaaaaacttcctaccactcaccctagcattacttatgtggtatgtctccatgcccattacaatctccagcattccccctcaaacctaagagcactgggacgcccaccgcccctttccctccgctgccaggcgagcatgttgtggtaattctggaacacaagaagagaaattgctgggtttagaacaagattataaacgaattcggtgctcagtgatcacttgacagttttttttttttttaaatattacccaaaatgctccccaaataagaaatgcatcagctcagtcagtgaatacaaaaaaggaattatttttccctttgagggtcttttatacatctctcctccaaccccaccctctattctgtttcttcctcctcacatgggggtacacatacacagcttcctcttttggttccatccttaccaccacaccacacgcacactccacatgcccagcagagtggcacttggtggccagaaagtgtgagcctcatgatctgctgtctgtagttctgtgagctcaggtccctcaaaggcctcggagcacccccttccttgtgactgagccagggcctgcatttttggttttccccaccccacacattctcaaccatagtccttctaacaataccaatagctaggacccggctgctgtgcactgggactggggattccacatgtttgccttgggagtctcaagctggactgcca

SEQ ID NO: 69 - DNA, 2463 bp, synthetic construct
  source 1..2463: mol_type = other DNA
atgtccgtcctgacgcgcctgctgctgcggggcttgacacggctcggctcggcggctccagtgcggcgcgccagaatccattcgttgatggccaacctgctgctgctgatcgtgcccatcctgatcgccatggccttcctgatgctgaccgagcgcaagatcctgggctacatgcagctgcgcaagggccccaacgtggtgggcccctacggcctgctgcagcccttcgccgacgccatcaagctgttcaccaaggagcccctgaagcccgccaccagcaccatcaccctgtacatcaccgcccccaccctggccctgaccatcgccctgctgctgtggacccccctgcccatgcccaaccccctggtgaacctgaacctgggcctgctgttcatcctggccaccagcagcctggccgtgtacagcatcctgtggagcggctgggccagcaacagcaactacgccctgatcggcgccctgcgcgccgtggcccagaccatcagctacgaggtgaccctggccatcatcctgctgagcaccctgctgatgagcggcagcttcaacctgagcaccctgatcaccacccaggagcacctgtggctgctgctgcccagctggcccctggccatgatgtggttcatcagcaccctggccgagaccaaccgcacccccttcgacctggccgagggcgagagcgagctggtgagcggcttcaacatcgagtacgccgccggccccttcgccctgttcttcatggccgagtacaccaacatcatcatgatgaacaccctgaccaccaccatcttcctgggcaccacctacgacgccctgagccccgagctgtacaccacctacttcgtgaccaagaccctgctgctgaccagcctgttcctgtggatccgcaccgcctacccccgcttccgctacgaccagctgatgcacctgctgtggaagaacttcctgcccctgaccctggccctgctgatgtggtacgtgagcatgcccatcaccatcagcagcatccccccccagacctaagagcactgggacgcccaccgcccctttccctccgctgccaggcgagcatgttgtggtaattctggaacacaagaagagaaattgctgggtttagaacaagattataaacgaattcggtgctcagtgatcacttgacagttttttttttttttaaatattacccaaaatgctccccaaataagaaatgcatcagctcagtcagtgaatacaaaaaaggaattatttttccctttgagggtcttttatacatctctcctccaaccccaccctctattctgtttcttcctcctcacatgggggtacacatacacagcttcctcttttggttccatccttaccaccacaccacacgcacactccacatgcccagcagagtggcacttggtggccagaaagtgtgagcctcatgatctgctgtctgtagttctgtgagctcaggtccctcaaaggcctcggagcacccccttccttgtgactgagccagggcctgcatttttggttttccccaccccacacattctcaaccatagtccttctaacaataccaatagctaggacccggctgctgtgcactgggactggggattccacatgtttgccttgggagtctcaagctggactgccagcccctgtcctcccttcacccccattgcgtatgagcatttcagaactccaaggagtcacaggcatctttatagttcacgttaacatatagacactgttggaagcagttccttctaaaagggtagccctggacttaataccagccggatacctctggcccccaccccattactgtacctctggagtcactactgtgggtcgccactcctctgctacacagcacggctttttcaaggctgtattgagaagggaagttaggaagaagggtgtgctgggctaaccagcccacagagctcacattcctgtcccttgggtgaaaaatacatgtccatcctgatatctcctgaattcagaaattagcctccacatgtgcaatggctttaagagccagaagcagggttctgggaattttgcaagttacctgtggccaggtgtggtctcggttaccaaatacggttacctgcagctttttagtcctttgtgctcccacgggtctacagagtcccatctgcccaaaggtcttgaagcttgacaggatgttttcgattactcagtctcccagggcactactggtccgtaggattcgattggtcggggtaggagagttaaacaacatttaaacagagttctctcaaaaatgtctaaagggattgtaggtagataacatccaatcactgtttgcacttatctgaaatcttccctcttggctgcccccaggtatttactgtggagaacattgcataggaatgtctggaaaaagcttctacaacttgttacagccttcacatttgtagaagcttt

SEQ ID NO: 70 - DNA, 1663 bp, synthetic construct
  source 1..1663: mol_type = other DNA
atgtccgtcctgacgcgcctgctgctgcggggcttgacacggctcggctcggcggctccagtgcggcgcgccagaatccattcgttgatggccaacctgctgctgctgatcgtgcccatcctgatcgccatggccttcctgatgctgaccgagcgcaagatcctgggctacatgcagctgcgcaagggccccaacgtggtgggcccctacggcctgctgcagcccttcgccgacgccatcaagctgttcaccaaggagcccctgaagcccgccaccagcaccatcaccctgtacatcaccgcccccaccctggccctgaccatcgccctgctgctgtggacccccctgcccatgcccaaccccctggtgaacctgaacctgggcctgctgttcatcctggccaccagcagcctggccgtgtacagcatcctgtggagcggctgggccagcaacagcaactacgccctgatcggcgccctgcgcgccgtggcccagaccatcagctacgaggtgaccctggccatcatcctgctgagcaccctgctgatgagcggcagcttcaacctgagcaccctgatcaccacccaggagcacctgtggctgctgctgcccagctggcccctggccatgatgtggttcatcagcaccctggccgagaccaaccgcacccccttcgacctggccgagggcgagagcgagctggtgagcggcttcaacatcgagtacgccgccggccccttcgccctgttcttcatggccgagtacaccaacatcatcatgatgaacaccctgaccaccaccatcttcctgggcaccacctacgacgccctgagccccgagctgtacaccacctacttcgtgaccaagaccctgctgctgaccagcctgttcctgtggatccgcaccgcctacccccgcttccgctacgaccagctgatgcacctgctgtggaagaacttcctgcccctgaccctggccctgctgatgtggtacgtgagcatgcccatcaccatcagcagcatccccccccagacctaagagcactgggacgcccaccgcccctttccctccgctgccaggcgagcatgttgtggtaattctggaacacaagaagagaaattgctgggtttagaacaagattataaacgaattcggtgctcagtgatcacttgacagttttttttttttttaaatattacccaaaatgctccccaaataagaaatgcatcagctcagtcagtgaatacaaaaaaggaattatttttccctttgagggtcttttatacatctctcctccaaccccaccctctattctgtttcttcctcctcacatgggggtacacatacacagcttcctcttttggttccatccttaccaccacaccacacgcacactccacatgcccagcagagtggcacttggtggccagaaagtgtgagcctcatgatctgctgtctgtagttctgtgagctcaggtccctcaaaggcctcggagcacccccttccttgtgactgagccagggcctgcatttttggttttccccaccccacacattctcaaccatagtccttctaacaataccaatagctaggacccggctgctgtgcactgggactggggattccacatgtttgccttgggagtctcaagctggactgcca

SEQ ID NO: 71 - DNA, 3071 bp, synthetic construct
  source 1..3071: mol_type = other DNA
gtgctgcccgcctagaaagggtgaagtggttgtttccgtgacggactgagtacgggtgcctgtcaggctcttgcggaagtccatgcgccattgggagggcctcggccgcggctctgtgcccttgctgctgagggccacttcctgggtcattcctggaccgggagccgggctggggctcacacgggggctcccgcgtggccgtctcggcgcctgcgtgacctccccgccggcgggatgtggcgactacgtcgggccgctgtggcctgatgctaaaactaatcgtcccaacaattatgttactaccactgacatggctttccaaaaaacacatgatttggatcaacacaaccacccacagcctaattattagcatcatccctctactattttttaaccaaatcaacaacaacctatttagctgttccccaaccttttcctccgaccccctaacaacccccctcctaatgctaactacctggctcctacccctcacaatcatggcaagccaacgccacttatccagtgaaccactatcacgaaaaaaactctacctctctatgctaatctccctacaaatctccttaattatgacattcacagccacagaactaatcatgttttatatcttcttcgaaaccacacttatccccaccttggctatcatcacccgatggggcaaccagccagaacgcctgaacgcaggcacatacttcctattctacaccctagtaggctcccttcccctactcatcgcactaatttacactcacaacaccctaggctcactaaacattctactactcactctcactgcccaagaactatcaaactcctgggccaacaacttaatgtggctagcttacacaatggcttttatggtaaagatgcctctttacggactccacttatggctccctaaagcccatgtcgaagcccccatcgctgggtcaatggtacttgccgcagtactcttaaaactaggcggctatggtatgatgcgcctcacactcattctcaaccccctgacaaaacacatggcctaccccttccttgtactatccctatggggcatgattatgacaagctccatctgcctacgacaaacagacctaaaatcgctcattgcatactcttcaatcagccacatggccctcgtagtaacagccattctcatccaaaccccctggagcttcaccggcgcagtcattctcatgatcgcccacgggcttacatcctcattactattctgcctagcaaactcaaactacgaacgcactcacagtcgcatcatgatcctctctcaaggacttcaaactctactcccactaatggctttttggtggcttctagcaagcctcgctaacctcgccttaccccccactattaacctactgggagaactctctgtgctagtaaccacgttctcctggtcaaatatcactctcctacttacaggactcaacatgctagtcacagccctatactccctctacatgtttaccacaacacaatggggctcactcacccaccacattaacaacatgaaaccctcattcacacgagaaaacaccctcatgttcatgcacctatcccccattctcctcctatccctcaaccccgacatcattaccgggttttcctcttaagagcactgggacgcccaccgcccctttccctccgctgccaggcgagcatgttgtggtaattctggaacacaagaagagaaattgctgggtttagaacaagattataaacgaattcggtgctcagtgatcacttgacagttttttttttttttaaatattacccaaaatgctccccaaataagaaatgcatcagctcagtcagtgaatacaaaaaaggaattatttttccctttgagggtcttttatacatctctcctccaaccccaccctctattctgtttcttcctcctcacatgggggtacacatacacagcttcctcttttggttccatccttaccaccacaccacacgcacactccacatgcccagcagagtggcacttggtggccagaaagtgtgagcctcatgatctgctgtctgtagttctgtgagctcaggtccctcaaaggcctcggagcacccccttccttgtgactgagccagggcctgcatttttggttttccccaccccacacattctcaaccatagtccttctaacaataccaatagctaggacccggctgctgtgcactgggactggggattccacatgtttgccttgggagtctcaagctggactgccagcccctgtcctcccttcacccccattgcgtatgagcatttcagaactccaaggagtcacaggcatctttatagttcacgttaacatatagacactgttggaagcagttccttctaaaagggtagccctggacttaataccagccggatacctctggcccccaccccattactgtacctctggagtcactactgtgggtcgccactcctctgctacacagcacggctttttcaaggctgtattgagaagggaagttaggaagaagggtgtgctgggctaaccagcccacagagctcacattcctgtcccttgggtgaaaaatacatgtccatcctgatatctcctgaattcagaaattagcctccacatgtgcaatggctttaagagccagaagcagggttctgggaattttgcaagttacctgtggccaggtgtggtctcggttaccaaatacggttacctgcagctttttagtcctttgtgctcccacgggtctacagagtcccatctgcccaaaggtcttgaagcttgacaggatgttttcgattactcagtctcccagggcactactggtccgtaggattcgattggtcggggtaggagagttaaacaacatttaaacagagttctctcaaaaatgtctaaagggattgtaggtagataacatccaatcactgtttgcacttatctgaaatcttccctcttggctgcccccaggtatttactgtggagaacattgcataggaatgtctggaaaaagcttctacaacttgttacagccttcacatttgtagaagcttt

SEQ ID NO: 72 - DNA, 2271 bp, synthetic construct
  source 1..2271: mol_type = other DNA
gtgctgcccgcctagaaagggtgaagtggttgtttccgtgacggactgagtacgggtgcctgtcaggctcttgcggaagtccatgcgccattgggagggcctcggccgcggctctgtgcccttgctgctgagggccacttcctgggtcattcctggaccgggagccgggctggggctcacacgggggctcccgcgtggccgtctcggcgcctgcgtgacctccccgccggcgggatgtggcgactacgtcgggccgctgtggcctgatgctaaaactaatcgtcccaacaattatgttactaccactgacatggctttccaaaaaacacatgatttggatcaacacaaccacccacagcctaattattagcatcatccctctactattttttaaccaaatcaacaacaacctatttagctgttccccaaccttttcctccgaccccctaacaacccccctcctaatgctaactacctggctcctacccctcacaatcatggcaagccaacgccacttatccagtgaaccactatcacgaaaaaaactctacctctctatgctaatctccctacaaatctccttaattatgacattcacagccacagaactaatcatgttttatatcttcttcgaaaccacacttatccccaccttggctatcatcacccgatggggcaaccagccagaacgcctgaacgcaggcacatacttcctattctacaccctagtaggctcccttcccctactcatcgcactaatttacactcacaacaccctaggctcactaaacattctactactcactctcactgcccaagaactatcaaactcctgggccaacaacttaatgtggctagcttacacaatggcttttatggtaaagatgcctctttacggactccacttatggctccctaaagcccatgtcgaagcccccatcgctgggtcaatggtacttgccgcagtactcttaaaactaggcggctatggtatgatgcgcctcacactcattctcaaccccctgacaaaacacatggcctaccccttccttgtactatccctatggggcatgattatgacaagctccatctgcctacgacaaacagacctaaaatcgctcattgcatactcttcaatcagccacatggccctcgtagtaacagccattctcatccaaaccccctggagcttcaccggcgcagtcattctcatgatcgcccacgggcttacatcctcattactattctgcctagcaaactcaaactacgaacgcactcacagtcgcatcatgatcctctctcaaggacttcaaactctactcccactaatggctttttggtggcttctagcaagcctcgctaacctcgccttaccccccactattaacctactgggagaactctctgtgctagtaaccacgttctcctggtcaaatatcactctcctacttacaggactcaacatgctagtcacagccctatactccctctacatgtttaccacaacacaatggggctcactcacccaccacattaacaacatgaaaccctcattcacacgagaaaacaccctcatgttcatgcacctatcccccattctcctcctatccctcaaccccgacatcattaccgggttttcctcttaagagcactgggacgcccaccgcccctttccctccgctgccaggcgagcatgttgtggtaattctggaacacaagaagagaaattgctgggtttagaacaagattataaacgaattcggtgctcagtgatcacttgacagttttttttttttttaaatattacccaaaatgctccccaaataagaaatgcatcagctcagtcagtgaatacaaaaaaggaattatttttccctttgagggtcttttatacatctctcctccaaccccaccctctattctgtttcttcctcctcacatgggggtacacatacacagcttcctcttttggttccatccttaccaccacaccacacgcacactccacatgcccagcagagtggcacttggtggccagaaagtgtgagcctcatgatctgctgtctgtagttctgtgagctcaggtccctcaaaggcctcggagcacccccttccttgtgactgagccagggcctgcatttttggttttccccaccccacacattctcaaccatagtccttctaacaataccaatagctaggacccggctgctgtgcactgggactggggattccacatgtttgccttgggagtctcaagctggactgcca

SEQ ID NO: 73 - DNA, 3071 bp, synthetic construct
  source 1..3071: mol_type = other DNA
gtgctgcccgcctagaaagggtgaagtggttgtttccgtgacggactgagtacgggtgcctgtcaggctcttgcggaagtccatgcgccattgggagggcctcggccgcggctctgtgcccttgctgctgagggccacttcctgggtcattcctggaccgggagccgggctggggctcacacgggggctcccgcgtggccgtctcggcgcctgcgtgacctccccgccggcgggatgtggcgactacgtcgggccgctgtggcctgatgctgaagctgatcgtgcccaccatcatgctgctgcctctgacctggctgagcaagaaacacatgatctggatcaacaccaccacgcacagcctgatcatcagcatcatccctctgctgttcttcaaccagatcaacaacaacctgttcagctgcagccccaccttcagcagcgaccctctgacaacacctctgctgatgctgaccacctggctgctgcccctcacaatcatggcctctcagagacacctgagcagcgagcccctgagccggaagaaactgtacctgagcatgctgatctccctgcagatctctctgatcatgaccttcaccgccaccgagctgatcatgttctacatctttttcgagacaacgctgatccccacactggccatcatcaccagatggggcaaccagcctgagagactgaacgccggcacctactttctgttctacaccctcgtgggcagcctgccactgctgattgccctgatctacacccacaacaccctgggctccctgaacatcctgctgctgacactgacagcccaagagctgagcaacagctgggccaacaatctgatgtggctggcctacacaatggccttcatggtcaagatgcccctgtacggcctgcacctgtggctgcctaaagctcatgtggaagcccctatcgccggctctatggtgctggctgcagtgctgctgaaactcggcggctacggcatgatgcggctgaccctgattctgaatcccctgaccaagcacatggcctatccatttctggtgctgagcctgtggggcatgattatgaccagcagcatctgcctgcggcagaccgatctgaagtccctgatcgcctacagctccatcagccacatggccctggtggtcaccgccatcctgattcagaccccttggagctttacaggcgccgtgatcctgatgattgcccacggcctgacaagcagcctgctgttttgtctggccaacagcaactacgagcggacccacagcagaatcatgatcctgtctcagggcctgcagaccctcctgcctcttatggctttttggtggctgctggcctctctggccaatctggcactgcctcctaccatcaatctgctgggcgagctgagcgtgctggtcaccacattcagctggtccaatatcaccctgctgctcaccggcctgaacatgctggttacagccctgtactccctgtacatgttcaccaccacacagtggggaagcctgacacaccacatcaacaatatgaagcccagcttcacccgcgagaacaccctgatgttcatgcatctgagccccattctgctgctgtccctgaatcctgatatcatcaccggcttctccagctgagagcactgggacgcccaccgcccctttccctccgctgccaggcgagcatgttgtggtaattctggaacacaagaagagaaattgctgggtttagaacaagattataaacgaattcggtgctcagtgatcacttgacagttttttttttttttaaatattacccaaaatgctccccaaataagaaatgcatcagctcagtcagtgaatacaaaaaaggaattatttttccctttgagggtcttttatacatctctcctccaaccccaccctctattctgtttcttcctcctcacatgggggtacacatacacagcttcctcttttggttccatccttaccaccacaccacacgcacactccacatgcccagcagagtggcacttggtggccagaaagtgtgagcctcatgatctgctgtctgtagttctgtgagctcaggtccctcaaaggcctcggagcacccccttccttgtgactgagccagggcctgcatttttggttttccccaccccacacattctcaaccatagtccttctaacaataccaatagctaggacccggctgctgtgcactgggactggggattccacatgtttgccttgggagtctcaagctggactgccagcccctgtcctcccttcacccccattgcgtatgagcatttcagaactccaaggagtcacaggcatctttatagttcacgttaacatatagacactgttggaagcagttccttctaaaagggtagccctggacttaataccagccggatacctctggcccccaccccattactgtacctctggagtcactactgtgggtcgccactcctctgctacacagcacggctttttcaaggctgtattgagaagggaagttaggaagaagggtgtgctgggctaaccagcccacagagctcacattcctgtcccttgggtgaaaaatacatgtccatcctgatatctcctgaattcagaaattagcctccacatgtgcaatggctttaagagccagaagcagggttctgggaattttgcaagttacctgtggccaggtgtggtctcggttaccaaatacggttacctgcagctttttagtcctttgtgctcccacgggtctacagagtcccatctgcccaaaggtcttgaagcttgacaggatgttttcgattactcagtctcccagggcactactggtccgtaggattcgattggtcggggtaggagagttaaacaacatttaaacagagttctctcaaaaatgtctaaagggattgtaggtagataacatccaatcactgtttgcacttatctgaaatcttccctcttggctgcccccaggtatttactgtggagaacattgcataggaatgtctggaaaaagcttctacaacttgttacagccttcacatttgtagaagcttt

SEQ ID NO: 74 - DNA, 2271 bp, synthetic construct
  source 1..2271: mol_type = other DNA
gtgctgcccgcctagaaagggtgaagtggttgtttccgtgacggactgagtacgggtgcctgtcaggctcttgcggaagtccatgcgccattgggagggcctcggccgcggctctgtgcccttgctgctgagggccacttcctgggtcattcctggaccgggagccgggctggggctcacacgggggctcccgcgtggccgtctcggcgcctgcgtgacctccccgccggcgggatgtggcgactacgtcgggccgctgtggcctgatgctgaagctgatcgtgcccaccatcatgctgctgcctctgacctggctgagcaagaaacacatgatctggatcaacaccaccacgcacagcctgatcatcagcatcatccctctgctgttcttcaaccagatcaacaacaacctgttcagctgcagccccaccttcagcagcgaccctctgacaacacctctgctgatgctgaccacctggctgctgcccctcacaatcatggcctctcagagacacctgagcagcgagcccctgagccggaagaaactgtacctgagcatgctgatctccctgcagatctctctgatcatgaccttcaccgccaccgagctgatcatgttctacatctttttcgagacaacgctgatccccacactggccatcatcaccagatggggcaaccagcctgagagactgaacgccggcacctactttctgttctacaccctcgtgggcagcctgccactgctgattgccctgatctacacccacaacaccctgggctccctgaacatcctgctgctgacactgacagcccaagagctgagcaacagctgggccaacaatctgatgtggctggcctacacaatggccttcatggtcaagatgcccctgtacggcctgcacctgtggctgcctaaagctcatgtggaagcccctatcgccggctctatggtgctggctgcagtgctgctgaaactcggcggctacggcatgatgcggctgaccctgattctgaatcccctgaccaagcacatggcctatccatttctggtgctgagcctgtggggcatgattatgaccagcagcatctgcctgcggcagaccgatctgaagtccctgatcgcctacagctccatcagccacatggccctggtggtcaccgccatcctgattcagaccccttggagctttacaggcgccgtgatcctgatgattgcccacggcctgacaagcagcctgctgttttgtctggccaacagcaactacgagcggacccacagcagaatcatgatcctgtctcagggcctgcagaccctcctgcctcttatggctttttggtggctgctggcctctctggccaatctggcactgcctcctaccatcaatctgctgggcgagctgagcgtgctggtcaccacattcagctggtccaatatcaccctgctgctcaccggcctgaacatgctggttacagccctgtactccctgtacatgttcaccaccacacagtggggaagcctgacacaccacatcaacaatatgaagcccagcttcacccgcgagaacaccctgatgttcatgcatctgagccccattctgctgctgtccctgaatcctgatatcatcaccggcttctccagctgagagcactgggacgcccaccgcccctttccctccgctgccaggcgagcatgttgtggtaattctggaacacaagaagagaaattgctgggtttagaacaagattataaacgaattcggtgctcagtgatcacttgacagttttttttttttttaaatattacccaaaatgctccccaaataagaaatgcatcagctcagtcagtgaatacaaaaaaggaattatttttccctttgagggtcttttatacatctctcctccaaccccaccctctattctgtttcttcctcctcacatgggggtacacatacacagcttcctcttttggttccatccttaccaccacaccacacgcacactccacatgcccagcagagtggcacttggtggccagaaagtgtgagcctcatgatctgctgtctgtagttctgtgagctcaggtccctcaaaggcctcggagcacccccttccttgtgactgagccagggcctgcatttttggttttccccaccccacacattctcaaccatagtccttctaacaataccaatagctaggacccggctgctgtgcactgggactggggattccacatgtttgccttgggagtctcaagctggactgcca

SEQ ID NO: 75 - DNA, 3071 bp, synthetic construct
  source 1..3071: mol_type = other DNA
gtgctgcccgcctagaaagggtgaagtggttgtttccgtgacggactgagtacgggtgcctgtcaggctcttgcggaagtccatgcgccattgggagggcctcggccgcggctctgtgcccttgctgctgagggccacttcctgggtcattcctggaccgggagccgggctggggctcacacgggggctcccgcgtggccgtctcggcgcctgcgtgacctccccgccggcgggatgtggcgactacgtcgggccgctgtggcctgatgctgaagctgatcgtgcccaccatcatgctgctgcccctgacctggctgagcaagaagcacatgatctggatcaacaccaccacccacagcctgatcatcagcatcatccccctgctgttcttcaaccagatcaacaacaacctgttcagctgcagccccaccttcagcagcgaccccctgaccacccccctgctgatgctgaccacctggctgctgcccctgaccatcatggccagccagcgccacctgagcagcgagcccctgagccgcaagaagctgtacctgagcatgctgatcagcctgcagatcagcctgatcatgaccttcaccgccaccgagctgatcatgttctacatcttcttcgagaccaccctgatccccaccctggccatcatcacccgctggggcaaccagcccgagcgcctgaacgccggcacctacttcctgttctacaccctggtgggcagcctgcccctgctgatcgccctgatctacacccacaacaccctgggcagcctgaacatcctgctgctgaccctgaccgcccaggagctgagcaacagctgggccaacaacctgatgtggctggcctacaccatggccttcatggtgaagatgcccctgtacggcctgcacctgtggctgcccaaggcccacgtggaggcccccatcgccggcagcatggtgctggccgccgtgctgctgaagctgggcggctacggcatgatgcgcctgaccctgatcctgaaccccctgaccaagcacatggcctaccccttcctggtgctgagcctgtggggcatgatcatgaccagcagcatctgcctgcgccagaccgacctgaagagcctgatcgcctacagcagcatcagccacatggccctggtggtgaccgccatcctgatccagaccccctggagcttcaccggcgccgtgatcctgatgatcgcccacggcctgaccagcagcctgctgttctgcctggccaacagcaactacgagcgcacccacagccgcatcatgatcctgagccagggcctgcagaccctgctgcccctgatggccttctggtggctgctggccagcctggccaacctggccctgccccccaccatcaacctgctgggcgagctgagcgtgctggtgaccaccttcagctggagcaacatcaccctgctgctgaccggcctgaacatgctggtgaccgccctgtacagcctgtacatgttcaccaccacccagtggggcagcctgacccaccacatcaacaacatgaagcccagcttcacccgcgagaacaccctgatgttcatgcacctgagccccatcctgctgctgagcctgaaccccgacatcatcaccggcttcagcagctaagagcactgggacgcccaccgcccctttccctccgctgccaggcgagcatgttgtggtaattctggaacacaagaagagaaattgctgggtttagaacaagattataaacgaattcggtgctcagtgatcacttgacagttttttttttttttaaatattacccaaaatgctccccaaataagaaatgcatcagctcagtcagtgaatacaaaaaaggaattatttttccctttgagggtcttttatacatctctcctccaaccccaccctctattctgtttcttcctcctcacatgggggtacacatacacagcttcctcttttggttccatccttaccaccacaccacacgcacactccacatgcccagcagagtggcacttggtggccagaaagtgtgagcctcatgatctgctgtctgtagttctgtgagctcaggtccctcaaaggcctcggagcacccccttccttgtgactgagccagggcctgcatttttggttttccccaccccacacattctcaaccatagtccttctaacaataccaatagctaggacccggctgctgtgcactgggactggggattccacatgtttgccttgggagtctcaagctggactgccagcccctgtcctcccttcacccccattgcgtatgagcatttcagaactccaaggagtcacaggcatctttatagttcacgttaacatatagacactgttggaagcagttccttctaaaagggtagccctggacttaataccagccggatacctctggcccccaccccattactgtacctctggagtcactactgtgggtcgccactcctctgctacacagcacggctttttcaaggctgtattgagaagggaagttaggaagaagggtgtgctgggctaaccagcccacagagctcacattcctgtcccttgggtgaaaaatacatgtccatcctgatatctcctgaattcagaaattagcctccacatgtgcaatggctttaagagccagaagcagggttctgggaattttgcaagttacctgtggccaggtgtggtctcggttaccaaatacggttacctgcagctttttagtcctttgtgctcccacgggtctacagagtcccatctgcccaaaggtcttgaagcttgacaggatgttttcgattactcagtctcccagggcactactggtccgtaggattcgattggtcggggtaggagagttaaacaacatttaaacagagttctctcaaaaatgtctaaagggattgtaggtagataacatccaatcactgtttgcacttatctgaaatcttccctcttggctgcccccaggtatttactgtggagaacattgcataggaatgtctggaaaaagcttctacaacttgttacagccttcacatttgtagaagcttt

SEQ ID NO: 76 - DNA, 2271 bp, synthetic construct
  source 1..2271: mol_type = other DNA
gtgctgcccgcctagaaagggtgaagtggttgtttccgtgacggactgagtacgggtgcctgtcaggctcttgcggaagtccatgcgccattgggagggcctcggccgcggctctgtgcccttgctgctgagggccacttcctgggtcattcctggaccgggagccgggctggggctcacacgggggctcccgcgtggccgtctcggcgcctgcgtgacctccccgccggcgggatgtggcgactacgtcgggccgctgtggcctgatgctgaagctgatcgtgcccaccatcatgctgctgcccctgacctggctgagcaagaagcacatgatctggatcaacaccaccacccacagcctgatcatcagcatcatccccctgctgttcttcaaccagatcaacaacaacctgttcagctgcagccccaccttcagcagcgaccccctgaccacccccctgctgatgctgaccacctggctgctgcccctgaccatcatggccagccagcgccacctgagcagcgagcccctgagccgcaagaagctgtacctgagcatgctgatcagcctgcagatcagcctgatcatgaccttcaccgccaccgagctgatcatgttctacatcttcttcgagaccaccctgatccccaccctggccatcatcacccgctggggcaaccagcccgagcgcctgaacgccggcacctacttcctgttctacaccctggtgggcagcctgcccctgctgatcgccctgatctacacccacaacaccctgggcagcctgaacatcctgctgctgaccctgaccgcccaggagctgagcaacagctgggccaacaacctgatgtggctggcctacaccatggccttcatggtgaagatgcccctgtacggcctgcacctgtggctgcccaaggcccacgtggaggcccccatcgccggcagcatggtgctggccgccgtgctgctgaagctgggcggctacggcatgatgcgcctgaccctgatcctgaaccccctgaccaagcacatggcctaccccttcctggtgctgagcctgtggggcatgatcatgaccagcagcatctgcctgcgccagaccgacctgaagagcctgatcgcctacagcagcatcagccacatggccctggtggtgaccgccatcctgatccagaccccctggagcttcaccggcgccgtgatcctgatgatcgcccacggcctgaccagcagcctgctgttctgcctggccaacagcaactacgagcgcacccacagccgcatcatgatcctgagccagggcctgcagaccctgctgcccctgatggccttctggtggctgctggccagcctggccaacctggccctgccccccaccatcaacctgctgggcgagctgagcgtgctggtgaccaccttcagctggagcaacatcaccctgctgctgaccggcctgaacatgctggtgaccgccctgtacagcctgtacatgttcaccaccacccagtggggcagcctgacccaccacatcaacaacatgaagcccagcttcacccgcgagaacaccctgatgttcatgcacctgagccccatcctgctgctgagcctgaaccccgacatcatcaccggcttcagcagctaagagcactgggacgcccaccgcccctttccctccgctgccaggcgagcatgttgtggtaattctggaacacaagaagagaaattgctgggtttagaacaagattataaacgaattcggtgctcagtgatcacttgacagttttttttttttttaaatattacccaaaatgctccccaaataagaaatgcatcagctcagtcagtgaatacaaaaaaggaattatttttccctttgagggtcttttatacatctctcctccaaccccaccctctattctgtttcttcctcctcacatgggggtacacatacacagcttcctcttttggttccatccttaccaccacaccacacgcacactccacatgcccagcagagtggcacttggtggccagaaagtgtgagcctcatgatctgctgtctgtagttctgtgagctcaggtccctcaaaggcctcggagcacccccttccttgtgactgagccagggcctgcatttttggttttccccaccccacacattctcaaccatagtccttctaacaataccaatagctaggacccggctgctgtgcactgggactggggattccacatgtttgccttgggagtctcaagctggactgcca

SEQ ID NO: 77 - DNA, 2216 bp, synthetic construct
  source 1..2216: mol_type = other DNA
gtgctgcccgcctagaaagggtgaagtggttgtttccgtgacggactgagtacgggtgcctgtcaggctcttgcggaagtccatgcgccattgggagggcctcggccgcggctctgtgcccttgctgctgagggccacttcctgggtcattcctggaccgggagccgggctggggctcacacgggggctcccgcgtggccgtctcggcgcctgcgtgacctccccgccggcgggatgtggcgactacgtcgggccgctgtggcctgatgatgtatgctttgtttctgttgagtgtgggtttagtaatggggtttgtggggttttcttctaagccttctcctatttatgggggtttagtattgattgttagcggtgtggtcgggtgtgttattattctgaattttgggggaggttatatgggtttaatggtttttttaatttatttagggggaatgatggttgtctttggatatactacagcgatggctattgaggagtatcctgaggcatgggggtcaggggttgaggtcttggtgagtgttttagtggggttagcgatggaggtaggattggtgctgtgggtgaaagagtatgatggggtggtggttgtggtaaactttaatagtgtaggaagctggatgatttatgaaggagaggggtcagggttgattcgggaggatcctattggtgcgggggctttgtatgattatgggcgttggttagtagtagttactggttggacattgtttgttggtgtatatattgtaattgagattgctcgggggaattaggagcactgggacgcccaccgcccctttccctccgctgccaggcgagcatgttgtggtaattctggaacacaagaagagaaattgctgggtttagaacaagattataaacgaattcggtgctcagtgatcacttgacagttttttttttttttaaatattacccaaaatgctccccaaataagaaatgcatcagctcagtcagtgaatacaaaaaaggaattatttttccctttgagggtcttttatacatctctcctccaaccccaccctctattctgtttcttcctcctcacatgggggtacacatacacagcttcctcttttggttccatccttaccaccacaccacacgcacactccacatgcccagcagagtggcacttggtggccagaaagtgtgagcctcatgatctgctgtctgtagttctgtgagctcaggtccctcaaaggcctcggagcacccccttccttgtgactgagccagggcctgcatttttggttttccccaccccacacattctcaaccatagtccttctaacaataccaatagctaggacccggctgctgtgcactgggactggggattccacatgtttgccttgggagtctcaagctggactgccagcccctgtcctcccttcacccccattgcgtatgagcatttcagaactccaaggagtcacaggcatctttatagttcacgttaacatatagacactgttggaagcagttccttctaaaagggtagccctggacttaataccagccggatacctctggcccccaccccattactgtacctctggagtcactactgtgggtcgccactcctctgctacacagcacggctttttcaaggctgtattgagaagggaagttaggaagaagggtgtgctgggctaaccagcccacagagctcacattcctgtcccttgggtgaaaaatacatgtccatcctgatatctcctgaattcagaaattagcctccacatgtgcaatggctttaagagccagaagcagggttctgggaattttgcaagttacctgtggccaggtgtggtctcggttaccaaatacggttacctgcagctttttagtcctttgtgctcccacgggtctacagagtcccatctgcccaaaggtcttgaagcttgacaggatgttttcgattactcagtctcccagggcactactggtccgtaggattcgattggtcggggtaggagagttaaacaacatttaaacagagttctctcaaaaatgtctaaagggattgtaggtagataacatccaatcactgtttgcacttatctgaaatcttccctcttggctgcccccaggtatttactgtggagaacattgcataggaatgtctggaaaaagcttctacaacttgttacagccttcacatttgtagaagcttt

SEQ ID NO: 78 - DNA, 1416 bp, synthetic construct
  source 1..1416: mol_type = other DNA
gtgctgcccgcctagaaagggtgaagtggttgtttccgtgacggactgagtacgggtgcctgtcaggctcttgcggaagtccatgcgccattgggagggcctcggccgcggctctgtgcccttgctgctgagggccacttcctgggtcattcctggaccgggagccgggctggggctcacacgggggctcccgcgtggccgtctcggcgcctgcgtgacctccccgccggcgggatgtggcgactacgtcgggccgctgtggcctgatgatgtatgctttgtttctgttgagtgtgggtttagtaatggggtttgtggggttttcttctaagccttctcctatttatgggggtttagtattgattgttagcggtgtggtcgggtgtgttattattctgaattttgggggaggttatatgggtttaatggtttttttaatttatttagggggaatgatggttgtctttggatatactacagcgatggctattgaggagtatcctgaggcatgggggtcaggggttgaggtcttggtgagtgttttagtggggttagcgatggaggtaggattggtgctgtgggtgaaagagtatgatggggtggtggttgtggtaaactttaatagtgtaggaagctggatgatttatgaaggagaggggtcagggttgattcgggaggatcctattggtgcgggggctttgtatgattatgggcgttggttagtagtagttactggttggacattgtttgttggtgtatatattgtaattgagattgctcgggggaattaggagcactgggacgcccaccgcccctttccctccgctgccaggcgagcatgttgtggtaattctggaacacaagaagagaaattgctgggtttagaacaagattataaacgaattcggtgctcagtgatcacttgacagttttttttttttttaaatattacccaaaatgctccccaaataagaaatgcatcagctcagtcagtgaatacaaaaaaggaattatttttccctttgagggtcttttatacatctctcctccaaccccaccctctattctgtttcttcctcctcacatgggggtacacatacacagcttcctcttttggttccatccttaccaccacaccacacgcacactccacatgcccagcagagtggcacttggtggccagaaagtgtgagcctcatgatctgctgtctgtagttctgtgagctcaggtccctcaaaggcctcggagcacccccttccttgtgactgagccagggcctgcatttttggttttccccaccccacacattctcaaccatagtccttctaacaataccaatagctaggacccggctgctgtgcactgggactggggattccacatgtttgccttgggagtctcaagctggactgcca

SEQ ID NO: 79 - DNA, 2216 bp, synthetic construct
  source 1..2216: mol_type = other DNA
gtgctgcccgcctagaaagggtgaagtggttgtttccgtgacggactgagtacgggtgcctgtcaggctcttgcggaagtccatgcgccattgggagggcctcggccgcggctctgtgcccttgctgctgagggccacttcctgggtcattcctggaccgggagccgggctggggctcacacgggggctcccgcgtggccgtctcggcgcctgcgtgacctccccgccggcgggatgtggcgactacgtcgggccgctgtggcctgatgatgtacgccctgttcctgctgagcgtgggcctggtgatgggcttcgtgggcttcagcagcaagcccagccccatctacggcggcctggtgctgatcgtgagcggcgtggtgggctgcgtgatcatcctgaacttcggcggcggctacatgggcctgatggtgttcctgatctacctgggcggcatgatggtggtgttcggctacaccaccgccatggccatcgaggagtaccccgaggcctggggcagcggcgtggaggtgctggtgagcgtgctggtgggcctggccatggaggtgggcctggtgctgtgggtgaaggagtacgacggcgtggtggtggtggtgaacttcaacagcgtgggcagctggatgatctacgagggcgagggcagcggcctgatccgcgaggaccccatcggcgccggcgccctgtacgactacggccgctggctggtggtggtgaccggctggaccctgttcgtgggcgtgtacatcgtgatcgagatcgcccgcggcaactaagagcactgggacgcccaccgcccctttccctccgctgccaggcgagcatgttgtggtaattctggaacacaagaagagaaattgctgggtttagaacaagattataaacgaattcggtgctcagtgatcacttgacagttttttttttttttaaatattacccaaaatgctccccaaataagaaatgcatcagctcagtcagtgaatacaaaaaaggaattatttttccctttgagggtcttttatacatctctcctccaaccccaccctctattctgtttcttcctcctcacatgggggtacacatacacagcttcctcttttggttccatccttaccaccacaccacacgcacactccacatgcccagcagagtggcacttggtggccagaaagtgtgagcctcatgatctgctgtctgtagttctgtgagctcaggtccctcaaaggcctcggagcacccccttccttgtgactgagccagggcctgcatttttggttttccccaccccacacattctcaaccatagtccttctaacaataccaatagctaggacccggctgctgtgcactgggactggggattccacatgtttgccttgggagtctcaagctggactgccagcccctgtcctcccttcacccccattgcgtatgagcatttcagaactccaaggagtcacaggcatctttatagttcacgttaacatatagacactgttggaagcagttccttctaaaagggtagccctggacttaataccagccggatacctctggcccccaccccattactgtacctctggagtcactactgtgggtcgccactcctctgctacacagcacggctttttcaaggctgtattgagaagggaagttaggaagaagggtgtgctgggctaaccagcccacagagctcacattcctgtcccttgggtgaaaaatacatgtccatcctgatatctcctgaattcagaaattagcctccacatgtgcaatggctttaagagccagaagcagggttctgggaattttgcaagttacctgtggccaggtgtggtctcggttaccaaatacggttacctgcagctttttagtcctttgtgctcccacgggtctacagagtcccatctgcccaaaggtcttgaagcttgacaggatgttttcgattactcagtctcccagggcactactggtccgtaggattcgattggtcggggtaggagagttaaacaacatttaaacagagttctctcaaaaatgtctaaagggattgtaggtagataacatccaatcactgtttgcacttatctgaaatcttccctcttggctgcccccaggtatttactgtggagaacattgcataggaatgtctggaaaaagcttctacaacttgttacagccttcacatttgtagaagcttt

SEQ ID NO: 80 - DNA, 1416 bp, synthetic construct
  source 1..1416: mol_type = other DNA
gtgctgcccgcctagaaagggtgaagtggttgtttccgtgacggactgagtacgggtgcctgtcaggctcttgcggaagtccatgcgccattgggagggcctcggccgcggctctgtgcccttgctgctgagggccacttcctgggtcattcctggaccgggagccgggctggggctcacacgggggctcccgcgtggccgtctcggcgcctgcgtgacctccccgccggcgggatgtggcgactacgtcgggccgctgtggcctgatgatgtacgccctgttcctgctgagcgtgggcctggtgatgggcttcgtgggcttcagcagcaagcccagccccatctacggcggcctggtgctgatcgtgagcggcgtggtgggctgcgtgatcatcctgaacttcggcggcggctacatgggcctgatggtgttcctgatctacctgggcggcatgatggtggtgttcggctacaccaccgccatggccatcgaggagtaccccgaggcctggggcagcggcgtggaggtgctggtgagcgtgctggtgggcctggccatggaggtgggcctggtgctgtgggtgaaggagtacgacggcgtggtggtggtggtgaacttcaacagcgtgggcagctggatgatctacgagggcgagggcagcggcctgatccgcgaggaccccatcggcgccggcgccctgtacgactacggccgctggctggtggtggtgaccggctggaccctgttcgtgggcgtgtacatcgtgatcgagatcgcccgcggcaactaagagcactgggacgcccaccgcccctttccctccgctgccaggcgagcatgttgtggtaattctggaacacaagaagagaaattgctgggtttagaacaagattataaacgaattcggtgctcagtgatcacttgacagttttttttttttttaaatattacccaaaatgctccccaaataagaaatgcatcagctcagtcagtgaatacaaaaaaggaattatttttccctttgagggtcttttatacatctctcctccaaccccaccctctattctgtttcttcctcctcacatgggggtacacatacacagcttcctcttttggttccatccttaccaccacaccacacgcacactccacatgcccagcagagtggcacttggtggccagaaagtgtgagcctcatgatctgctgtctgtagttctgtgagctcaggtccctcaaaggcctcggagcacccccttccttgtgactgagccagggcctgcatttttggttttccccaccccacacattctcaaccatagtccttctaacaataccaatagctaggacccggctgctgtgcactgggactggggattccacatgtttgccttgggagtctcaagctggactgcca

SEQ ID NO: 81 - DNA, 2642 bp, synthetic construct
  source 1..2642: mol_type = other DNA
gtgctgcccgcctagaaagggtgaagtggttgtttccgtgacggactgagtacgggtgcctgtcaggctcttgcggaagtccatgcgccattgggagggcctcggccgcggctctgtgcccttgctgctgagggccacttcctgggtcattcctggaccgggagccgggctggggctcacacgggggctcccgcgtggccgtctcggcgcctgcgtgacctccccgccggcgggatgtggcgactacgtcgggccgctgtggcctgatggccaacctcctactcctcattgtacccattctaatcgcaatggcattcctaatgcttaccgaacgaaaaattctaggctatatgcaactacgcaaaggccccaacgttgtaggcccctacgggctactacaacccttcgctgacgccataaaactcttcaccaaagagcccctaaaacccgccacatctaccatcaccctctacatcaccgccccgaccttagctctcaccatcgctcttctactatggacccccctccccatgcccaaccccctggtcaacctcaacctaggcctcctatttattctagccacctctagcctagccgtttactcaatcctctggtcagggtgggcatcaaactcaaactacgccctgatcggcgcactgcgagcagtagcccaaacaatctcatatgaagtcaccctagccatcattctactatcaacattactaatgagtggctcctttaacctctccacccttatcacaacacaagaacacctctggttactcctgccatcatggcccttggccatgatgtggtttatctccacactagcagagaccaaccgaacccccttcgaccttgccgaaggggagtccgaactagtctcaggcttcaacatcgaatacgccgcaggccccttcgccctattcttcatggccgaatacacaaacattattatgatgaacaccctcaccactacaatcttcctaggaacaacatatgacgcactctcccctgaactctacacaacatattttgtcaccaagaccctacttctaacctccctgttcttatggattcgaacagcatacccccgattccgctacgaccaactcatgcacctcctatggaaaaacttcctaccactcaccctagcattacttatgtggtatgtctccatgcccattacaatctccagcattccccctcaaacctaagagcactgggacgcccaccgcccctttccctccgctgccaggcgagcatgttgtggtaattctggaacacaagaagagaaattgctgggtttagaacaagattataaacgaattcggtgctcagtgatcacttgacagttttttttttttttaaatattacccaaaatgctccccaaataagaaatgcatcagctcagtcagtgaatacaaaaaaggaattatttttccctttgagggtcttttatacatctctcctccaaccccaccctctattctgtttcttcctcctcacatgggggtacacatacacagcttcctcttttggttccatccttaccaccacaccacacgcacactccacatgcccagcagagtggcacttggtggccagaaagtgtgagcctcatgatctgctgtctgtagttctgtgagctcaggtccctcaaaggcctcggagcacccccttccttgtgactgagccagggcctgcatttttggttttccccaccccacacattctcaaccatagtccttctaacaataccaatagctaggacccggctgctgtgcactgggactggggattccacatgtttgccttgggagtctcaagctggactgccagcccctgtcctcccttcacccccattgcgtatgagcatttcagaactccaaggagtcacaggcatctttatagttcacgttaacatatagacactgttggaagcagttccttctaaaagggtagccctggacttaataccagccggatacctctggcccccaccccattactgtacctctggagtcactactgtgggtcgccactcctctgctacacagcacggctttttcaaggctgtattgagaagggaagttaggaagaagggtgtgctgggctaaccagcccacagagctcacattcctgtcccttgggtgaaaaatacatgtccatcctgatatctcctgaattcagaaattagcctccacatgtgcaatggctttaagagccagaagcagggttctgggaattttgcaagttacctgtggccaggtgtggtctcggttaccaaatacggttacctgcagctttttagtcctttgtgctcccacgggtctacagagtcccatctgcccaaaggtcttgaagcttgacaggatgttttcgattactcagtctcccagggcactactggtccgtaggattcgattggtcggggtaggagagttaaacaacatttaaacagagttctctcaaaaatgtctaaagggattgtaggtagataacatccaatcactgtttgcacttatctgaaatcttccctcttggctgcccccaggtatttactgtggagaacattgcataggaatgtctggaaaaagcttctacaacttgttacagccttcacatttgtagaagcttt

SEQ ID NO: 82 - DNA, 1842 bp, synthetic construct
  source 1..1842: mol_type = other DNA
gtgctgcccgcctagaaagggtgaagtggttgtttccgtgacggactgagtacgggtgcctgtcaggctcttgcggaagtccatgcgccattgggagggcctcggccgcggctctgtgcccttgctgctgagggccacttcctgggtcattcctggaccgggagccgggctggggctcacacgggggctcccgcgtggccgtctcggcgcctgcgtgacctccccgccggcgggatgtggcgactacgtcgggccgctgtggcctgatggccaacctcctactcctcattgtacccattctaatcgcaatggcattcctaatgcttaccgaacgaaaaattctaggctatatgcaactacgcaaaggccccaacgttgtaggcccctacgggctactacaacccttcgctgacgccataaaactcttcaccaaagagcccctaaaacccgccacatctaccatcaccctctacatcaccgccccgaccttagctctcaccatcgctcttctactatggacccccctccccatgcccaaccccctggtcaacctcaacctaggcctcctatttattctagccacctctagcctagccgtttactcaatcctctggtcagggtgggcatcaaactcaaactacgccctgatcggcgcactgcgagcagtagcccaaacaatctcatatgaagtcaccctagccatcattctactatcaacattactaatgagtggctcctttaacctctccacccttatcacaacacaagaacacctctggttactcctgccatcatggcccttggccatgatgtggtttatctccacactagcagagaccaaccgaacccccttcgaccttgccgaaggggagtccgaactagtctcaggcttcaacatcgaatacgccgcaggccccttcgccctattcttcatggccgaatacacaaacattattatgatgaacaccctcaccactacaatcttcctaggaacaacatatgacgcactctcccctgaactctacacaacatattttgtcaccaagaccctacttctaacctccctgttcttatggattcgaacagcatacccccgattccgctacgaccaactcatgcacctcctatggaaaaacttcctaccactcaccctagcattacttatgtggtatgtctccatgcccattacaatctccagcattccccctcaaacctaagagcactgggacgcccaccgcccctttccctccgctgccaggcgagcatgttgtggtaattctggaacacaagaagagaaattgctgggtttagaacaagattataaacgaattcggtgctcagtgatcacttgacagttttttttttttttaaatattacccaaaatgctccccaaataagaaatgcatcagctcagtcagtgaatacaaaaaaggaattatttttccctttgagggtcttttatacatctctcctccaaccccaccctctattctgtttcttcctcctcacatgggggtacacatacacagcttcctcttttggttccatccttaccaccacaccacacgcacactccacatgcccagcagagtggcacttggtggccagaaagtgtgagcctcatgatctgctgtctgtagttctgtgagctcaggtccctcaaaggcctcggagcacccccttccttgtgactgagccagggcctgcatttttggttttccccaccccacacattctcaaccatagtccttctaacaataccaatagctaggacccggctgctgtgcactgggactggggattccacatgtttgccttgggagtctcaagctggactgcca

SEQ ID NO: 83 - DNA, 2642 bp, synthetic construct
  source 1..2642: mol_type = other DNA
gtgctgcccgcctagaaagggtgaagtggttgtttccgtgacggactgagtacgggtgcctgtcaggctcttgcggaagtccatgcgccattgggagggcctcggccgcggctctgtgcccttgctgctgagggccacttcctgggtcattcctggaccgggagccgggctggggctcacacgggggctcccgcgtggccgtctcggcgcctgcgtgacctccccgccggcgggatgtggcgactacgtcgggccgctgtggcctgatggccaacctgctgctgctgatcgtgcccatcctgatcgccatggccttcctgatgctgaccgagcgcaagatcctgggctacatgcagctgcgcaagggccccaacgtggtgggcccctacggcctgctgcagcccttcgccgacgccatcaagctgttcaccaaggagcccctgaagcccgccaccagcaccatcaccctgtacatcaccgcccccaccctggccctgaccatcgccctgctgctgtggacccccctgcccatgcccaaccccctggtgaacctgaacctgggcctgctgttcatcctggccaccagcagcctggccgtgtacagcatcctgtggagcggctgggccagcaacagcaactacgccctgatcggcgccctgcgcgccgtggcccagaccatcagctacgaggtgaccctggccatcatcctgctgagcaccctgctgatgagcggcagcttcaacctgagcaccctgatcaccacccaggagcacctgtggctgctgctgcccagctggcccctggccatgatgtggttcatcagcaccctggccgagaccaaccgcacccccttcgacctggccgagggcgagagcgagctggtgagcggcttcaacatcgagtacgccgccggccccttcgccctgttcttcatggccgagtacaccaacatcatcatgatgaacaccctgaccaccaccatcttcctgggcaccacctacgacgccctgagccccgagctgtacaccacctacttcgtgaccaagaccctgctgctgaccagcctgttcctgtggatccgcaccgcctacccccgcttccgctacgaccagctgatgcacctgctgtggaagaacttcctgcccctgaccctggccctgctgatgtggtacgtgagcatgcccatcaccatcagcagcatccccccccagacctaagagcactgggacgcccaccgcccctttccctccgctgccaggcgagcatgttgtggtaattctggaacacaagaagagaaattgctgggtttagaacaagattataaacgaattcggtgctcagtgatcacttgacagttttttttttttttaaatattacccaaaatgctccccaaataagaaatgcatcagctcagtcagtgaatacaaaaaaggaattatttttccctttgagggtcttttatacatctctcctccaaccccaccctctattctgtttcttcctcctcacatgggggtacacatacacagcttcctcttttggttccatccttaccaccacaccacacgcacactccacatgcccagcagagtggcacttggtggccagaaagtgtgagcctcatgatctgctgtctgtagttctgtgagctcaggtccctcaaaggcctcggagcacccccttccttgtgactgagccagggcctgcatttttggttttccccaccccacacattctcaaccatagtccttctaacaataccaatagctaggacccggctgctgtgcactgggactggggattccacatgtttgccttgggagtctcaagctggactgccagcccctgtcctcccttcacccccattgcgtatgagcatttcagaactccaaggagtcacaggcatctttatagttcacgttaacatatagacactgttggaagcagttccttctaaaagggtagccctggacttaataccagccggatacctctggcccccaccccattactgtacctctggagtcactactgtgggtcgccactcctctgctacacagcacggctttttcaaggctgtattgagaagggaagttaggaagaagggtgtgctgggctaaccagcccacagagctcacattcctgtcccttgggtgaaaaatacatgtccatcctgatatctcctgaattcagaaattagcctccacatgtgcaatggctttaagagccagaagcagggttctgggaattttgcaagttacctgtggccaggtgtggtctcggttaccaaatacggttacctgcagctttttagtcctttgtgctcccacgggtctacagagtcccatctgcccaaaggtcttgaagcttgacaggatgttttcgattactcagtctcccagggcactactggtccgtaggattcgattggtcggggtaggagagttaaacaacatttaaacagagttctctcaaaaatgtctaaagggattgtaggtagataacatccaatcactgtttgcacttatctgaaatcttccctcttggctgcccccaggtatttactgtggagaacattgcataggaatgtctggaaaaagcttctacaacttgttacagccttcacatttgtagaagcttt

SEQ ID NO: 84 - DNA, 1842 bp, synthetic construct
  source 1..1842: mol_type = other DNA
gtgctgcccgcctagaaagggtgaagtggttgtttccgtgacggactgagtacgggtgcctgtcaggctcttgcggaagtccatgcgccattgggagggcctcggccgcggctctgtgcccttgctgctgagggccacttcctgggtcattcctggaccgggagccgggctggggctcacacgggggctcccgcgtggccgtctcggcgcctgcgtgacctccccgccggcgggatgtggcgactacgtcgggccgctgtggcctgatggccaacctgctgctgctgatcgtgcccatcctgatcgccatggccttcctgatgctgaccgagcgcaagatcctgggctacatgcagctgcgcaagggccccaacgtggtgggcccctacggcctgctgcagcccttcgccgacgccatcaagctgttcaccaaggagcccctgaagcccgccaccagcaccatcaccctgtacatcaccgcccccaccctggccctgaccatcgccctgctgctgtggacccccctgcccatgcccaaccccctggtgaacctgaacctgggcctgctgttcatcctggccaccagcagcctggccgtgtacagcatcctgtggagcggctgggccagcaacagcaactacgccctgatcggcgccctgcgcgccgtggcccagaccatcagctacgaggtgaccctggccatcatcctgctgagcaccctgctgatgagcggcagcttcaacctgagcaccctgatcaccacccaggagcacctgtggctgctgctgcccagctggcccctggccatgatgtggttcatcagcaccctggccgagaccaaccgcacccccttcgacctggccgagggcgagagcgagctggtgagcggcttcaacatcgagtacgccgccggccccttcgccctgttcttcatggccgagtacaccaacatcatcatgatgaacaccctgaccaccaccatcttcctgggcaccacctacgacgccctgagccccgagctgtacaccacctacttcgtgaccaagaccctgctgctgaccagcctgttcctgtggatccgcaccgcctacccccgcttccgctacgaccagctgatgcacctgctgtggaagaacttcctgcccctgaccctggccctgctgatgtggtacgtgagcatgcccatcaccatcagcagcatccccccccagacctaagagcactgggacgcccaccgcccctttccctccgctgccaggcgagcatgttgtggtaattctggaacacaagaagagaaattgctgggtttagaacaagattataaacgaattcggtgctcagtgatcacttgacagttttttttttttttaaatattacccaaaatgctccccaaataagaaatgcatcagctcagtcagtgaatacaaaaaaggaattatttttccctttgagggtcttttatacatctctcctccaaccccaccctctattctgtttcttcctcctcacatgggggtacacatacacagcttcctcttttggttccatccttaccaccacaccacacgcacactccacatgcccagcagagtggcacttggtggccagaaagtgtgagcctcatgatctgctgtctgtagttctgtgagctcaggtccctcaaaggcctcggagcacccccttccttgtgactgagccagggcctgcatttttggttttccccaccccacacattctcaaccatagtccttctaacaataccaatagctaggacccggctgctgtgcactgggactggggattccacatgtttgccttgggagtctcaagctggactgcca

SEQ ID NO: 85 - DNA, 18 bp, synthetic construct
  source 1..18: mol_type = other DNA
cgagatcgtgcgggacat

SEQ ID NO: 86 - DNA, 19 bp, synthetic construct
  source 1..19: mol_type = other DNA
caggaaggagggctggaac

SEQ ID NO: 87 - DNA, 19 bp, synthetic construct
  source 1..19: mol_type = other DNA
ctgcctacgacaaacagac

SEQ ID NO: 88 - DNA, 19 bp, synthetic construct
  source 1..19: mol_type = other DNA
agtgcgttcgtagtttgag

SEQ ID NO: 89 - DNA, 21 bp, synthetic construct
  source 1..21: mol_type = other DNA
atgatgtatgctttgtttctg

SEQ ID NO: 90 - DNA, 21 bp, synthetic construct
  source 1..21: mol_type = other DNA
ctaattcccccgagcaatctc

SEQ ID NO: 91 - DNA, 18 bp, synthetic construct
  source 1..18: mol_type = other DNA
agtgtgggtttagtaatg

SEQ ID NO: 92 - DNA, 18 bp, synthetic construct
  source 1..18: mol_type = other DNA
tgcctcaggatactcctc

SEQ ID NO: 93 - DNA, 20 bp, synthetic construct
  source 1..20: mol_type = other DNA
ctccatcctggcctcgctgt

SEQ ID NO: 94 - DNA, 20 bp, synthetic construct
  source 1..20: mol_type = other DNA
gctgtcaccttcaccgttcc

SEQ ID NO: 95 - DNA, 23 bp, synthetic construct
  source 1..23: mol_type = other DNA
gggttttcttctaagccttctcc

SEQ ID NO: 96 - DNA, 23 bp, synthetic construct
  source 1..23: mol_type = other DNA
ccatcatactctttcacccacag

SEQ ID NO: 97 - DNA, 20 bp, synthetic construct
  source 1..20: mol_type = other DNA
cgcctgctgaccggctgcgt

SEQ ID NO: 98 - DNA, 20 bp, synthetic construct
  source 1..20: mol_type = other DNA
ccaggcctcggggtactcct

SEQ ID NO: 99 - DNA, 21 bp, synthetic construct
  source 1..21: mol_type = other DNA
atggccgcatctccgcacact

SEQ ID NO: 100 - DNA, 21 bp, synthetic construct
  source 1..21: mol_type = other DNA
ttaggtttgagggggaatgct

SEQ ID NO: 101 - DNA, 21 bp, synthetic construct
  source 1..21: mol_type = other DNA
aacctcaacctaggcctccta

SEQ ID NO: 102 - DNA, 21 bp, synthetic construct
  source 1..21: mol_type = other DNA
tggcaggagtaaccagaggtg

SEQ ID NO: 103 - DNA, 23 bp, synthetic construct
  source 1..23: mol_type = other DNA
aggaggctctgtctggtatcttg

SEQ ID NO: 104 - DNA, 21 bp, synthetic construct
  source 1..21: mol_type = other DNA
ttttaggggctctttggtgaa

SEQ ID NO: 105 - DNA, 22 bp, synthetic construct
  source 1..22: mol_type = other DNA
gccgcctgctgaccggctgcgt

SEQ ID NO: 106 - DNA, 24 bp, synthetic construct
  source 1..24: mol_type = other DNA
tgatgtacagggtgatggtgctgg

SEQ ID NO: 107 - DNA, 19 bp, synthetic construct
  source 1..19: mol_type = other DNA
gccaacagcaactacgagc

SEQ ID NO: 108 - DNA, 20 bp, synthetic construct
  source 1..20: mol_type = other DNA
tgatgttgctccagctgaag

SEQ ID NO: 109 - DNA, 20 bp, synthetic construct
  source 1..20: mol_type = other DNA
gcctgaccctgatcctgaac

SEQ ID NO: 110 - DNA, 20 bp, synthetic construct
  source 1..20: mol_type = other DNA
gtgcgctcgtagttgctgtt

SEQ ID NO: 111 - DNA, 376 bp, synthetic construct
  source 1..376: mol_type = other DNA
gggcagtgcctccccgccccgccgctggcgtcaagttcagctccacgtgtgccatcagtggatccgatccgtccagccatggcttcctattccaagatggtgtgaccagacatgcttcctgctccccgcttagcccacggagtgactgtggttgtggtgggggggttcttaaaataactttttagcccccgtcttcctattttgagtttggttcagatcttaagcagctccatgcaactgtatttatttttgatgacaagactcccatctaaagtttttctcctgcctgatcatttcattggtggctgaaggattctagagaaccttttgttcttgcaaggaaaacaagaatccaaaaccagtgactgttctgtga

SEQ ID NO: 112 - DNA, 146 bp, synthetic construct
  source 1..146: mol_type = other DNA
ggggtctttgtcctctgtactgtctctctccttgcccctaacccaaaaagcttcatttttctgtgtaggctgcacaagagccttgattgaagatatattctttctgaacagtatttaaggtttccaataaaatgtacacccctcag

SEQ ID NO: 113 - DNA, 1956 bp, synthetic construct
  source 1..1956: mol_type = other DNA
tgttgggtccaagaaggaatttctttccatccctgtgaggcaatgggtgggaatgataggacaggcaaagagaagcttcctcaggctagcaaaaatatcatttgatgtattgattaaaaaagcacttgcttgatgtatctttggcgtgtgtgctactctcatctgtgtgtatgtgtgttgtgtgtgtgtgtgtgtgcatgcacatatgtgttcactctgctactttgtaagttttaggctaggttgctttaccagctgtttacttcttttttgttgttgttttgagacaaggtttcgctctgccaccctggctggagtgcagtggcgtgatcttggctcacggcaacctctgcctcctggggctcaagcaattatcccacctcagcctcctgagcagctgggactacaggtgcatgccacaacacctggctgatatttgtattttttgtagagacaggattttgccaagttgcccaggctggtcttgaactcctaggcttaagcaatccacccaccttggcctcctgaagtgccaggatcacagacgtgagccactacacccagcccagctgtttacttctttaaccatacttttgattttattttttgaccaaaatgaactaacccaggtaatcttccagggaccgcaattccagaacctcatagtatttcttccatttccagcagctgattagaagtccaggatcatgtgaagtcaggcagggtcacagttcctgatggcacattatggacagagaattccattttgttttctaacccatgatgaaaacccacgtgagtcagtgtgtgaacagggatcattaattttttccccctaggtggaaggaaaaaggcacttactttgcaggttacagaaattactgggagaggatatcgtcataaaaagagccaggccaaattggaatatttttgtgatctgcatcatgatgctgaaaatagcaattatttgggaattgggtttgaaaactgaattgttgccagagaattaaaccaggtgaaaggtccttttgaattcagattgtcttctgaacatccaggctgatcatctgagagcagtcaaatctacttccccaaaaagagaccagggtaggtttatttgcttttatttttaatgtttgcctgtgtttccaagtgtgaacaaaacagtgtgtgatctattcttggattcattttgatcagtatttattcaaacccagtctctctccaggacataaaactgaaatcagatatgttctttttaagcccaaaccctctcctttctagatccaacccttcacccctaattttatgatggctatagccatggacttccccaagaaaagatcacccagaaataagaccacctgtgacagttaccagcttttattcataaccttagcttcccaactattgagcattttctaaggtccctgctgtcttttggtctctggtttgatttgtggcaaacagatgaagtaacagactgctatgaaggaccacaaaaacggcagcctctggaaaaaccattagaaagtcagtggcagatccagtaaataatatcgccagcctcagcataatctgctgctgactcgattcagtggactctaaagtgcccagcctcctgacctgagctctcctgccatctgtgagactaccagaggtcttatctgctgtccacatggcaactgggcatgagtacctggccaccttgcttccctctttgcctggtccaagtgagtgtctgctgcctctgtcctgccttgttttcctggctctaaaccaactccacccactcttaatggaaactcagtctggctttgtgtgtttctgggaagcacatgacttctgggaatgggcaaggaagaggagtgaaacaaaaactgtcagctatgtgtgcctggtctgggatccttctctgggtgacagtggcatcatgaatcttagaatcagctcccc

SEQ ID NO: 114 - DNA, 411 bp, synthetic construct
  source 1..411: mol_type = other DNA
gaatcatgcaagcttcctccctcagccattgatggaaagttcagcaagatcagcaacaaaaccaagaaaaatgatccttgcgtgctgaatatctgaaaagagaaatttttcctacaaaatctcttgggtcaagaaagttctagaatttgaattgataaacatggtgggttggctgagggtaagagtatatgaggaaccttttaaacgacaacaatactgctagctttcaggatgatttttaaaaaatagattcaaatgtgttatcctctctctgaaacgcttcctataactcgagtttataggggaagaaaaagctattgtttacaattatatcaccattaaggcaactgctacaccctgctttgtattctgggctaagattcattaaaaactagctgctcttaacttaca

SEQ ID NO: 115 - DNA, 1465 bp, synthetic construct
  source 1..1465: mol_type = other DNA
gagcactgggacgcccaccgcccctttccctccgctgccaggcgagcatgttgtggtaattctggaacacaagaagagaaattgctgggtttagaacaagattataaacgaattcggtgctcagtgatcacttgacagttttttttttttttaaatattacccaaaatgctccccaaataagaaatgcatcagctcagtcagtgaatacaaaaaaggaattatttttccctttgagggtctttatacatctctcctccaaccccaccctctattctgtttcttcctcctcacatgggggtacacatacacagcttcctcttttggttccatccttaccaccacaccacacgcacactccacatgcccagcagagtggcacttggtggccagaaagtgtgagcctcatgatctgctgtctgtagttctgtgagctcaggtccctcaaaggcctcggagcacccccttcctggtgactgagccagggcctgcatttttggttttccccaccccacacattctcaaccatagtccttctaacaataccaatagctaggacccggctgctgtgcactgggactggggattccacatgtttgccttgggagtctcaagctggactgccagcccctgtcctcccttcacccccattgcgtatgagcatttcagaactccaaggagtcacaggcatctttatagttcacgttaacatatagacactgttggaagcagttccttctaaaagggtagccctggacttaataccagccggatacctctggcccccaccccattactgtacctctggagtcactactgtgggtcgccactcctctgctacacagcacggctttttcaaggctgtattgagaagggaagttaggaagaagggtgtgctgggctaaccagcccacagagctcacattcctgtcccttgggtgaaaaatacatgtccatcctgatatctcctgaattcagaaattagcctccacatgtgcaatggctttaagagccagaagcagggttctgggaattttgcaagttatcctgtggccaggtgtggtctcggttaccaaatacggttacctgcagctttttagtcctttgtgctcccacgggtctgcagagtcccatctgcccaaaggtcttgaagcttgacaggatgttttcattactcagtctcccagggcactgctggtccgtagggattcattggtcggggtgggagagttaaacaacatttaaacagagttctctcaaaaatgtctaaagggattgtaggtagataacatccaatcactgtttgcacttatctgaaatcttccctcttggctgcccccaggtatttactgtggagaacattgcataggaatgtctggaaaaagcctctacaacttgttacagccttcacatttgtacaattcattgattctcttttccttccacaataaaatggtatacaagaac

SEQ ID NO: 116 - DNA, 288 bp, synthetic construct
  source 1..288: mol_type = other DNA
gagacttggactcaagtcataggcttctttcagtctttatgtcacctcaggagacttatttgagaggaagccttctgtacttgaagttgatttgaaatatgtaagaattgatgatgtatttgcaaacattaatgtgaaataaattgaatttaatgttgaatactttcaggcattcacttaataaagacactgttaagcactgttatgctcagtcatacacgcgaaaggtacaatgtcttttagctaattctaattaaaaattacagactggtgtacaagatacttgtg

SEQ ID NO: 117 - DNA, 83 bp, synthetic construct
  source 1..83: mol_type = other DNA
cccaccaccctggcctgctgtcctgcgtctatccatgtggaatgctggacaataaagcgagtgctgcccaccctccagctgcc

SEQ ID NO: 118 - DNA, 66 bp, synthetic construct
  source 1..66: mol_type = other DNA
tttatattgaactgtaaatatgtcactagagaaataaaatatggacttccaatctacgtaaactta

SEQ ID NO: 119 - DNA, 214 bp, synthetic construct
  source 1..214: mol_type = other DNA
accacgatcgttatgctgagtatgttaagctctttatgactgtttttgtagtggtatagagtactgcagaatacagtaagctgctctattgtagcatttcttgatgttgcttagtcacttatttcataaacaacttaatgttctgaataatttcttactaaacattttgttattgggcaagtgattgaaaatagtaaatgctttgtgtgattga

SEQ ID NO: 120 - DNA, 286 bp, synthetic construct
  source 1..286: mol_type = other DNA
tcttggaatataaagaatttcttcaggttgaattacctagaagtttgtcactgacttgtgttcctgaactatgacacatgaatatgtgggctaagaaatagttcctcttgataaataaacaattaacaaatactttggacagtaagtctttctcagttcttaatgataatgcagggcacttactagcataagaattggtttgggatttaactgtttatgaagctaacttgatttccgtgttttgttaaaatttcattgttctagcacatctttaactgtgatagtt

SEQ ID NO: 121 - DNA, 721 bp, synthetic construct
  source 1..721: mol_type = other DNA
gagacgtgcacttggtcgtgcgcccagggaggaagccgcaccaccagccagcgcaggccctggtggagaggcctccctggctgcctctgggaggggtgctgccttgtagatggagcaagtgagcactgagggtctggtgccaatcctgtaggcacaaaaccagaagtttctacattctctatttttgttaatcatcttctctttttccagaatttggaagctagaatggtgggaatgtcagtagtgccagaaagagagaaccaagcttgtctttaaagttactgatcacaggacgttgctttttcactgtttcctattaatcttcagctgaacacaagcaaaccttctcaggaggtgtctcctaccctcttattgttcctcttacgctctgctcaatgaaaccttcctcttgagggtcattttcctttctgtattaattataccagtgttaagtgacatagataagaactttgcacacttcaaatcagagcagtgattctctcttctctccccttttccttcagagtgaatcatccagactcctcatggataggtcgggtgttaaagttgttttgattatgtaccttttgatagatccacataaaaagaaatgtgaagttttcttttactatcttttcatttatcaagcagagacctttgttgggaggcggtttgggagaacacatttctaatttgaatgaaatgaaatctattttcagtg

SEQ ID NO: 122 - DNA, 163 bp, synthetic construct
  source 1..163: mol_type = other DNA
cagaagaagtgacggctgggggcacagtgggctgggcgcccctgcagaacatgaaccttccgctcctggctgccacagggtcctccgatgctggcctttgcgcctctagaggcagccactcatggattcaagtcctggctccgcctcttccatcaggaccact

SEQ ID NO: 123 - DNA, 60 bp, synthetic construct
  source 1..60: mol_type = other DNA
agaggacacactctgcacccccccaccccacgaccttggcccgagcccctccgtgaggaa

SEQ ID NO: 124 - DNA, 65 bp, synthetic construct
  source 1..65: mol_type = other DNA
agcccttccgccaggctgtgtgtcaggcccgtggtgggtgttttgtagtagtgtagagcattgca

SEQ ID NO: 125 - DNA, 231 bp, synthetic construct
  source 1..231: mol_type = other DNA
cttatgttctgtgcgcattctggcaggaattctgtctcttcagagactcatcctcaaaacaagacttgacactgtgtccttgccccagtcctaggaactgtggcacacagagatgttcattttaaaaacggatttcatgaaacactcttgtacttatgtttataagagagcactgggtagccaagtgatcttcccattcacagagttagtaaacctctgtactacatgctg

SEQ ID NO: 126 - protein, 28 aa, synthetic construct
MAASPHTLSSRLLTGCVGGSVWYLERRT

SEQ ID NO: 127 - protein, 29 aa, synthetic construct
MSVLTRLLLRGLTRLGSAAPVRRARIHSL

SEQ ID NO: 128 - protein, 10 aa, synthetic construct
MWRLRRAAVA

SEQ ID NO: 129 - protein, 28 aa, synthetic construct
MAASPHTLSSRLLTGCVGGSVWYLERRT

SEQ ID NO: 130 - protein, 122 aa, synthetic construct
MAFKSFIYSKGYHRSAAQKKTATSFFDSSYQYLRQNQGLVNSDPVLHASHLHPHPVVVANVNYNNVDDILHPHDLDSSINNTNNPLTHEELLYNQNVSLRSLKQQQSTNYVNNNNNNQHRYY

SEQ ID NO: 131 - protein, 174 aa, synthetic construct
MRKRSLRCHLWSANASLSPRKDEVTSRKESENLVKGKKNKKSHLHLLLFTASKIGTDSVFDVQKSKECCKELGLLFTSLIHSIGSFPFDEEPKAAAVFLPGSLPQLTVLVLAPGSGSCPTGKSTPHLAASGRNAELLRPQNSMIVRQFTCRGTISSHLCAHLRKPHDSRNMARP

SEQ ID NO: 132 - protein, 56 aa, synthetic construct
MLRRTSFNFTGRAMISRGSPEWSHRLDLKKGKKTTMMHKLGTSKPNNALQYAQMTL

SEQ ID NO: 133 - protein, 46 aa, synthetic construct
MISRSALSRGSQLALRRPAAAKTAQRGFAAAAASPAASYEPTTIAG

SEQ ID NO: 134 - protein, 128 aa, synthetic construct
MPELILYVAITLSVAERLVGPGHACAEPSFRSSRCSAPLCLLCSGSSSPATAPHPLKMFACSKFVSTPSLVKSTSQLLSRPLSAVVLKRPEILTDESLSSLAVSCPLTSLVSSRSFQTSAISRDIDTA

SEQ ID NO: 135 - protein, 115 aa, synthetic construct
MYRLMSAVTARAAAPGGLASSCGRRGVHQRAGLPPLGHGWVGGLGLGLGLALGVKLAGGLRGAAPAQSPAAPDPEASPLAEPPQEQSLAPWSPQTPAPPCSRCFARAIESSRDLL

SEQ ID NO: 136 - protein, 140 aa, synthetic construct
MTVLAPLRRLHTRAAFSSYGREIALQKRFLNLNSCSAVRRYGTGFSNNLRIKKLKNAFGVVRANSTKSTSTVTTASPIKYDSSFVGKTGGEIFHDMMLKHNVKHVFGYPGGAILPVFDAIYRSPHFEFILPRHEQAAGHA

SEQ ID NO: 137 - protein, 125 aa, synthetic construct
MILCPLEAFIVQHILTISVMGLLSCFRSTVLRKCSKGSSGMSRFLYTNNFQRNLISSGGNESYYGYFNRRSYTSLYMGTGTVGGITSARIRVPNVGCEGFMCSSHLSITQRNSRLIHSTSKIVPN

SEQ ID NO: 138 - protein, 107 aa, synthetic construct
MALQQAAPRVFGLLGRAPVALGQSGILTGSSGFKNQGFNGSLQSVENHVYAQAFSTSSQEEQAAPSIQGASGMKLPGMAGSMLLGKSRSGLRTGSMVPFAAQQAMNM

SEQ ID NO: 139 - protein, 87 aa, synthetic construct
MWRLRRAAVACEVCQSLVKHSSGIKGSLPLQKLHLVSRSIYHSHHPTLKLQRPQLRTSFQQFSSLTNLPLRKLKFSPIKYGYQPRRN

SEQ ID NO: 140 - protein, 56 aa, synthetic construct
MAVLWRLSAVCGALGGRALLLRTPVVRPAHISAFLQDRPIPEWCGVQHIHLSPSHH

SEQ ID NO: 141 - protein, 162 aa, synthetic construct
MAAILGDTIMVAKGLVKLTQAAVETHLQHLGIGGELIMAARALQSTAVEQIGMFLGKVQGQDKHEEYFAENFGGPEGEFHFSVPHAAGASTDFSSASAPDQSAPPSLGHAHSEGPAPAYVASGPFREAGFPGQASSPLGRANGRLFANPRDSFSAMGFQRRF

SEQ ID NO: 142 - protein, 117 aa, synthetic construct
MALLLRHSPKLRRAHAILGCERGTVVRHFSSSTCSSLVKEDTVSSSNLHPEYAKKIGGSDFSHDRQSGKELQNFKVSPQEASRASNFMRASKYGMPITANGVHSLFSCGQVVPSRCF

SEQ ID NO: 143 - protein, 66 aa, synthetic construct
MASTRVLASRLASQMAASAKVARPAVRVAQVSKRTIQTGSPLQTLKRTQMTSIVNATTRQAFQKRA

SEQ ID NO: 144 - protein, 44 aa, synthetic construct
MLAARLVCLRTLPSRVFHPAFTKASPVVKNSITKNQWLLTPSRE

SEQ ID NO: 145 - protein, 68 aa, synthetic construct
MASRVLSAYVSRLPAAFAPLPRVRMLAVARPLSTALCSAGTQTRLGTLQPALVLAQVPGRVTQLCRQY

SEQ ID NO: 146 - protein, 67 aa, synthetic construct
MFACAKLACTPSLIRAGSRVAYRPISASVLSRPEASRTGEGSTVFNGAQNGVSQLIQREFQTSAISR

SEQ ID NO: 147 - protein, 273 aa, synthetic construct
MALQQAAPRVFGLLGRAPVALGQSGILTGSSGFKNQGFNGSLQSVENHVYAQAFSTSSQEEQAAPSIQGASGMKLPGMAGSMLLGKSRSGLRTGSMVPFAAQQAMNMGGMAAILGDTIMVAKGLVKLTQAAVETHLQHLGIGGELIMAARALQSTAVEQIGMFLGKVQGQDKHEEYFAENFGGPEGEFHFSVPHAAGASTDFSSASAPDQSAPPSLGHAHSEGPAPAYVASGPFREAGFPGQASSPLGRANGRLFANPRDSFSAMGFQRRFGG

SEQ ID NO: 148 - protein, 132 aa, synthetic construct
MASTRVLASRLASQMAASAKVARPAVRVAQVSKRTIQTGSPLQTLKRTQMTSIVNATTRQAFQKRAMASTRVLASRLASQMAASAKVARPAVRVAQVSKRTIQTGSPLQTLKRTQMTSIVNATTRQAFQKRA

SEQ ID NO: 149 - protein, 119 aa, synthetic construct
MALLRAAVSELRRRGRGALTPLPALSSLLSSLSPRSPASTRPEPNNPHADRRHVIALRRCPPLPASAVLAPELLHARGLLPRHWSHASPLSTSSSSSRPADKAQLTWVDKWIPEAARPY

SEQ ID NO: 150 - protein, 391 aa, synthetic construct
MASTRVLASRLASQMAASAKVARPAVRVAQVSKRTIQTGSPLQTLKRTQMTSIVNATTRQAFQKRAMALLRAAVSELRRRGRGALTPLPALSSLLSSLSPRSPASTRPEPNNPHADRRHVIALRRCPPLPASAVLAPELLHARGLLPRHWSHASPLSTSSSSSRPADKAQLTWVDKWIPEAARPYMTVLAPLRRLHTRAAFSSYGREIALQKRFLNLNSCSAVRRYGTGFSNNLRIKKLKNAFGVVRANSTKSTSTVTTASPIKYDSSFVGKTGGEIFHDMMLKHNVKHVFGYPGGAILPVFDAIYRSPHFEFILPRHEQAAGHAMASTRVLASRLASQMAASAKVARPAVRVAQVSKRTIQTGSPLQTLKRTQMTSIVNATTRQAFQKRA

SEQ ID NO: 151 - protein, 455 aa, synthetic construct
MALLRAAVSELRRRGRGALTPLPALSSLLSSLSPRSPASTRPEPNNPHADRRHVIALRRCPPLPASAVLAPELLHARGLLPRHWSHASPLSTSSSSSRPADKAQLTWVDKWIPEAARPYMAAILGDTIMVAKGLVKLTQAAVETHLQHLGIGGELIMAARALQSTAVEQIGMFLGKVQGQDKHEEYFAENFGGPEGEFHFSVPHAAGASTDFSSASAPDQSAPPSLGHAHSEGPAPAYVASGPFREAGFPGQASSPLGRANGRLFANPRDSFSAMGFQRRFMALQQAAPRVFGLLGRAPVALGQSGILTGSSGFKNQGFNGSLQSVENHVYAQAFSTSSQEEQAAPSIQGASGMKLPGMAGSMLLGKSRSGLRTGSMVPFAAQQAMNMMFACAKLACTPSLIRAGSRVAYRPISASVLSRPEASRTGEGSTVFNGAQNGVSQLIQREFQTSAISR

SEQ ID NO: 152 - protein, 348 aa, synthetic construct
MALLRAAVSELRRRGRGALTPLPALSSLLSSLSPRSPASTRPEPNNPHADRRHVIALRRCPPLPASAVLAPELLHARGLLPRHWSHASPLSTSSSSSRPADKAQLTWVDKWIPEAARPYMAAILGDTIMVAKGLVKLTQAAVETHLQHLGIGGELIMAARALQSTAVEQIGMFLGKVQGQDKHEEYFAENFGGPEGEFHFSVPHAAGASTDFSSASAPDQSAPPSLGHAHSEGPAPAYVASGPFREAGFPGQASSPLGRANGRLFANPRDSFSAMGFQRRFMFACAKLACTPSLIRAGSRVAYRPISASVLSRPEASRTGEGSTVFNGAQNGVSQLIQREFQTSAISR

SEQ ID NO: 153 - protein, 185 aa, synthetic construct
MASTRVLASRLASQMAASAKVARPAVRVAQVSKRTIQTGSPLQTLKRTQMTSIVNATTRQAFQKRAMALLRAAVSELRRRGRGALTPLPALSSLLSSLSPRSPASTRPEPNNPHADRRHVIALRRCPPLPASAVLAPELLHARGLLPRHWSHASPLSTSSSSSRPADKAQLTWVDKWIPEAARPY

SEQ ID NO: 154 - protein, 455 aa, synthetic construct
MAAILGDTIMVAKGLVKLTQAAVETHLQHLGIGGELIMAARALQSTAVEQIGMFLGKVQGQDKHEEYFAENFGGPEGEFHFSVPHAAGASTDFSSASAPDQSAPPSLGHAHSEGPAPAYVASGPFREAGFPGQASSPLGRANGRLFANPRDSFSAMGFQRRFMALLRAAVSELRRRGRGALTPLPALSSLLSSLSPRSPASTRPEPNNPHADRRHVIALRRCPPLPASAVLAPELLHARGLLPRHWSHASPLSTSSSSSRPADKAQLTWVDKWIPEAARPYMALQQAAPRVFGLLGRAPVALGQSGILTGSSGFKNQGFNGSLQSVENHVYAQAFSTSSQEEQAAPSIQGASGMKLPGMAGSMLLGKSRSGLRTGSMVPFAAQQAMNMMFACAKLACTPSLIRAGSRVAYRPISASVLSRPEASRTGEGSTVFNGAQNGVSQLIQREFQTSAISR

SEQ ID NO: 155 - protein, 455 aa, synthetic construct
MALQQAAPRVFGLLGRAPVALGQSGILTGSSGFKNQGFNGSLQSVENHVYAQAFSTSSQEEQAAPSIQGASGMKLPGMAGSMLLGKSRSGLRTGSMVPFAAQQAMNMMAAILGDTIMVAKGLVKLTQAAVETHLQHLGIGGELIMAARALQSTAVEQIGMFLGKVQGQDKHEEYFAENFGGPEGEFHFSVPHAAGASTDFSSASAPDQSAPPSLGHAHSEGPAPAYVASGPFREAGFPGQASSPLGRANGRLFANPRDSFSAMGFQRRFMALLRAAVSELRRRGRGALTPLPALSSLLSSLSPRSPASTRPEPNNPHADRRHVIALRRCPPLPASAVLAPELLHARGLLPRHWSHASPLSTSSSSSRPADKAQLTWVDKWIPEAARPYMFACAKLACTPSLIRAGSRVAYRPISASVLSRPEASRTGEGSTVFNGAQNGVSQLIQREFQTSAISR

SEQ ID NO: 156 - protein, 285 aa, synthetic construct
MAAILGDTIMVAKGLVKLTQAAVETHLQHLGIGGELIMAARALQSTAVEQIGMFLGKVQGQDKHEEYFAENFGGPEGEFHFSVPHAAGASTDFSSASAPDQSAPPSLGHAHSEGPAPAYVASGPFREAGFPGQASSPLGRANGRLFANPRDSFSAMGFQRRFGGMALLRAAVSELRRRGRGALTPLPALSSLLSSLSPRSPASTRPEPNNPHADRRHVIALRRCPPLPASAVLAPELLHARGLLPRHWSHASPLSTSSSSSRPADKAQLTWVDKWIPEAARPYGG

SEQ ID NO: 157 - protein, 394 aa, synthetic construct
MAAILGDTIMVAKGLVKLTQAAVETHLQHLGIGGELIMAARALQSTAVEQIGMFLGKVQGQDKHEEYFAENFGGPEGEFHFSVPHAAGASTDFSSASAPDQSAPPSLGHAHSEGPAPAYVASGPFREAGFPGQASSPLGRANGRLFANPRDSFSAMGFQRRFGGMALLRAAVSELRRRGRGALTPLPALSSLLSSLSPRSPASTRPEPNNPHADRRHVIALRRCPPLPASAVLAPELLHARGLLPRHWSHASPLSTSSSSSRPADKAQLTWVDKWIPEAARPYGGMALQQAAPRVFGLLGRAPVALGQSGILTGSSGFKNQGFNGSLQSVENHVYAQAFSTSSQEEQAAPSIQGASGMKLPGMAGSMLLGKSRSGLRTGSMVPFAAQQAMNMGG

SEQ ID NO: 158 - protein, 574 aa, synthetic construct
MASTRVLASRLASQMAASAKVARPAVRVAQVSKRTIQTGSPLQTLKRTQMTSIVNATTRQAFQKRAMALLRAAVSELRRRGRGALTPLPALSSLLSSLSPRSPASTRPEPNNPHADRRHVIALRRCPPLPASAVLAPELLHARGLLPRHWSHASPLSTSSSSSRPADKAQLTWVDKWIPEAARPYMTVLAPLRRLHTRAAFSSYGREIALQKRFLNLNSCSAVRRYGTGFSNNLRIKKLKNAFGVVRANSTKSTSTVTTASPIKYDSSFVGKTGGEIFHDMMLKHNVKHVFGYPGGAILPVFDAIYRSPHFEFILPRHEQAAGHAVSGEGDATYGKLTLKFICTTGKLPVPWPTLVTTLTYGVQCFSRYPDHMKQHDFFKSAMPEGYVQERTIFFKDDGNYKTRAEVKFEGDTLVNRIELKGIDFKEDGNILGHKLEYNYNSHNVYIMADKQKNGIKVNFKIRHNIEDGSVQLADHYQQNTPIGDGPVLLPDNHYLSTQSALSKDPNEMASTRVLASRLASQMAASAKVARPAVRVAQVSKRTIQTGSPLQTLKRTQMTSIVNATTRQAFQKRA

SEQ ID NO: 159 - protein, 810 aa, synthetic construct
MASTRVLASRLASQMAASAKVARPAVRVAQVSKRTIQTGSPLQTLKRTQMTSIVNATTRQAFQKRAMALLRAAVSELRRRGRGALTPLPALSSLLSSLSPRSPASTRPEPNNPHADRRHVIALRRCPPLPASAVLAPELLHARGLLPRHWSHASPLSTSSSSSRPADKAQLTWVDKWIPEAARPYMTVLAPLRRLHTRAAFSSYGREIALQKRFLNLNSCSAVRRYGTGFSNNLRIKKLKNAFGVVRANSTKSTSTVTTASPIKYDSSFVGKTGGEIFHDMMLKHNVKHVFGYPGGAILPVFDAIYRSPHFEFILPRHEQAAGHAMRKRSLRCHLWSANASLSPRKDEVTSRKESENLVKGKKNKKSHLHLLLFTASKIGTDSVFDVQKSKECCKELGLLFTSLIHSIGSFPFDEEPKAAAVFLPGSLPQLTVLVLAPGSGSCPTGKSTPHLAASGRNAELLRPQNSMIVRQFTCRGTISSHLCAHLRKPHDSRNMARPMALLLRHSPKLRRAHAILGCERGTVVRHFSSSTCSSLVKEDTVSSSNLHPEYAKKIGGSDFSHDRQSGKELQNFKVSPQEASRASNFMRASKYGMPITANGVHSLFSCGQVVPSRCFMPELILYVAITLSVAERLVGPGHACAEPSFRSSRCSAPLCLLCSGSSSPATAPHPLKMFACSKFVSTPSLVKSTSQLLSRPLSAVVLKRPEILTDESLSSLAVSCPLTSLVSSRSFQTSAISRDIDTAMASTRVLASRLASQMAASAKVARPAVRVAQVSKRTIQTGSPLQTLKRTQMTSIVNATTRQAFQKRA

SEQ ID NO: 160 - protein, 459 aa, synthetic construct
MLKLIVPTIMLLPLTWLSKKHMIWINTTTHSLIISIIPLLFFNQINNNLFSCSPTFSSDPLTTPLLMLTTWLLPLTIMASQRHLSSEPLSRKKLYLSMLISLQISLIMTFTATELIMFYIFFETTLIPTLAIITRWGNQPERLNAGTYFLFYTLVGSLPLLIALIYTHNTLGSLNILLLTLTAQELSNSWANNLMWLAYTMAFMVKMPLYGLHLWLPKAHVEAPIAGSMVLAAVLLKLGGYGMMRLTLILNPLTKHMAYPFLVLSLWGMIMTSSICLRQTDLKSLIAYSSISHMALVVTAILIQTPWSFTGAVILMIAHGLTSSLLFCLANSNYERTHSRIMILSQGLQTLLPLMAFWWLLASLANLALPPTINLLGELSVLVTTFSWSNITLLLTGLNMLVTALYSLYMFTTTQWGSLTHHINNMKPSFTRENTLMFMHLSPILLLSLNPDIITGFSS

SEQ ID NO: 161 - protein, 174 aa, synthetic construct
MMYALFLLSVGLVMGFVGFSSKPSPIYGGLVLIVSGVVGCVIILNFGGGYMGLMVFLIYLGGMMVVFGYTTAMAIEEYPEAWGSGVEVLVSVLVGLAMEVGLVLWVKEYDGVVVVVNFNSVGSWMIYEGEGSGLIREDPIGAGALYDYGRWLVVVTGWTLFVGVYIVIEIARGN

SEQ ID NO: 162 - protein, 316 aa, synthetic construct
MANLLLLIVPILIAMAFLMLTERKILGYMQLRKGPNVVGPYGLLQPFADAIKLFTKEPLKPATSTITLYITAPTLALTIALLLWTPLPMPNPLVNLNLGLLFILATSSLAVYSILWSGWASNSNYALIGALRAVAQTISYEVTLAIILLSTLLMSGSFNLSTLITTQEHLWLLLPSWPLAMMWFISTLAETNRTPFDLAEGESELVSGFNIEYAAGPFALFFMAEYTNIIMMNTLTTTIFLGTTYDALSPELYTTYFVTKTLLLTSLFLWIRTAYPRFRYDQLMHLLWKNFLPLTLALLMWYVSMPITISSIPPQT

SEQ ID NO: 163 - DNA, 18 bp, synthetic construct
  source 1..18: mol_type = other DNA
acaagttcagcgtgtccg

SEQ ID NO: 164 - DNA, 18 bp, synthetic construct
  source 1..18: mol_type = other DNA
ctcgttggggtctttgct

SEQ ID NO: 165 - DNA, 22 bp, synthetic construct
  source 1..22: mol_type = other DNA
atctccgcacactctctcctca

SEQ ID NO: 166 - DNA, 21 bp, synthetic construct
  source 1..21: mol_type = other DNA
taggttgttgttgatttggtt

SEQ ID NO: 167 - DNA, 18 bp, synthetic construct
  source 1..18: mol_type = other DNA
cctagaagcatttgcggt

SEQ ID NO: 168 - DNA, 18 bp, synthetic construct
  source 1..18: mol_type = other DNA
gagctacgagctgcctga

SEQ ID NO: 169 - DNA, 507 bp, synthetic construct
  source 1..507: mol_type = other DNA
cgttacataacttacggtaaatggcccgcctggctgaccgcccaacgacccccgcccattgacgtcaataatgacgtatgttcccatagtaacgccaatagggactttccattgacgtcaatgggtggagtatttacggtaaactgcccacttggcagtacatcaagtgtatcatatgccaagtacgccccctattgacgtcaatgacggtaaatggcccgcctggcattatgcccagtacatgaccttatgggactttcctacttggcagtacatctacgtattagtcatcgctattaccatggtgatgcggttttggcagtacatcaatgggcgtggatagcggtttgactcacggggatttccaagtctccaccccattgacgtcaatgggagtttgttttgcaccaaaatcaacgggactttccaaaatgtcgtaacaactccgccccattgacgcaaatgggcggtaggcgtgtacggtgggaggtctatataagcagagct

SEQ ID NO: 170 - DNA, 133 bp, synthetic construct
  source 1..133: mol_type = other DNA
gtaagtatcaaggttacaagacaggtttaaggagaccaatagaaactgggcttgtcgagacagagaagactcttgcgtttctgataggcacctattggtcttactgacatccactttgcctttctctccacag

SEQ ID NO: 171 - skipped

SEQ ID NO: 172 - DNA, 208 bp, synthetic construct
  source 1..208: mol_type = other DNA
ctgtgccttctagttgccagccatctgttgtttgcccctcccccgtgccttccttgaccctggaaggtgccactcccactgtcctttcctaataaaatgaggaaattgcatcgcattgtctgagtaggtgtcattctattctggggggtggggtggggcaggacagcaagggggaggattgggaagagaatagcaggcatgctgggga

SEQ ID NO: 173 - DNA, 122 bp, synthetic construct
  source 1..122: mol_type = other DNA
taagatacattgatgagtttggacaaaccacaactagaatgcagtgaaaaaaatgctttatttgtgaaatttgtgatgctattgctttatttgtaaccattataagctgcaataaacaagtt

SEQ ID NO: 174 - DNA, 3776 bp, synthetic construct
  source 1..3776: mol_type = other DNA
cgttacataacttacggtaaatggcccgcctggctgaccgcccaacgacccccgcccattgacgtcaataatgacgtatgttcccatagtaacgccaatagggactttccattgacgtcaatgggtggagtatttacggtaaactgcccacttggcagtacatcaagtgtatcatatgccaagtacgccccctattgacgtcaatgacggtaaatggcccgcctggcattatgcccagtacatgaccttatgggactttcctacttggcagtacatctacgtattagtcatcgctattaccatggtgatgcggttttggcagtacatcaatgggcgtggatagcggtttgactcacggggatttccaagtctccaccccattgacgtcaatgggagtttgttttgcaccaaaatcaacgggactttccaaaatgtcgtaacaactccgccccattgacgcaaatgggcggtaggcgtgtacggtgggaggtctatataagcagagctcgtttagtgaaccgtcagatcactagaagctttattgcggtagtttatcacagttaaattgctaacgcagtcagtgcttctgacacaacagtctcgaacttaagctgcagaagttggtcgtgaggcactgggcaggtaagtatcaaggttacaagacaggtttaaggagaccaatagaaactgggcttgtcgagacagagaagactcttgcgtttctgataggcacctattggtcttactgacatccactttgcctttctctccacaggtgtccactcccagttcaattacagctcttaaggctagagtacttaatacgactcactataggctagcctcgagaattcacgcgtggtaccgccaccggatccgccgccaccatggccgcatctccgcacactctctcctcacgcctcctgacaggttgcgtaggaggctctgtctggtatcttgaaagaagaactatgctaaaactaatcgtcccaacaattatgttactaccactgacatggctttccaaaaaacacatgatttggatcaacacaaccacccacagcctaattattagcatcatccctctactattttttaaccaaatcaacaacaacctatttagctgttccccaaccttttcctccgaccccctaacaacccccctcctaatgctaactacctggctcctacccctcacaatcatggcaagccaacgccacttatccagtgaaccactatcacgaaaaaaactctacctctctatgctaatctccctacaaatctccttaattatgacattcacagccacagaactaatcatgttttatatcttcttcgaaaccacacttatccccaccttggctatcatcacccgatggggcaaccagccagaacgcctgaacgcaggcacatacttcctattctacaccctagtaggctcccttcccctactcatcgcactaatttacactcacaacaccctaggctcactaaacattctactactcactctcactgcccaagaactatcaaactcctgggccaacaacttaatgtggctagcttacacaatggcttttatggtaaagatgcctctttacggactccacttatggctccctaaagcccatgtcgaagcccccatcgctgggtcaatggtacttgccgcagtactcttaaaactaggcggctatggtatgatgcgcctcacactcattctcaaccccctgacaaaacacatggcctaccccttccttgtactatccctatggggcatgattatgacaagctccatctgcctacgacaaacagacctaaaatcgctcattgcatactcttcaatcagccacatggccctcgtagtaacagccattctcatccaaaccccctggagcttcaccggcgcagtcattctcatgatcgcccacgggcttacatcctcattactattctgcctagcaaactcaaactacgaacgcactcacagtcgcatcatgatcctctctcaaggacttcaaactctactcccactaatggctttttggtggcttctagcaagcctcgctaacctcgccttaccccccactattaacctactgggagaactctctgtgctagtaaccacgttctcctggtcaaatatcactctcctacttacaggactcaacatgctagtcacagccctatactccctctacatgtttaccacaacacaatggggctcactcacccaccacattaacaacatgaaaccctcattcacacgagaaaacaccctcatgttcatgcacctatcccccattctcctcctatccctcaaccccgacatcattaccgggttttcctcttaagagcactgggacgcccaccgcccctttccctccgctgccaggcgagcatgttgtggtaattctggaacacaagaagagaaattgctgggtttagaacaagattataaacgaattcggtgctcagtgatcacttgacagttttttttttttttaaatattacccaaaatgctccccaaataagaaatgcatcagctcagtcagtgaatacaaaaaaggaattatttttccctttgagggtcttttatacatctctcctccaaccccaccctctattctgtttcttcctcctcacatgggggtacacatacacagcttcctcttttggttccatccttaccaccacaccacacgcacactccacatgcccagcagagtggcacttggtggccagaaagtgtgagcctcatgatctgctgtctgtagttctgtgagctcaggtccctcaaaggcctcggagcacccccttccttgtgactgagccagggcctgcatttttggttttccccaccccacacattctcaaccatagtccttctaacaataccaatagctaggacccggctgctgtgcactgggactggggattccacatgtttgccttgggagtctcaagctggactgccagcccctgtcctcccttcacccccattgcgtatgagcatttcagaactccaaggagtcacaggcatctttatagttcacgttaacatatagacactgttggaagcagttccttctaaaagggtagccctggacttaataccagccggatacctctggcccccaccccattactgtacctctggagtcactactgtgggtcgccactcctctgctacacagcacggctttttcaaggctgtattgagaagggaagttaggaagaagggtgtgctgggctaaccagcccacagagctcacattcctgtcccttgggtgaaaaatacatgtccatcctgatatctcctgaattcagaaattagcctccacatgtgcaatggctttaagagccagaagcagggttctgggaattttgcaagttacctgtggccaggtgtggtctcggttaccaaatacggttacctgcagctttttagtcctttgtgctcccacgggtctacagagtcccatctgcccaaaggtcttgaagcttgacaggatgttttcgattactcagtctcccagggcactactggtccgtaggattcgattggtcggggtaggagagttaaacaacatttaaacagagttctctcaaaaatgtctaaagggattgtaggtagataacatccaatcactgtttgcacttatctgaaatcttccctcttggctgcccccaggtatttactgtggagaacattgcataggaatgtctggaaaaagcttctacaacttgttacagccttcacatttgtagaagcttt

SEQ ID NO: 175 - DNA, 4007 bp, synthetic construct
  source 1..4007: mol_type = other DNA
cgttacataacttacggtaaatggcccgcctggctgaccgcccaacgacccccgcccattgacgtcaataatgacgtatgttcccatagtaacgccaatagggactttccattgacgtcaatgggtggagtatttacggtaaactgcccacttggcagtacatcaagtgtatcatatgccaagtacgccccctattgacgtcaatgacggtaaatggcccgcctggcattatgcccagtacatgaccttatgggactttcctacttggcagtacatctacgtattagtcatcgctattaccatggtgatgcggttttggcagtacatcaatgggcgtggatagcggtttgactcacggggatttccaagtctccaccccattgacgtcaatgggagtttgttttgcaccaaaatcaacgggactttccaaaatgtcgtaacaactccgccccattgacgcaaatgggcggtaggcgtgtacggtgggaggtctatataagcagagctcgtttagtgaaccgtcagatcactagaagctttattgcggtagtttatcacagttaaattgctaacgcagtcagtgcttctgacacaacagtctcgaacttaagctgcagaagttggtcgtgaggcactgggcaggtaagtatcaaggttacaagacaggtttaaggagaccaatagaaactgggcttgtcgagacagagaagactcttgcgtttctgataggcacctattggtcttactgacatccactttgcctttctctccacaggtgtccactcccagttcaattacagctcttaaggctagagtacttaatacgactcactataggctagcctcgagaattcacgcgtggtaccgccaccggatccgccgccaccatggccgcatctccgcacactctctcctcacgcctcctgacaggttgcgtaggaggctctgtctggtatcttgaaagaagaactatgctaaaactaatcgtcccaacaattatgttactaccactgacatggctttccaaaaaacacatgatttggatcaacacaaccacccacagcctaattattagcatcatccctctactattttttaaccaaatcaacaacaacctatttagctgttccccaaccttttcctccgaccccctaacaacccccctcctaatgctaactacctggctcctacccctcacaatcatggcaagccaacgccacttatccagtgaaccactatcacgaaaaaaactctacctctctatgctaatctccctacaaatctccttaattatgacattcacagccacagaactaatcatgttttatatcttcttcgaaaccacacttatccccaccttggctatcatcacccgatggggcaaccagccagaacgcctgaacgcaggcacatacttcctattctacaccctagtaggctcccttcccctactcatcgcactaatttacactcacaacaccctaggctcactaaacattctactactcactctcactgcccaagaactatcaaactcctgggccaacaacttaatgtggctagcttacacaatggcttttatggtaaagatgcctctttacggactccacttatggctccctaaagcccatgtcgaagcccccatcgctgggtcaatggtacttgccgcagtactcttaaaactaggcggctatggtatgatgcgcctcacactcattctcaaccccctgacaaaacacatggcctaccccttccttgtactatccctatggggcatgattatgacaagctccatctgcctacgacaaacagacctaaaatcgctcattgcatactcttcaatcagccacatggccctcgtagtaacagccattctcatccaaaccccctggagcttcaccggcgcagtcattctcatgatcgcccacgggcttacatcctcattactattctgcctagcaaactcaaactacgaacgcactcacagtcgcatcatgatcctctctcaaggacttcaaactctactcccactaatggctttttggtggcttctagcaagcctcgctaacctcgccttaccccccactattaacctactgggagaactctctgtgctagtaaccacgttctcctggtcaaatatcactctcctacttacaggactcaacatgctagtcacagccctatactccctctacatgtttaccacaacacaatggggctcactcacccaccacattaacaacatgaaaccctcattcacacgagaaaacaccctcatgttcatgcacctatcccccattctcctcctatccctcaaccccgacatcattaccgggttttcctcttaagagcactgggacgcccaccgcccctttccctccgctgccaggcgagcatgttgtggtaattctggaacacaagaagagaaattgctgggtttagaacaagattataaacgaattcggtgctcagtgatcacttgacagttttttttttttttaaatattacccaaaatgctccccaaataagaaatgcatcagctcagtcagtgaatacaaaaaaggaattatttttccctttgagggtcttttatacatctctcctccaaccccaccctctattctgtttcttcctcctcacatgggggtacacatacacagcttcctcttttggttccatccttaccaccacaccacacgcacactccacatgcccagcagagtggcacttggtggccagaaagtgtgagcctcatgatctgctgtctgtagttctgtgagctcaggtccctcaaaggcctcggagcacccccttccttgtgactgagccagggcctgcatttttggttttccccaccccacacattctcaaccatagtccttctaacaataccaatagctaggacccggctgctgtgcactgggactggggattccacatgtttgccttgggagtctcaagctggactgccagcccctgtcctcccttcacccccattgcgtatgagcatttcagaactccaaggagtcacaggcatctttatagttcacgttaacatatagacactgttggaagcagttccttctaaaagggtagccctggacttaataccagccggatacctctggcccccaccccattactgtacctctggagtcactactgtgggtcgccactcctctgctacacagcacggctttttcaaggctgtattgagaagggaagttaggaagaagggtgtgctgggctaaccagcccacagagctcacattcctgtcccttgggtgaaaaatacatgtccatcctgatatctcctgaattcagaaattagcctccacatgtgcaatggctttaagagccagaagcagggttctgggaattttgcaagttacctgtggccaggtgtggtctcggttaccaaatacggttacctgcagctttttagtcctttgtgctcccacgggtctacagagtcccatctgcccaaaggtcttgaagcttgacaggatgttttcgattactcagtctcccagggcactactggtccgtaggattcgattggtcggggtaggagagttaaacaacatttaaacagagttctctcaaaaatgtctaaagggattgtaggtagataacatccaatcactgtttgcacttatctgaaatcttccctcttggctgcccccaggtatttactgtggagaacattgcataggaatgtctggaaaaagcttctacaacttgttacagccttcacatttgtagaagctttgcggccgcttcgagcagacatgactgtgccttctagttgccagccatctgttgtttgcccctcccccgtgccttccttgaccctggaaggtgccactcccactgtcctttcctaataaaatgaggaaattgcatcgcattgtctgagtaggtgtcattctattctggggggtggggtggggcaggacagcaagggggaggattgggaagagaatagcaggcatgctgggga

SEQ ID NO: 176 - DNA, 3921 bp, synthetic construct
  source 1..3921: mol_type = other DNA
cgttacataacttacggtaaatggcccgcctggctgaccgcccaacgacccccgcccattgacgtcaataatgacgtatgttcccatagtaacgccaatagggactttccattgacgtcaatgggtggagtatttacggtaaactgcccacttggcagtacatcaagtgtatcatatgccaagtacgccccctattgacgtcaatgacggtaaatggcccgcctggcattatgcccagtacatgaccttatgggactttcctacttggcagtacatctacgtattagtcatcgctattaccatggtgatgcggttttggcagtacatcaatgggcgtggatagcggtttgactcacggggatttccaagtctccaccccattgacgtcaatgggagtttgttttgcaccaaaatcaacgggactttccaaaatgtcgtaacaactccgccccattgacgcaaatgggcggtaggcgtgtacggtgggaggtctatataagcagagctcgtttagtgaaccgtcagatcactagaagctttattgcggtagtttatcacagttaaattgctaacgcagtcagtgcttctgacacaacagtctcgaacttaagctgcagaagttggtcgtgaggcactgggcaggtaagtatcaaggttacaagacaggtttaaggagaccaatagaaactgggcttgtcgagacagagaagactcttgcgtttctgataggcacctattggtcttactgacatccactttgcctttctctccacaggtgtccactcccagttcaattacagctcttaaggctagagtacttaatacgactcactataggctagcctcgagaattcacgcgtggtaccgccaccggatccgccgccaccatggccgcatctccgcacactctctcctcacgcctcctgacaggttgcgtaggaggctctgtctggtatcttgaaagaagaactatgctaaaactaatcgtcccaacaattatgttactaccactgacatggctttccaaaaaacacatgatttggatcaacacaaccacccacagcctaattattagcatcatccctctactattttttaaccaaatcaacaacaacctatttagctgttccccaaccttttcctccgaccccctaacaacccccctcctaatgctaactacctggctcctacccctcacaatcatggcaagccaacgccacttatccagtgaaccactatcacgaaaaaaactctacctctctatgctaatctccctacaaatctccttaattatgacattcacagccacagaactaatcatgttttatatcttcttcgaaaccacacttatccccaccttggctatcatcacccgatggggcaaccagccagaacgcctgaacgcaggcacatacttcctattctacaccctagtaggctcccttcccctactcatcgcactaatttacactcacaacaccctaggctcactaaacattctactactcactctcactgcccaagaactatcaaactcctgggccaacaacttaatgtggctagcttacacaatggcttttatggtaaagatgcctctttacggactccacttatggctccctaaagcccatgtcgaagcccccatcgctgggtcaatggtacttgccgcagtactcttaaaactaggcggctatggtatgatgcgcctcacactcattctcaaccccctgacaaaacacatggcctaccccttccttgtactatccctatggggcatgattatgacaagctccatctgcctacgacaaacagacctaaaatcgctcattgcatactcttcaatcagccacatggccctcgtagtaacagccattctcatccaaaccccctggagcttcaccggcgcagtcattctcatgatcgcccacgggcttacatcctcattactattctgcctagcaaactcaaactacgaacgcactcacagtcgcatcatgatcctctctcaaggacttcaaactctactcccactaatggctttttggtggcttctagcaagcctcgctaacctcgccttaccccccactattaacctactgggagaactctctgtgctagtaaccacgttctcctggtcaaatatcactctcctacttacaggactcaacatgctagtcacagccctatactccctctacatgtttaccacaacacaatggggctcactcacccaccacattaacaacatgaaaccctcattcacacgagaaaacaccctcatgttcatgcacctatcccccattctcctcctatccctcaaccccgacatcattaccgggttttcctcttaagagcactgggacgcccaccgcccctttccctccgctgccaggcgagcatgttgtggtaattctggaacacaagaagagaaattgctgggtttagaacaagattataaacgaattcggtgctcagtgatcacttgacagttttttttttttttaaatattacccaaaatgctccccaaataagaaatgcatcagctcagtcagtgaatacaaaaaaggaattatttttccctttgagggtcttttatacatctctcctccaaccccaccctctattctgtttcttcctcctcacatgggggtacacatacacagcttcctcttttggttccatccttaccaccacaccacacgcacactccacatgcccagcagagtggcacttggtggccagaaagtgtgagcctcatgatctgctgtctgtagttctgtgagctcaggtccctcaaaggcctcggagcacccccttccttgtgactgagccagggcctgcatttttggttttccccaccccacacattctcaaccatagtccttctaacaataccaatagctaggacccggctgctgtgcactgggactggggattccacatgtttgccttgggagtctcaagctggactgccagcccctgtcctcccttcacccccattgcgtatgagcatttcagaactccaaggagtcacaggcatctttatagttcacgttaacatatagacactgttggaagcagttccttctaaaagggtagccctggacttaataccagccggatacctctggcccccaccccattactgtacctctggagtcactactgtgggtcgccactcctctgctacacagcacggctttttcaaggctgtattgagaagggaagttaggaagaagggtgtgctgggctaaccagcccacagagctcacattcctgtcccttgggtgaaaaatacatgtccatcctgatatctcctgaattcagaaattagcctccacatgtgcaatggctttaagagccagaagcagggttctgggaattttgcaagttacctgtggccaggtgtggtctcggttaccaaatacggttacctgcagctttttagtcctttgtgctcccacgggtctacagagtcccatctgcccaaaggtcttgaagcttgacaggatgttttcgattactcagtctcccagggcactactggtccgtaggattcgattggtcggggtaggagagttaaacaacatttaaacagagttctctcaaaaatgtctaaagggattgtaggtagataacatccaatcactgtttgcacttatctgaaatcttccctcttggctgcccccaggtatttactgtggagaacattgcataggaatgtctggaaaaagcttctacaacttgttacagccttcacatttgtagaagctttgcggccgcttcgagcagacatgataagatacattgatgagtttggacaaaccacaactagaatgcagtgaaaaaaatgctttatttgtgaaatttgtgatgctattgctttatttgtaaccattataagctgcaataaacaagtt

SEQ ID NO: 177 - DNA, 10 bp, synthetic construct
  source 1..10: mol_type = other DNA
gccaccatgg

SEQ ID NO: 178 - DNA, 141 bp, synthetic construct
  source 1..141: mol_type = other DNA
cctgcaggcagctgcgcgctcgctcgctcactgaggccgcccgggcgtcgggcgacctttggtcgcccgacgcccgggcggcctcagtgagcgagcgagcgcgcagagagggagtggccaactccatcactaggggttcct

SEQ ID NO: 179 - DNA, 141 bp, synthetic construct
  source 1..141: mol_type = other DNA
aggaacccctagtgatggagttggccactccctctctgcgcgctcgctcgctcactgaggccgggcgaccaaaggtcgcccgacgcccgggctttgcccgggcggcctcagtgagcgagcgagcgcgcagctgcctgcagg

SEQ ID NO: 180 - DNA, 4375 bp, synthetic construct
  source 1..4375: mol_type = other DNA
cctgcaggcagctgcgcgctcgctcgctcactgaggccgcccgggcgtcgggcgacctttggtcgcccgacgcccgggcggcctcagtgagcgagcgagcgcgcagagagggagtggccaactccatcactaggggttcctgcggccgcacgcgtctagttattaatagtaatcaattacggggtcattagttcatagcccatatatggagttccgcgttacataacttacggtaaatggcccgcctggctgaccgcccaacgacccccgcccattgacgtcaataatgacgtatgttcccatagtaacgccaatagggactttccattgacgtcaatgggtggagtatttacggtaaactgcccacttggcagtacatcaagtgtatcatatgccaagtacgccccctattgacgtcaatgacggtaaatggcccgcctggcattatgcccagtacatgaccttatgggactttcctacttggcagtacatctacgtattagtcatcgctattaccatggtgatgcggttttggcagtacatcaatgggcgtggatagcggtttgactcacggggatttccaagtctccaccccattgacgtcaatgggagtttgttttgcaccaaaatcaacgggactttccaaaatgtcgtaacaactccgccccattgacgcaaatgggcggtaggcgtgtacggtgggaggtctatataagcagagctcgtttagtgaaccgtcagatcactagaagctttattgcggtagtttatcacagttaaattgctaacgcagtcagtgcttctgacacaacagtctcgaacttaagctgcagaagttggtcgtgaggcactgggcaggtaagtatcaaggttacaagacaggtttaaggagaccaatagaaactgggcttgtcgagacagagaagactcttgcgtttctgataggcacctattggtcttactgacatccactttgcctttctctccacaggtgtccactcccagttcaattacagctcttaaggctagagtacttaatacgactcactataggctagcctcgagaattcacgcgtggtaccgccaccggatccgccgccaccatggccgcatctccgcacactctctcctcacgcctcctgacaggttgcgtaggaggctctgtctggtatcttgaaagaagaactatgctaaaactaatcgtcccaacaattatgttactaccactgacatggctttccaaaaaacacatgatttggatcaacacaaccacccacagcctaattattagcatcatccctctactattttttaaccaaatcaacaacaacctatttagctgttccccaaccttttcctccgaccccctaacaacccccctcctaatgctaactacctggctcctacccctcacaatcatggcaagccaacgccacttatccagtgaaccactatcacgaaaaaaactctacctctctatgctaatctccctacaaatctccttaattatgacattcacagccacagaactaatcatgttttatatcttcttcgaaaccacacttatccccaccttggctatcatcacccgatggggcaaccagccagaacgcctgaacgcaggcacatacttcctattctacaccctagtaggctcccttcccctactcatcgcactaatttacactcacaacaccctaggctcactaaacattctactactcactctcactgcccaagaactatcaaactcctgggccaacaacttaatgtggctagcttacacaatggcttttatggtaaagatgcctctttacggactccacttatggctccctaaagcccatgtcgaagcccccatcgctgggtcaatggtacttgccgcagtactcttaaaactaggcggctatggtatgatgcgcctcacactcattctcaaccccctgacaaaacacatggcctaccccttccttgtactatccctatggggcatgattatgacaagctccatctgcctacgacaaacagacctaaaatcgctcattgcatactcttcaatcagccacatggccctcgtagtaacagccattctcatccaaaccccctggagcttcaccggcgcagtcattctcatgatcgcccacgggcttacatcctcattactattctgcctagcaaactcaaactacgaacgcactcacagtcgcatcatgatcctctctcaaggacttcaaactctactcccactaatggctttttggtggcttctagcaagcctcgctaacctcgccttaccccccactattaacctactgggagaactctctgtgctagtaaccacgttctcctggtcaaatatcactctcctacttacaggactcaacatgctagtcacagccctatactccctctacatgtttaccacaacacaatggggctcactcacccaccacattaacaacatgaaaccctcattcacacgagaaaacaccctcatgttcatgcacctatcccccattctcctcctatccctcaaccccgacatcattaccgggttttcctcttaagagcactgggacgcccaccgcccctttccctccgctgccaggcgagcatgttgtggtaattctggaacacaagaagagaaattgctgggtttagaacaagattataaacgaattcggtgctcagtgatcacttgacagttttttttttttttaaatattacccaaaatgctccccaaataagaaatgcatcagctcagtcagtgaatacaaaaaaggaattatttttccctttgagggtcttttatacatctctcctccaaccccaccctctattctgtttcttcctcctcacatgggggtacacatacacagcttcctcttttggttccatccttaccaccacaccacacgcacactccacatgcccagcagagtggcacttggtggccagaaagtgtgagcctcatgatctgctgtctgtagttctgtgagctcaggtccctcaaaggcctcggagcacccccttccttgtgactgagccagggcctgcatttttggttttccccaccccacacattctcaaccatagtccttctaacaataccaatagctaggacccggctgctgtgcactgggactggggattccacatgtttgccttgggagtctcaagctggactgccagcccctgtcctcccttcacccccattgcgtatgagcatttcagaactccaaggagtcacaggcatctttatagttcacgttaacatatagacactgttggaagcagttccttctaaaagggtagccctggacttaataccagccggatacctctggcccccaccccattactgtacctctggagtcactactgtgggtcgccactcctctgctacacagcacggctttttcaaggctgtattgagaagggaagttaggaagaagggtgtgctgggctaaccagcccacagagctcacattcctgtcccttgggtgaaaaatacatgtccatcctgatatctcctgaattcagaaattagcctccacatgtgcaatggctttaagagccagaagcagggttctgggaattttgcaagttacctgtggccaggtgtggtctcggttaccaaatacggttacctgcagctttttagtcctttgtgctcccacgggtctacagagtcccatctgcccaaaggtcttgaagcttgacaggatgttttcgattactcagtctcccagggcactactggtccgtaggattcgattggtcggggtaggagagttaaacaacatttaaacagagttctctcaaaaatgtctaaagggattgtaggtagataacatccaatcactgtttgcacttatctgaaatcttccctcttggctgcccccaggtatttactgtggagaacattgcataggaatgtctggaaaaagcttctacaacttgttacagccttcacatttgtagaagctttgcggccgcttcgagcagacatgataagatacattgatgagtttggacaaaccacaactagaatgcagtgaaaaaaatgctttatttgtgaaatttgtgatgctattgctttatttgtaaccattataagctgcaataaacaagttaacaacaacactcgagttaagggcgaattcccgataaggatcttcctagagcatggctacgtagataagtagcatggcgggttaatcattaactacaaggaacccctagtgatggagttggccactccctctctgcgcgctcgctcgctcactgaggccgggcgaccaaaggtcgcccgacgcccgggctttgcccgggcggcctcagtgagcgagcgagcgcgcagctgcctgcagg

SEQ ID NO: 181 - DNA, 16 bp, synthetic construct
  source 1..16: mol_type = other DNA
agaccatgacggtgat

SEQ ID NO: 182 - DNA, 17 bp, synthetic construct
  source 1..17: mol_type = other DNA
cttgtcatcgtcatcct

SEQ ID NO: 183 - DNA, 20 bp, synthetic construct
  source 1..20: mol_type = other DNA
ggacttcgagcaagagatgg

SEQ ID NO: 184 - DNA, 20 bp, synthetic construct
  source 1..20: mol_type = other DNA
aggaaggaaggctggaagag

SEQ ID NO: 185 - DNA, 23 bp, synthetic construct
  source 1..23: mol_type = other DNA
gcggccgcttcgagcagacatga